European Patent Application EP 4 711 004 A2, published March 18, 2026. Title: METHOD OF TREATING MELANOCORTIN-4 RECEPTOR PATHWAY-ASSOCIATED DISORDERS. Applicant: RHYTHM PHARMACEUTICALS, INC. Application EP 25218416.3, filed September 29, 2016. The sequence listing filed with the application follows.

SEQUENCE LISTING (614 sequences)

SEQ ID NO: 1 - protein, 8 aa, synthetic construct
  REGION 1..8: note = Description of Artificial Sequence: Synthetic peptide
  MOD_RES 1: note = Nle
  MOD_RES 4: note = D-Phenylalanine
  MOD_RES 7: note = Beta-Alanine
XDHFRWAK

SEQ ID NO: 2 - protein, 8 aa, synthetic construct
  REGION 1..8: note = Description of Artificial Sequence: Synthetic peptide
  MOD_RES 1: note = Nle
  MOD_RES 4: note = D-Phenylalanine
  MOD_RES 7: note = 1-amino-1-cyclohexanecarboxylic acid
XDHFRWXK

SEQ ID NO: 3 - protein, 8 aa, synthetic construct
  REGION 1..8: note = Description of Artificial Sequence: Synthetic peptide
  MOD_RES 1: note = Nle
  MOD_RES 4: note = D-Phenylalanine
  MOD_RES 7: note = 6-aminohexanoic acid
XCHFRWXC

SEQ ID NO: 4 - protein, 9 aa, synthetic construct
  REGION 1..9: note = Description of Artificial Sequence: Synthetic peptide
  MOD_RES 1: note = D-Phenylalanine
  MOD_RES 4: note = D-Phenylalanine
  MOD_RES 8: note = D-Cysteine
FCHFRWACT

SEQ ID NO: 5 - protein, 9 aa, synthetic construct
  REGION 1..9: note = Description of Artificial Sequence: Synthetic peptide
  MOD_RES 1: note = D-Phenylalanine
  MOD_RES 4: note = D-Phenylalanine
  MOD_RES 7: note = Beta-Alanine
  MOD_RES 8: note = D-Cysteine
FCHFRWACT

SEQ ID NO: 6 - protein, 9 aa, synthetic construct
  REGION 1..9: note = Description of Artificial Sequence: Synthetic peptide
  MOD_RES 1: note = D-Phenylalanine
  MOD_RES 4: note = D-Phenylalanine
  MOD_RES 7: note = 4-aminobutyric acid
  MOD_RES 8: note = D-Cysteine
FCHFRWXCT

SEQ ID NO: 7 - protein, 8 aa, synthetic construct
  REGION 1..8: note = Description of Artificial Sequence: Synthetic peptide
  MOD_RES 1: note = Nle
  MOD_RES 4: note = D-Phenylalanine
  MOD_RES 7: note = 5-aminopentanoic acid (HN-(CH2)4-C(O)
XCHFRWXC

SEQ ID NO: 8 - protein, 8 aa, synthetic construct
  REGION 1..8: note = Description of Artificial Sequence: Synthetic peptide
  MOD_RES 1: note = Nle
  MOD_RES 4: note = D-Phenylalanine
  MOD_RES 7: note = Beta-Alanine
XDHFRWXK

SEQ ID NO: 9 - protein, 8 aa, synthetic construct
  REGION 1..8: note = Description of Artificial Sequence: Synthetic peptide
  MOD_RES 1: note = 1-amino-1-cyclohexanecarboxylic acid
  MOD_RES 4: note = D-Phenylalanine
  MOD_RES 7: note = 4-aminobutyric acid
XDHFRWXK

SEQ ID NO: 10 - protein, 8 aa, synthetic construct
  REGION 1..8: note = Description of Artificial Sequence: Synthetic peptide
  MOD_RES 1: note = D-Beta-(2-naphthyl)alanine
  MOD_RES 4: note = D-Phenylalanine
  MOD_RES 7: note = 4-aminobutyric acid
XDHFRWXK

SEQ ID NO: 11 - protein, 8 aa, synthetic construct
  REGION 1..8: note = Description of Artificial Sequence: Synthetic peptide
  MOD_RES 1: note = beta-cyclohexylalanine
  MOD_RES 4: note = D-Phenylalanine
  MOD_RES 7: note = 4-aminobutyric acid
XDHFRWXK

SEQ ID NO: 12 - protein, 8 aa, synthetic construct
  REGION 1..8: note = Description of Artificial Sequence: Synthetic peptide
  MOD_RES 1: note = Nle
  MOD_RES 4: note = D-Phenylalanine
  MOD_RES 7: note = 4-aminobutyric acid
XDHFRWXK

SEQ ID NO: 13 - protein, 8 aa, synthetic construct
  REGION 1..8: note = Description of Artificial Sequence: Synthetic peptide
  MOD_RES 1: note = Nle
  MOD_RES 3: note = D-Alanine
  MOD_RES 5: note = D-Phenylalanine
XCAHFRWC

SEQ ID NO: 14 - protein, 8 aa, synthetic construct
  REGION 1..8: note = Description of Artificial Sequence: Synthetic peptide
  MOD_RES 1: note = Nle
  MOD_RES 3: note = Beta-Alanine
  MOD_RES 5: note = D-Phenylalanine
XCAHFRWC

SEQ ID NO: 15 - protein, 8 aa, synthetic construct
  REGION 1..8: note = Description of Artificial Sequence: Synthetic peptide
  MOD_RES 1: note = Nle
  MOD_RES 3: note = 4-aminobutyric acid
  MOD_RES 5: note = D-Phenylalanine
XCXHFRWC

SEQ ID NO: 16 - protein, 8 aa, synthetic construct
  REGION 1..8: note = Description of Artificial Sequence: Synthetic peptide
  MOD_RES 1: note = Nle
  MOD_RES 3: note = alpha-aminoisobutyric acid
  MOD_RES 5: note = D-Phenylalanine
XCXHFRWC

SEQ ID NO: 17 - protein, 8 aa, synthetic construct
  REGION 1..8: note = Description of Artificial Sequence: Synthetic peptide
  MOD_RES 1: note = Nle
  MOD_RES 5: note = D-Phenylalanine
XCGHFRWC

SEQ ID NO: 18 - protein, 8 aa, synthetic construct
  REGION 1..8: note = Description of Artificial Sequence: Synthetic peptide
  MOD_RES 1: note = Nle
  MOD_RES 2: note = D-Cysteine
  MOD_RES 5: note = D-Phenylalanine
XCAHFRWC

SEQ ID NO: 19 - protein, 8 aa, synthetic construct
  REGION 1..8: note = Description of Artificial Sequence: Synthetic peptide
  MOD_RES 1: note = Nle
  MOD_RES 2: note = D-Cysteine
  MOD_RES 3: note = D-Alanine
  MOD_RES 5: note = D-Phenylalanine
XCAHFRWC

SEQ ID NO: 20 - protein, 8 aa, synthetic construct
  REGION 1..8: note = Description of Artificial Sequence: Synthetic peptide
  MOD_RES 1: note = Nle
  MOD_RES 2: note = D-Cysteine
  MOD_RES 3: note = Beta-Alanine
  MOD_RES 5: note = D-Phenylalanine
XCAHFRWC

SEQ ID NO: 21 - protein, 8 aa, synthetic construct
  REGION 1..8: note = Description of Artificial Sequence: Synthetic peptide
  MOD_RES 1: note = Nle
  MOD_RES 2: note = D-Cysteine
  MOD_RES 3: note = 4-aminobutyric acid
  MOD_RES 5: note = D-Phenylalanine
XCXHFRWC

SEQ ID NO: 22 - protein, 8 aa, synthetic construct
  REGION 1..8: note = Description of Artificial Sequence: Synthetic peptide
  MOD_RES 1: note = Nle
  MOD_RES 2: note = D-Cysteine
  MOD_RES 3: note = alpha-aminoisobutyric acid
  MOD_RES 5: note = D-Phenylalanine
XCXHFRWC

SEQ ID NO: 23 - protein, 8 aa, synthetic construct
  REGION 1..8: note = Description of Artificial Sequence: Synthetic peptide
  MOD_RES 1: note = Nle
  MOD_RES 2: note = D-Cysteine
  MOD_RES 5: note = D-Phenylalanine
XCGHFRWC

SEQ ID NO: 24 - protein, 8 aa, synthetic construct
  REGION 1..8: note = Description of Artificial Sequence: Synthetic peptide
  MOD_RES 1: note = Nle
  MOD_RES 3: note = D-Alanine
  MOD_RES 5: note = D-Phenylalanine
  MOD_RES 8: note = D-Cysteine
XCAHFRWC

SEQ ID NO: 25 - protein, 8 aa, synthetic construct
  REGION 1..8: note = Description of Artificial Sequence: Synthetic peptide
  MOD_RES 1: note = Nle
  MOD_RES 3: note = Beta-Alanine
  MOD_RES 5: note = D-Phenylalanine
  MOD_RES 8: note = D-Cysteine
XCAHFRWC

SEQ ID NO: 26 - protein, 8 aa, synthetic construct
  REGION 1..8: note = Description of Artificial Sequence: Synthetic peptide
  MOD_RES 1: note = Nle
  MOD_RES 3: note = 4-aminobutyric acid
  MOD_RES 5: note = D-Phenylalanine
  MOD_RES 8: note = D-Cysteine
XCXHFRWC

SEQ ID NO: 27 - protein, 8 aa, synthetic construct
  REGION 1..8: note = Description of Artificial Sequence: Synthetic peptide
  MOD_RES 1: note = Nle
  MOD_RES 3: note = alpha-aminoisobutyric acid
  MOD_RES 5: note = D-Phenylalanine
  MOD_RES 8: note = D-Cysteine
XCXHFRWC

SEQ ID NO: 28 - protein, 8 aa, synthetic construct
  REGION 1..8: note = Description of Artificial Sequence: Synthetic peptide
  MOD_RES 1: note = Nle
  MOD_RES 5: note = D-Phenylalanine
  MOD_RES 8: note = D-Cysteine
XCGHFRWC

SEQ ID NO: 29 - protein, 8 aa, synthetic construct
  REGION 1..8: note = Description of Artificial Sequence: Synthetic peptide
  MOD_RES 1: note = Nle
  MOD_RES 2: note = D-Cysteine
  MOD_RES 5: note = D-Phenylalanine
  MOD_RES 8: note = D-Cysteine
XCAHFRWC

SEQ ID NO: 30 - protein, 8 aa, synthetic construct
  REGION 1..8: note = Description of Artificial Sequence: Synthetic peptide
  MOD_RES 1: note = Nle
  MOD_RES 2: note = D-Cysteine
  MOD_RES 3: note = D-Alanine
  MOD_RES 5: note = D-Phenylalanine
  MOD_RES 8: note = D-Cysteine
XCAHFRWC

SEQ ID NO: 31 - protein, 8 aa, synthetic construct
  REGION 1..8: note = Description of Artificial Sequence: Synthetic peptide
  MOD_RES 1: note = Nle
  MOD_RES 2: note = D-Cysteine
  MOD_RES 3: note = Beta-Alanine
  MOD_RES 5: note = D-Phenylalanine
  MOD_RES 8: note = D-Cysteine
XCAHFRWC

SEQ ID NO: 32 - protein, 8 aa, synthetic construct
  REGION 1..8: note = Description of Artificial Sequence: Synthetic peptide
  MOD_RES 1: note = Nle
  MOD_RES 2: note = D-Cysteine
  MOD_RES 3: note = 4-aminobutyric acid
  MOD_RES 5: note = D-Phenylalanine
  MOD_RES 8: note = D-Cysteine
XCXHFRWC

SEQ ID NO: 33 - protein, 8 aa, synthetic construct
  REGION 1..8: note = Description of Artificial Sequence: Synthetic peptide
  MOD_RES 1: note = Nle
  MOD_RES 2: note = D-Cysteine
  MOD_RES 3: note = alpha-aminoisobutyric acid
  MOD_RES 5: note = D-Phenylalanine
  MOD_RES 8: note = D-Cysteine
XCXHFRWC

SEQ ID NO: 34 - protein, 8 aa, synthetic construct
  REGION 1..8: note = Description of Artificial Sequence: Synthetic peptide
  MOD_RES 1: note = Oic
  MOD_RES 4: note = D-Phenylalanine
  MOD_RES 7: note = 4-aminobutyric acid
XDHFRWXK

SEQ ID NO: 35 - protein, 8 aa, synthetic construct
  REGION 1..8: note = Description of Artificial Sequence: Synthetic peptide
  MOD_RES 1: note = Cyclohexylglycine
  MOD_RES 4: note = D-Phenylalanine
  MOD_RES 7: note = 4-aminobutyric acid
XDHFRWXK

SEQ ID NO: 36 - protein, 8 aa, synthetic construct
  REGION 1..8: note = Description of Artificial Sequence: Synthetic peptide
  MOD_RES 1: note = homo-cyclohexylalanine
  MOD_RES 4: note = D-Phenylalanine
  MOD_RES 7: note = 4-aminobutyric acid
XDHFRWXK

SEQ ID NO: 37 - protein, 8 aa, synthetic construct
  REGION 1..8: note = Description of Artificial Sequence: Synthetic peptide
  MOD_RES 1: note = D-beta-cyclohexylalanine
  MOD_RES 4: note = D-Phenylalanine
  MOD_RES 7: note = 4-aminobutyric acid
XDHFRWXK

SEQ ID NO: 38 - protein, 8 aa, synthetic construct
  REGION 1..8: note = Description of Artificial Sequence: Synthetic peptide
  MOD_RES 1: note = D-homo-cyclohexylalanine
  MOD_RES 4: note = D-Phenylalanine
  MOD_RES 7: note = 4-aminobutyric acid
XDHFRWXK

SEQ ID NO: 39 - protein, 8 aa, synthetic construct
  REGION 1..8: note = Description of Artificial Sequence: Synthetic peptide
  MOD_RES 1: note = nipecotic acid
  MOD_RES 4: note = D-Phenylalanine
  MOD_RES 7: note = 4-aminobutyric acid
XDHFRWXK

SEQ ID NO: 40 - protein, 8 aa, synthetic construct
  REGION 1..8: note = Description of Artificial Sequence: Synthetic peptide
  MOD_RES 4: note = D-Phenylalanine
  MOD_RES 7: note = 4-aminobutyric acid
PDHFRWXK

SEQ ID NO: 41 - protein, 8 aa, synthetic construct
  REGION 1..8: note = Description of Artificial Sequence: Synthetic peptide
  MOD_RES 4: note = D-Phenylalanine
  MOD_RES 7: note = 4-aminobutyric acid
LDHFRWXK

SEQ ID NO: 42 - protein, 8 aa, synthetic construct
  REGION 1..8: note = Description of Artificial Sequence: Synthetic peptide
  MOD_RES 4: note = D-Phenylalanine
  MOD_RES 7: note = 4-aminobutyric acid
FDHFRWXK

SEQ ID NO: 43 - protein, 8 aa, synthetic construct
  REGION 1..8: note = Description of Artificial Sequence: Synthetic peptide
  MOD_RES 1: note = D-Phenylalanine
  MOD_RES 4: note = D-Phenylalanine
  MOD_RES 7: note = 4-aminobutyric acid
FDHFRWXK

SEQ ID NO: 44 - protein, 8 aa, synthetic construct
  REGION 1..8: note = Description of Artificial Sequence: Synthetic peptide
  MOD_RES 1: note = D-Cyclohexylglycine
  MOD_RES 4: note = D-Phenylalanine
  MOD_RES 7: note = 4-aminobutyric acid
XDHFRWXK

SEQ ID NO: 45 - protein, 8 aa, synthetic construct
  REGION 1..8: note = Description of Artificial Sequence: Synthetic peptide
  MOD_RES 1: note = beta-cyclohexylalanine
  MOD_RES 4: note = D-Phenylalanine
  MOD_RES 7: note = 4-aminobutyric acid
XDHFRWXK

SEQ ID NO: 46 - protein, 8 aa, synthetic construct
  REGION 1..8: note = Description of Artificial Sequence: Synthetic peptide
  MOD_RES 1: note = beta-cyclohexylalanine
  MOD_RES 4: note = D-Phenylalanine
  MOD_RES 7: note = 4-aminobutyric acid
XDHFRWXK

SEQ ID NO: 47 - protein, 8 aa, synthetic construct
  REGION 1..8: note = Description of Artificial Sequence: Synthetic peptide
  MOD_RES 4: note = D-Phenylalanine
  MOD_RES 7: note = 4-aminobutyric acid
FDHFRWXK

SEQ ID NO: 48 - protein, 8 aa, synthetic construct
  REGION 1..8: note = Description of Artificial Sequence: Synthetic peptide
  MOD_RES 1: note = Beta-homomethionine
  MOD_RES 4: note = D-Phenylalanine
  MOD_RES 7: note = 4-aminobutyric acid
MDHFRWXK

SEQ ID NO: 49 - protein, 8 aa, synthetic construct
  REGION 1..8: note = Description of Artificial Sequence: Synthetic peptide
  MOD_RES 1: note = 4-aminobutyric acid
  MOD_RES 4: note = D-Phenylalanine
  MOD_RES 7: note = 4-aminobutyric acid
XDHFRWXK

SEQ ID NO: 50 - protein, 8 aa, synthetic construct
  REGION 1..8: note = Description of Artificial Sequence: Synthetic peptide
  MOD_RES 1: note = beta-cyclohexylalanine
  MOD_RES 4: note = D-Phenylalanine
  MOD_RES 6: note = D-Tryptophan
XDHFRWAK

SEQ ID NO: 51 - protein, 8 aa, synthetic construct
  REGION 1..8: note = Description of Artificial Sequence: Synthetic peptide
  MOD_RES 1: note = homo-cyclohexylalanine
  MOD_RES 4: note = D-Phenylalanine
  MOD_RES 6: note = D-Tryptophan
XDHFRWAK

SEQ ID NO: 52 - protein, 8 aa, synthetic construct
  REGION 1..8: note = Description of Artificial Sequence: Synthetic peptide
  MOD_RES 4: note = D-Phenylalanine
  MOD_RES 6: note = D-Tryptophan
LDHFRWAK

SEQ ID NO: 53 - protein, 8 aa, synthetic construct
  REGION 1..8: note = Description of Artificial Sequence: Synthetic peptide
  MOD_RES 4: note = D-Phenylalanine
  MOD_RES 6: note = D-Tryptophan
LDHFRWAK

SEQ ID NO: 54 - protein, 8 aa, synthetic construct
  REGION 1..8: note = Description of Artificial Sequence: Synthetic peptide
  MOD_RES 4: note = D-Phenylalanine
  MOD_RES 6: note = D-Tryptophan
FDHFRWAK

SEQ ID NO: 55 - protein, 8 aa, synthetic construct
  REGION 1..8: note = Description of Artificial Sequence: Synthetic peptide
  MOD_RES 1: note = Nle
  MOD_RES 4: note = D-Phenylalanine
  MOD_RES 6: note = D-Tryptophan
  MOD_RES 7: note = D-Alanine
XDHFRWAK

SEQ ID NO: 56 - protein, 8 aa, synthetic construct
  REGION 1..8: note = Description of Artificial Sequence: Synthetic peptide
  MOD_RES 1: note = Nle
  MOD_RES 4: note = D-Phenylalanine
  MOD_RES 6: note = D-Tryptophan
  MOD_RES 7: note = Beta-Alanine
XDHFRWAK

SEQ ID NO: 57 - protein, 8 aa, synthetic construct
  REGION 1..8: note = Description of Artificial Sequence: Synthetic peptide
  MOD_RES 1: note = Nle
  MOD_RES 4: note = D-Phenylalanine
  MOD_RES 6: note = D-Tryptophan
  MOD_RES 7: note = 4-aminobutyric acid
XDHFRWXK

SEQ ID NO: 58 - protein, 8 aa, synthetic construct
  REGION 1..8: note = Description of Artificial Sequence: Synthetic peptide
  MOD_RES 1: note = Nle
  MOD_RES 4: note = D-Phenylalanine
  MOD_RES 6: note = D-Tryptophan
  MOD_RES 7: note = 7-aminoheptanoic acid
XDHFRWXK

SEQ ID NO: 59 - protein, 8 aa, synthetic construct
  REGION 1..8: note = Description of Artificial Sequence: Synthetic peptide
  MOD_RES 1: note = Nle
  MOD_RES 4: note = D-Phenylalanine
  MOD_RES 6: note = D-Tryptophan
  MOD_RES 7: note = 5-aminopentanoic acid (HN-(CH2)4-C(O)
XDHFRWXK

SEQ ID NO: 60 - protein, 8 aa, synthetic construct
  REGION 1..8: note = Description of Artificial Sequence: Synthetic peptide
  MOD_RES 1: note = Nle
  MOD_RES 4: note = D-Phenylalanine
  MOD_RES 6: note = D-Tryptophan
  MOD_RES 7: note = 5-aminopentanoic acid (HN-(CH2)4-C(O)
XCHFRWXC

SEQ ID NO: 61 - protein, 8 aa, synthetic construct
  REGION 1..8: note = Description of Artificial Sequence: Synthetic peptide
  MOD_RES 1: note = Nle
  MOD_RES 4: note = D-Phenylalanine
  MOD_RES 6: note = D-Tryptophan
  MOD_RES 7: note = 4-aminobutyric acid
XCHFRWXC

SEQ ID NO: 62 - protein, 8 aa, synthetic construct
  REGION 1..8: note = Description of Artificial Sequence: Synthetic peptide
  MOD_RES 1: note = Nle
  MOD_RES 4: note = D-Phenylalanine
  MOD_RES 6: note = D-Tryptophan
  MOD_RES 7: note = 6-aminohexanoic acid
XCHFRWXC

SEQ ID NO: 63 - protein, 8 aa, synthetic construct
  REGION 1..8: note = Description of Artificial Sequence: Synthetic peptide
  MOD_RES 1: note = Nle
  MOD_RES 4: note = D-Phenylalanine
  MOD_RES 6: note = D-Tryptophan
  MOD_RES 7: note = Beta-Alanine
XCHFRWAC

SEQ ID NO: 64 - protein, 8 aa, synthetic construct
  REGION 1..8: note = Description of Artificial Sequence: Synthetic peptide
  MOD_RES 1: note = Nle
  MOD_RES 4: note = D-Phenylalanine
  MOD_RES 6: note = D-Tryptophan
  MOD_RES 7: note = D-Alanine
XCHFRWAC

SEQ ID NO: 65 - protein, 8 aa, synthetic construct
  REGION 1..8: note = Description of Artificial Sequence: Synthetic peptide
  MOD_RES 1: note = Nle
  MOD_RES 3: note = D-Alanine
  MOD_RES 5: note = D-Beta-(2-naphthyl)alanine
XCAHXRWC

SEQ ID NO: 66 - protein, 8 aa, synthetic construct
  REGION 1..8: note = Description of Artificial Sequence: Synthetic peptide
  MOD_RES 1: note = Nle
  MOD_RES 3: note = D-Alanine
  MOD_RES 5: note = D-Beta-(2-naphthyl)alanine
  MOD_RES 7: note = Beta-(2-naphthyl)alanine
XCAHXRXC

SEQ ID NO: 67 - protein, 8 aa, synthetic construct
  REGION 1..8: note = Description of Artificial Sequence: Synthetic peptide
  MOD_RES 1: note = Nle
  MOD_RES 3: note = D-Alanine
  MOD_RES 5: note = D-Beta-(2-naphthyl)alanine
  MOD_RES 7: note = Beta-(1-naphthyl)alanine
XCAHXRXC

SEQ ID NO: 68 - protein, 8 aa, synthetic construct
  REGION 1..8: note = Description of Artificial Sequence: Synthetic peptide
  MOD_RES 1: note = Nle
  MOD_RES 3: note = D-Alanine
  MOD_RES 5: note = D-Phenylalanine
  MOD_RES 7: note = Beta-(2-naphthyl)alanine
XCAHFRXC

SEQ ID NO: 69 - protein, 8 aa, synthetic construct
  REGION 1..8: note = Description of Artificial Sequence: Synthetic peptide
  MOD_RES 1: note = Nle
  MOD_RES 3: note = D-Alanine
  MOD_RES 5: note = D-Phenylalanine
XCAHFRWC

SEQ ID NO: 70 - protein, 8 aa, synthetic construct
  REGION 1..8: note = Description of Artificial Sequence: Synthetic peptide
  MOD_RES 1: note = Nle
  MOD_RES 3: note = D-Alanine
  MOD_RES 5: note = D-Phenylalanine
  MOD_RES 7: note = Beta-(2-naphthyl)alanine
XCAHFRXC

SEQ ID NO: 71 - protein, 8 aa, synthetic construct
  REGION 1..8: note = Description of Artificial Sequence: Synthetic peptide
  MOD_RES 1: note = Nle
  MOD_RES 3: note = D-Alanine
  MOD_RES 5: note = D-Phenylalanine
  MOD_RES 7: note = Beta-(1-naphthyl)alanine
XCAHFRXC

SEQ ID NO: 72 - protein, 8 aa, synthetic construct
  REGION 1..8: note = Description of Artificial Sequence: Synthetic peptide
  MOD_RES 1: note = Nle
  MOD_RES 3: note = D-Alanine
  MOD_RES 5: note = D-Phenylalanine
  MOD_RES 7: note = 3-benzothienylalanine
XCAHFRXC

SEQ ID NO: 73 - protein, 8 aa, synthetic construct
  REGION 1..8: note = Description of Artificial Sequence: Synthetic peptide
  MOD_RES 1: note = Nle
  MOD_RES 3: note = D-glutamic acid
  MOD_RES 5: note = D-Phenylalanine
XCEHFRWC

SEQ ID NO: 74 - protein, 8 aa, synthetic construct
  REGION 1..8: note = Description of Artificial Sequence: Synthetic peptide
  MOD_RES 1: note = Nle
  MOD_RES 4: note = D-Phenylalanine
  MOD_RES 7: note = D-Alanine
XDHFRWAK

SEQ ID NO: 75 - protein, 8 aa, synthetic construct
  REGION 1..8: note = Description of Artificial Sequence: Synthetic peptide
  MOD_RES 1: note = Nle
  MOD_RES 3: note = D-Alanine
  MOD_RES 5: note = D-Beta-(2-naphthyl)alanine
  MOD_RES 7: note = 3-benzothienylalanine
XCAHXRXC

SEQ ID NO: 76 - protein, 8 aa, synthetic construct
  REGION 1..8: note = Description of Artificial Sequence: Synthetic peptide
  MOD_RES 1: note = Nle
  MOD_RES 2: note = Penicillamine
  MOD_RES 3: note = D-Alanine
  MOD_RES 5: note = D-Phenylalanine
XXAHFRWC

SEQ ID NO: 77 - protein, 8 aa, synthetic construct
  REGION 1..8: note = Description of Artificial Sequence: Synthetic peptide
  MOD_RES 1: note = Nle
  MOD_RES 3: note = D-Alanine
  MOD_RES 5: note = D-Phenylalanine
  MOD_RES 8: note = Penicillamine
XCAHFRWX

SEQ ID NO: 78 - protein, 8 aa, synthetic construct
  REGION 1..8: note = Description of Artificial Sequence: Synthetic peptide
  MOD_RES 1: note = Nle
  MOD_RES 2: note = Penicillamine
  MOD_RES 3: note = D-Alanine
  MOD_RES 5: note = D-Phenylalanine
  MOD_RES 8: note = Penicillamine
XXAHFRWX

SEQ ID NO: 79 - protein, 9 aa, synthetic construct
  REGION 1..9: note = Description of Artificial Sequence: Synthetic peptide
  MOD_RES 1: note = D-Phenylalanine
  MOD_RES 4: note = D-Phenylalanine
  MOD_RES 7: note = Beta-Alanine
  MOD_RES 8: note = D-Cysteine
FCHFRWACT

SEQ ID NO: 80 - protein, 9 aa, synthetic construct
  REGION 1..9: note = Description of Artificial Sequence: Synthetic peptide
  MOD_RES 1: note = D-Phenylalanine
  MOD_RES 4: note = O-Ethyl-D-Tyrosine
  MOD_RES 7: note = Beta-Alanine
  MOD_RES 8: note = D-Cysteine
FCHYRWACT

SEQ ID NO: 81 - protein, 9 aa, synthetic construct
  REGION 1..9: note = Description of Artificial Sequence: Synthetic peptide
  MOD_RES 1: note = D-Phenylalanine
  MOD_RES 4: note = D-Phenylalanine
  MOD_RES 6: note = 4,4 -biphenylalanine
  MOD_RES 7: note = Beta-Alanine
  MOD_RES 8: note = D-Cysteine
FCHFRXACT

SEQ ID NO: 82 - protein, 9 aa, synthetic construct
  REGION 1..9: note = Description of Artificial Sequence: Synthetic peptide
  MOD_RES 1: note = D-Phenylalanine
  MOD_RES 4: note = O-Ethyl-D-Tyrosine
  MOD_RES 7: note = Beta-Alanine
  MOD_RES 8: note = D-Cysteine
FCHYRWACT

SEQ ID NO: 83 - protein, 9 aa, synthetic construct
  REGION 1..9: note = Description of Artificial Sequence: Synthetic peptide
  MOD_RES 1: note = D-Phenylalanine
  MOD_RES 4: note = D-Phenylalanine
  MOD_RES 6: note = 4,4 -biphenylalanine
  MOD_RES 7: note = Beta-Alanine
  MOD_RES 8: note = D-Cysteine
FCHFRXACT

SEQ ID NO: 84 - protein, 9 aa, synthetic construct
  REGION 1..9: note = Description of Artificial Sequence: Synthetic peptide
  MOD_RES 1: note = D-Phenylalanine
  MOD_RES 4: note = O-Ethyl-D-Tyrosine
  MOD_RES 6: note = 4,4 -biphenylalanine
  MOD_RES 7: note = Beta-Alanine
  MOD_RES 8: note = D-Cysteine
FCHYRXACT

SEQ ID NO: 85 - protein, 8 aa, synthetic construct
  REGION 1..8: note = Description of Artificial Sequence: Synthetic peptide
  MOD_RES 1: note = Nle
  MOD_RES 4: note = D-Phenylalanine
  MOD_RES 7: note = 5-aminopentanoic acid (HN-(CH2)4-C(O)
XCHFRWXC

SEQ ID NO: 86 - protein, 8 aa, synthetic construct
  REGION 1..8: note = Description of Artificial Sequence: Synthetic peptide
  MOD_RES 1: note = Nle
  MOD_RES 3: note = D-Alanine
  MOD_RES 5: note = D-Phenylalanine
XDAHFRWK

SEQ ID NO: 87 - protein, 8 aa, synthetic construct
  REGION 1..8: note = Description of Artificial Sequence: Synthetic peptide
  MOD_RES 1: note = Nle
  MOD_RES 3: note = D-Alanine
  MOD_RES 5: note = D-Phenylalanine
  MOD_RES 7: note = 3-benzothienylalanine
XDAHFRXK

SEQ ID NO: 88 - protein, 8 aa, synthetic construct
  REGION 1..8: note = Description of Artificial Sequence: Synthetic peptide
  MOD_RES 1: note = Nle
  MOD_RES 3: note = D-Alanine
  MOD_RES 5: note = D-Phenylalanine
  MOD_RES 8: note = Penicillamine
XCAHFRWX

SEQ ID NO: 89 - protein, 8 aa, synthetic construct
  REGION 1..8: note = Description of Artificial Sequence: Synthetic peptide
  MOD_RES 1: note = Nle
  MOD_RES 3: note = D-alpha-aminobutyric acid
  MOD_RES 5: note = D-Phenylalanine
XCXHFRWC

SEQ ID NO: 90 - protein, 8 aa, synthetic construct
  REGION 1..8: note = Description of Artificial Sequence: Synthetic peptide
  MOD_RES 1: note = Nle
  MOD_RES 3: note = D-valine
  MOD_RES 5: note = D-Phenylalanine
XCVHFRWC

SEQ ID NO: 91 - protein, 8 aa, synthetic construct
  REGION 1..8: note = Description of Artificial Sequence: Synthetic peptide
  MOD_RES 1: note = Nle
  MOD_RES 3: note = D-Isoleucine
  MOD_RES 5: note = D-Phenylalanine
XCIHFRWC

SEQ ID NO: 92 - protein, 8 aa, synthetic construct
  REGION 1..8: note = Description of Artificial Sequence: Synthetic peptide
  MOD_RES 1: note = Nle
  MOD_RES 3: note = D-Leucine
  MOD_RES 5: note = D-Phenylalanine
XCLHFRWC

SEQ ID NO: 93 - protein, 8 aa, synthetic construct
  REGION 1..8: note = Description of Artificial Sequence: Synthetic peptide
  MOD_RES 1: note = Nle
  MOD_RES 3: note = D-Tle
  MOD_RES 5: note = D-Phenylalanine
XCXHFRWC

SEQ ID NO: 94 - protein, 8 aa, synthetic construct
  REGION 1..8: note = Description of Artificial Sequence: Synthetic peptide
  MOD_RES 1: note = Nle
  MOD_RES 3: note = D-beta-cyclohexylalanine
  MOD_RES 5: note = D-Phenylalanine
XCXHFRWC

SEQ ID NO: 95 - protein, 8 aa, synthetic construct
  REGION 1..8: note = Description of Artificial Sequence: Synthetic peptide
  MOD_RES 1: note = Nle
  MOD_RES 2: note = Penicillamine
  MOD_RES 4: note = D-Phenylalanine
  MOD_RES 7: note = 4-aminobutyric acid
XXHFRWXC

SEQ ID NO: 96 - protein, 8 aa, synthetic construct
  REGION 1..8: note = Description of Artificial Sequence: Synthetic peptide
  MOD_RES 1: note = Nle
  MOD_RES 4: note = D-Phenylalanine
  MOD_RES 7: note = 4-aminobutyric acid
  MOD_RES 8: note = Penicillamine
XCHFRWXX

SEQ ID NO: 97 - protein, 8 aa, synthetic construct
  REGION 1..8: note = Description of Artificial Sequence: Synthetic peptide
  MOD_RES 1: note = Nle
  MOD_RES 2: note = Penicillamine
  MOD_RES 4: note = D-Phenylalanine
  MOD_RES 7: note = 4-aminobutyric acid
  MOD_RES 8: note = Penicillamine
XXHFRWXX

SEQ ID NO: 98 - protein, 8 aa, synthetic construct
  REGION 1..8: note = Description of Artificial Sequence: Synthetic peptide
  MOD_RES 4: note = D-Phenylalanine
  MOD_RES 7: note = 4-aminobutyric acid
LCHFRWXC

SEQ ID NO: 99 - protein, 8 aa, synthetic construct
  REGION 1..8: note = Description of Artificial Sequence: Synthetic peptide
  MOD_RES 1: note = beta-cyclohexylalanine
  MOD_RES 4: note = D-Phenylalanine
  MOD_RES 7: note = 4-aminobutyric acid
XCHFRWXC

SEQ ID NO: 100 - protein, 8 aa, synthetic construct
  REGION 1..8: note = Description of Artificial Sequence: Synthetic peptide
  MOD_RES 4: note = D-Phenylalanine
  MOD_RES 7: note = 4-aminobutyric acid
ICHFRWXC

SEQ ID NO: 101 - protein, 8 aa, synthetic construct
  REGION 1..8: note = Description of Artificial Sequence: Synthetic peptide
  MOD_RES 4: note = D-Phenylalanine
  MOD_RES 7: note = 4-aminobutyric acid
FCHFRWXC

SEQ ID NO: 102 - protein, 8 aa, synthetic construct
  REGION 1..8: note = Description of Artificial Sequence: Synthetic peptide
  MOD_RES 4: note = D-Phenylalanine
  MOD_RES 7: note = 4-aminobutyric acid
VCHFRWXC

SEQ ID NO: 103 - protein, 8 aa, synthetic construct
  REGION 1..8: note = Description of Artificial Sequence: Synthetic peptide
  MOD_RES 1: note = Beta-(2-naphthyl)alanine
  MOD_RES 4: note = D-Phenylalanine
  MOD_RES 7: note = 4-aminobutyric acid
XCHFRWXC

SEQ ID NO: 104 - protein, 8 aa, synthetic construct
  REGION 1..8: note = Description of Artificial Sequence: Synthetic peptide
  MOD_RES 1: note = Nle
  MOD_RES 4: note = D-Phenylalanine
  MOD_RES 7: note = 4-aminobutyric acid
XCHFRWXC

SEQ ID NO: 105 - protein, 8 aa, synthetic construct
  REGION 1..8: note = Description of Artificial Sequence: Synthetic peptide
  MOD_RES 4: note = D-Phenylalanine
  MOD_RES 7: note = 4-aminobutyric acid
FCHFRWXC

SEQ ID NO: 106 - protein, 8 aa, synthetic construct
  REGION 1..8: note = Description of Artificial Sequence: Synthetic peptide
  MOD_RES 1: note = Nle
  MOD_RES 3: note = beta-(3-pyridiyl)alanine
  MOD_RES 4: note = D-Phenylalanine
  MOD_RES 7: note = 4-aminobutyric acid
XCXFRWXC

SEQ ID NO: 107 - protein, 8 aa, synthetic construct
  REGION 1..8: note = Description of Artificial Sequence: Synthetic peptide
  MOD_RES 1: note = Nle
  MOD_RES 3: note = D-Alanine
  MOD_RES 5: note = D-Phenylalanine
XCAHFRWC

SEQ ID NO: 108 - protein, 8 aa, synthetic construct
  REGION 1..8: note = Description of Artificial Sequence: Synthetic peptide
  MOD_RES 1: note = Nle
  MOD_RES 6: note = D-Tryptophan
  MOD_RES 7: note = 4-aminobutyric acid
XCHFRWXC

SEQ ID NO: 109 - protein, 8 aa, synthetic construct
  REGION 1..8: note = Description of Artificial Sequence: Synthetic peptide
  MOD_RES 1: note = Nle
  MOD_RES 4: note = D-Beta-(2-naphthyl)alanine
XDHXRWAK

SEQ ID NO: 110 - protein, 8 aa, synthetic construct
  REGION 1..8: note = Description of Artificial Sequence: Synthetic peptide
  MOD_RES 1: note = Nle
  MOD_RES 4: note = D-Beta-(2-naphthyl)alanine
  MOD_RES 7: note = Beta-Alanine
XDHXRWAK

SEQ ID NO: 111 - protein, 8 aa, synthetic construct
  REGION 1..8: note = Description of Artificial Sequence: Synthetic peptide
  MOD_RES 1: note = Nle
  MOD_RES 4: note = D-Beta-(2-naphthyl)alanine
  MOD_RES 7: note = 4-aminobutyric acid
XCHXRWXC

SEQ ID NO: 112 - protein, 8 aa, synthetic construct
  REGION 1..8: note = Description of Artificial Sequence: Synthetic peptide
  MOD_RES 1: note = Nle
  MOD_RES 4: note = D-Beta-(2-naphthyl)alanine
  MOD_RES 7: note = 6-aminohexanoic acid
XCHXRWXC

SEQ ID NO: 113 - protein, 8 aa, synthetic construct
  REGION 1..8: note = Description of Artificial Sequence: Synthetic peptide
  MOD_RES 4: note = D-Beta-(2-naphthyl)alanine
  MOD_RES 7: note = 4-aminobutyric acid
FDHXRWXK

SEQ ID NO: 114 - protein, 8 aa, synthetic construct
  REGION 1..8: note = Description of Artificial Sequence: Synthetic peptide
  MOD_RES 1: note = beta-cyclohexylalanine
  MOD_RES 4: note = D-Beta-(2-naphthyl)alanine
  MOD_RES 7: note = 4-aminobutyric acid
XDHXRWXK

SEQ ID NO: 115 - protein, 8 aa, synthetic construct
  REGION 1..8: note = Description of Artificial Sequence: Synthetic peptide
  MOD_RES 1: note = Nle
  MOD_RES 4: note = D-Phenylalanine
  MOD_RES 7: note = Beta-Alanine
XDHFRWAK

SEQ ID NO: 116 - protein, 8 aa, synthetic construct
  REGION 1..8: note = Description of Artificial Sequence: Synthetic peptide
  MOD_RES 1: note = Nle
  MOD_RES 4: note = D-Phenylalanine
  MOD_RES 7: note = 6-aminohexanoic acid
XCHFRWXC

SEQ ID NO: 117 - protein, 9 aa, synthetic construct
  REGION 1..9: note = Description of Artificial Sequence: Synthetic peptide
  MOD_RES 1: note = D-Phenylalanine
  MOD_RES 4: note = D-Phenylalanine
  MOD_RES 8: note = D-Cysteine
FCHFRWACT

SEQ ID NO: 118 - protein, 9 aa, synthetic construct
  REGION 1..9: note = Description of Artificial Sequence: Synthetic peptide
  MOD_RES 1: note = D-Phenylalanine
  MOD_RES 4: note = D-Phenylalanine
  MOD_RES 7: note = Beta-Alanine
  MOD_RES 8: note = D-Cysteine
FCHFRWACT

SEQ ID NO: 119 - protein, 9 aa, synthetic construct
  REGION 1..9: note = Description of Artificial Sequence: Synthetic peptide
  MOD_RES 1: note = D-Phenylalanine
  MOD_RES 4: note = D-Phenylalanine
  MOD_RES 7: note = 4-aminobutyric acid
  MOD_RES 8: note = D-Cysteine
FCHFRWXCT

SEQ ID NO: 120 - protein, 8 aa, synthetic construct
  REGION 1..8: note = Description of Artificial Sequence: Synthetic peptide
  MOD_RES 1: note = Nle
  MOD_RES 4: note = D-Phenylalanine
  MOD_RES 7: note = 5-aminopentanoic acid (HN-(CH2)4-C(O)
XCHFRWXC

SEQ ID NO: 121 - protein, 8 aa, synthetic construct
  REGION 1..8: note = Description of Artificial Sequence: Synthetic peptide
  MOD_RES 1: note = Nle
  MOD_RES 4: note = D-Phenylalanine
  MOD_RES 7: note = 5-aminopentanoic acid (HN-(CH2)4-C(O)
XDHFRWXK

SEQ ID NO: 122 - protein, 8 aa, synthetic construct
  REGION 1..8: note = Description of Artificial Sequence: Synthetic peptide
  MOD_RES 1: note = beta-cyclohexylalanine
  MOD_RES 4: note = D-Phenylalanine
  MOD_RES 7: note = 4-aminobutyric acid
XDHFRWXK

SEQ ID NO: 123 - protein, 8 aa, synthetic construct
  REGION 1..8: note = Description of Artificial Sequence: Synthetic peptide
  MOD_RES 1: note = Nle
  MOD_RES 4: note = D-Phenylalanine
  MOD_RES 7: note = 4-aminobutyric acid
XDHFRWXK

SEQ ID NO: 124 - protein, 8 aa, synthetic construct
  REGION 1..8: note = Description of Artificial Sequence: Synthetic peptide
  MOD_RES 1: note = Cyclohexylglycine
  MOD_RES 4: note = D-Phenylalanine
  MOD_RES 7: note = 4-aminobutyric acid
XDHFRWXK

SEQ ID NO: 125 - protein, 8 aa, synthetic construct
  REGION 1..8: note = Description of Artificial Sequence: Synthetic peptide
  MOD_RES 1: note = D-beta-cyclohexylalanine
  MOD_RES 4: note = D-Phenylalanine
  MOD_RES 7: note = 4-aminobutyric acid
XDHFRWXK

SEQ ID NO: 126 - protein, 8 aa, synthetic construct
  REGION 1..8: note = Description of Artificial Sequence: Synthetic peptide
  MOD_RES 1: note = homo-cyclohexylalanine
  MOD_RES 4: note = D-Phenylalanine
  MOD_RES 7: note = 4-aminobutyric acid
XDHFRWXK

SEQ ID NO: 127 - protein, 8 aa, synthetic construct
  REGION 1..8: note = Description of Artificial Sequence: Synthetic peptide
  MOD_RES 1: note = D-Cyclohexylglycine
  MOD_RES 4: note = D-Phenylalanine
  MOD_RES 7: note = 4-aminobutyric acid
XDHFRWXK

SEQ ID NO: 128 - protein, 8 aa, synthetic construct
  REGION 1..8: note = Description of Artificial Sequence: Synthetic peptide
  MOD_RES 4: note = D-Phenylalanine
  MOD_RES 7: note = 4-aminobutyric acid
FDHFRWXK

SEQ ID NO: 129 - protein, 8 aa, synthetic construct
  REGION 1..8: note = Description of Artificial Sequence: Synthetic peptide
  MOD_RES 1: note = Nle
  MOD_RES 4: note = D-Phenylalanine
  MOD_RES 6: note = D-Tryptophan
  MOD_RES 7: note = 4-aminobutyric acid
XCHFRWXC

SEQ ID NO: 130 - protein, 8 aa, synthetic construct
  REGION 1..8: note = Description of Artificial Sequence: Synthetic peptide
  MOD_RES 1: note = Nle
  MOD_RES 4: note = D-Phenylalanine
  MOD_RES 6: note = D-Tryptophan
  MOD_RES 7: note = 6-aminohexanoic acid
XCHFRWXC

SEQ ID NO: 131 - protein, 8 aa, synthetic construct
  REGION 1..8: note = Description of Artificial Sequence: Synthetic peptide
  MOD_RES 1: note = Nle
  MOD_RES 4: note = D-Phenylalanine
  MOD_RES 6: note = D-Tryptophan
  MOD_RES 7: note = Beta-Alanine
XCHFRWAC

SEQ ID NO: 132 - protein, 8 aa, synthetic construct
  REGION 1..8: note = Description of Artificial Sequence: Synthetic peptide
  MOD_RES 1: note = Nle
  MOD_RES 4: note = D-Phenylalanine
  MOD_RES 6: note = D-Tryptophan
  MOD_RES 7: note = D-Alanine
XCHFRWAC

SEQ ID NO: 133 - protein, 8 aa, synthetic construct
  REGION 1..8: note = Description of Artificial Sequence: Synthetic peptide
  MOD_RES 1: note = Nle
  MOD_RES 3: note = D-Alanine
  MOD_RES 5: note = D-Beta-(2-naphthyl)alanine
XCAHXRWC

SEQ ID NO: 134 - protein, 8 aa, synthetic construct
  REGION 1..8: note = Description of Artificial Sequence: Synthetic peptide
  MOD_RES 1: note = Nle
  MOD_RES 3: note = D-Alanine
  MOD_RES 5: note = D-Beta-(2-naphthyl)alanine
  MOD_RES 7: note = Beta-(2-naphthyl)alanine
XCAHXRXC

SEQ ID NO: 135 - protein, 8 aa, synthetic construct
  REGION 1..8: note = Description of Artificial Sequence: Synthetic peptide
  MOD_RES 1: note = Nle
  MOD_RES 3: note = D-Alanine
  MOD_RES 5: note = D-Beta-(2-naphthyl)alanine
  MOD_RES 7: note = Beta-(1-naphthyl)alanine
XCAHXRXC

SEQ ID NO: 136 - protein, 8 aa, synthetic construct
  REGION 1..8: note = Description of Artificial Sequence: Synthetic peptide
  MOD_RES 1: note = Nle
  MOD_RES 3: note = D-Alanine
  MOD_RES 5: note = D-Beta-(2-naphthyl)alanine
  MOD_RES 7: note = 3-benzothienylalanine
XCAHXRXC

SEQ ID NO: 137 - protein, 8 aa, synthetic construct
  REGION 1..8: note = Description of Artificial Sequence: Synthetic peptide
  MOD_RES 1: note = Nle
  MOD_RES 2: note = Penicillamine
  MOD_RES 3: note = D-Alanine
  MOD_RES 5: note = D-Phenylalanine
XXAHFRWC

SEQ ID NO: 138 - protein, 8 aa, synthetic construct
  REGION 1..8: note = Description of Artificial Sequence: Synthetic peptide
  MOD_RES 1: note = Nle
  MOD_RES 4: note = D-Phenylalanine
  MOD_RES 7: note = 4-aminobutyric acid
  MOD_RES 8: note = Penicillamine
XCHFRWXX

SEQ ID NO: 139 - protein, 8 aa, synthetic construct
  REGION 1..8: note = Description of Artificial Sequence: Synthetic peptide
  MOD_RES 3: note = D-Alanine
  MOD_RES 5: note = D-Beta-(2-naphthyl)alanine
RCAHXRWC

SEQ ID NO: 140 - protein, 8 aa, synthetic construct
  REGION 1..8: note = Description of Artificial Sequence: Synthetic peptide
  MOD_RES 3: note = D-Alanine
  MOD_RES 5: note = D-Phenylalanine
RCAHFRWC

SEQ ID NO: 141 - protein, 8 aa, synthetic construct
  REGION 1..8: note = Description of Artificial Sequence: Synthetic peptide
  MOD_RES 1: note = D-Arginine
  MOD_RES 3: note = D-Alanine
  MOD_RES 5: note = D-Phenylalanine
RCAHFRWC

SEQ ID NO: 142 - protein, 8 aa, synthetic construct
  REGION 1..8: note = Description of Artificial Sequence: Synthetic peptide
  MOD_RES 1: note = D-Arginine
  MOD_RES 3: note = D-Alanine
  MOD_RES 5: note = D-Phenylalanine
  MOD_RES 8: note = Penicillamine
RCAHFRWX

SEQ ID NO: 143 - protein, 8 aa, synthetic construct
  REGION 1..8: note = Description of Artificial Sequence: Synthetic peptide
  MOD_RES 1: note = D-Arginine
  MOD_RES 4: note = D-Phenylalanine
  MOD_RES 7: note = 4-aminobutyric acid
  MOD_RES 8: note = Penicillamine
RCHFRWXX

SEQ ID NO: 144 - protein, 8 aa, synthetic construct
  REGION 1..8: note = Description of Artificial Sequence: Synthetic peptide
  MOD_RES 4: note = D-Phenylalanine
  MOD_RES 7: note = 4-aminobutyric acid
  MOD_RES 8: note = Penicillamine
RCHFRWXX

SEQ ID NO: 145 - protein, 8 aa, synthetic construct
  REGION 1..8: note = Description of Artificial Sequence: Synthetic peptide
  MOD_RES 3: note = D-Alanine
  MOD_RES 5: note = D-Phenylalanine
  MOD_RES 8: note = Penicillamine
RCAHFRWX

SEQ ID NO: 146 - protein, 8 aa, synthetic construct
  REGION 1..8: note = Description of Artificial Sequence: Synthetic peptide
  MOD_RES 1: note = D-Arginine
  MOD_RES 4: note = D-Phenylalanine
RDHFRWAK

SEQ ID NO: 147 - protein, 8 aa, synthetic construct
  REGION 1..8: note = Description of Artificial Sequence: Synthetic peptide
  MOD_RES 4: note = D-Phenylalanine
RDHFRWAK

SEQ ID NO: 148 - protein, 9 aa, synthetic construct
  REGION 1..9: note = Description of Artificial Sequence: Synthetic peptide
  MOD_RES 1: note = Nle
  MOD_RES 3: note = D-Alanine
  MOD_RES 5: note = D-Phenylalanine
XCAHFRWGC

SEQ ID NO: 149 - protein, 9 aa, synthetic construct
  REGION 1..9: note = Description of Artificial Sequence: Synthetic peptide
  MOD_RES 1: note = Nle
  MOD_RES 3: note = D-Alanine
  MOD_RES 5: note = D-Phenylalanine
  MOD_RES 8: note = D-Alanine
XCAHFRWAC

SEQ ID NO: 150 - protein, 9 aa, synthetic construct
  REGION 1..9: note = Description of Artificial Sequence: Synthetic peptide
  MOD_RES 1: note = Nle
  MOD_RES 3: note = D-Alanine
  MOD_RES 5: note = D-Phenylalanine
  MOD_RES 8: note = Beta-Alanine
XCAHFRWAC

SEQ ID NO: 151 - protein, 9 aa, synthetic construct
  REGION 1..9: note = Description of Artificial Sequence: Synthetic peptide
  MOD_RES 1: note = Nle
  MOD_RES 3: note = D-Alanine
  MOD_RES 5: note = D-Phenylalanine
  MOD_RES 8: note = 4-aminobutyric acid
XCAHFRWXC

SEQ ID NO: 152 - protein, 9 aa, synthetic construct
  REGION 1..9: note = Description of Artificial Sequence: Synthetic peptide
  MOD_RES 1: note = Nle
  MOD_RES 3: note = D-Alanine
  MOD_RES 5: note = D-Phenylalanine
  MOD_RES 8: note = 5-aminopentanoic acid (HN-(CH2)4-C(O)
XCAHFRWXC

SEQ ID NO: 153 - protein, 8 aa, synthetic construct
  REGION 1..8: note = Description of Artificial Sequence: Synthetic peptide
  MOD_RES 4: note = D-Phenylalanine
CEHFRWAC

SEQ ID NO: 154 - protein, 8 aa, synthetic construct
  REGION 1..8: note = Description of Artificial Sequence: Synthetic peptide
  MOD_RES 4: note = D-Phenylalanine
  MOD_RES 6: note = Beta-(2-naphthyl)alanine
CEHFRXAC

SEQ ID NO: 155 - protein, 8 aa, synthetic construct
  REGION 1..8: note = Description of Artificial Sequence: Synthetic peptide
  MOD_RES 2: note = D-Alanine
  MOD_RES 4: note = D-Phenylalanine
CAHFRWAC

SEQ ID NO: 156 - protein, 8 aa, synthetic construct
  REGION 1..8: note = Description of Artificial Sequence: Synthetic peptide
  MOD_RES 2: note = D-Alanine
  MOD_RES 4: note = D-Phenylalanine
  MOD_RES 6: note = Beta-(2-naphthyl)alanine
CAHFRXAC

SEQ ID NO: 157 - protein, 9 aa, synthetic construct
  REGION 1..9: note = Description of Artificial Sequence: Synthetic peptide
  MOD_RES 1: note = Nle
  MOD_RES 3: note = D-Alanine
  MOD_RES 5: note = D-Phenylalanine
XCAHFRWAC

SEQ ID NO: 158 - protein, 9 aa, synthetic construct
  REGION 1..9: note = Description of Artificial Sequence: Synthetic peptide
  MOD_RES 1: note = Nle
  MOD_RES 3: note = D-Alanine
  MOD_RES 5: note = D-Phenylalanine
  MOD_RES 7: note = 3-benzothienylalanine
XDAHFRXAK

SEQ ID NO: 159 - protein, 18 aa, synthetic construct
  REGION 1..18: note = Description of Artificial Sequence: Synthetic peptide
  MOD_RES 12: note = Nle
  MOD_RES 15: note = D-Beta-(2-naphthyl)alanine
YGRKKRRQRRRXDHXRWK

SEQ ID NO: 160 - protein, 19 aa, synthetic construct
  REGION 1..19: note = Description of Artificial Sequence: Synthetic peptide
  MOD_RES 12: note = 8-amino-3,6-dioxaoctanoic acid
  MOD_RES 13: note = Nle
  MOD_RES 16: note = D-Beta-(2-naphthyl)alanine
YGRKKRRQRRRXXDHXRWK

SEQ ID NO: 161 - protein, 19 aa, synthetic construct
  REGION 1..19: note = Description of Artificial Sequence: Synthetic peptide
  MOD_RES 1: note = Nle
  MOD_RES 4: note = D-Beta-(2-naphthyl)alanine
  MOD_RES 8: note = Beta-Alanine
XDHXRWKAYGRKKRRQRRR

SEQ ID NO: 162 - protein, 19 aa, synthetic construct
  REGION 1..19: note = Description of Artificial Sequence: Synthetic peptide
  MOD_RES 1: note = Nle
  MOD_RES 4: note = D-Beta-(2-naphthyl)alanine
  MOD_RES 8: note = Beta-Alanine
XDHXRWKAYGRKKRRQRRR

SEQ ID NO: 163 - protein, 20 aa, synthetic construct
  REGION 1..20: note = Description of Artificial Sequence: Synthetic peptide
  MOD_RES 1: note = Nle
  MOD_RES 4: note = D-Beta-(2-naphthyl)alanine
  MOD_RES 8: note = 8-amino-3,6-dioxaoctanoic acid
  MOD_RES 9: note = 8-amino-3,6-dioxaoctanoic acid
XDHXRWKXXYGRKKRRQRRR

SEQ ID NO: 164 - protein, 22 aa, synthetic construct
  REGION 1..22: note = Description of Artificial Sequence: Synthetic peptide
  MOD_RES 1: note = Nle
  MOD_RES 4: note = D-Beta-(2-naphthyl)alanine
XDHXRWKPPKDYGRKKRRQRRR

SEQ ID NO: 165 - protein, 23 aa, synthetic construct
  REGION 1..23: note = Description of Artificial Sequence: Synthetic peptide
  MOD_RES 4: note = D-Beta-(2-naphthyl)alanine
CEHXRWGCPPKDYGRKKRRQRRR

SEQ ID NO: 166 - protein, 20 aa, synthetic construct
  REGION 1..20: note = Description of Artificial Sequence: Synthetic peptide
  MOD_RES 1: note = Nle
  MOD_RES 4: note = D-Beta-(2-naphthyl)alanine
  MOD_RES 8: note = Beta-Alanine
  MOD_RES 9: note = Beta-Alanine
XDHXRWKAAYGRKKRRQRRR

SEQ ID NO: 167 - protein, 23 aa, synthetic construct
  REGION 1..23: note = Description of Artificial Sequence: Synthetic peptide
  MOD_RES 1: note = Nle
  MOD_RES 4: note = D-Beta-(2-naphthyl)alanine
  MOD_RES 12: note = 8-amino-3,6-dioxaoctanoic acid
XDHXRWKPPKDXYGRKKRRQRRR

SEQ ID NO: 168 - protein, 24 aa, synthetic construct
  REGION 1..24: note = Description of Artificial Sequence: Synthetic peptide
  MOD_RES 4: note = D-Beta-(2-naphthyl)alanine
  MOD_RES 13: note = 8-amino-3,6-dioxaoctanoic acid
CEHXRWGCPPKDXYGRKKRRQRRR

SEQ ID NO: 169 - protein, 24 aa, synthetic construct
  REGION 1..24: note = Description of Artificial Sequence: Synthetic peptide
  MOD_RES 4: note = D-Beta-(2-naphthyl)alanine
  MOD_RES 13: note = Beta-Alanine
CEHXRWACPPKDAYGRKKRRQRRR

SEQ ID NO: 170 - protein, 24 aa, synthetic construct
  REGION 1..24: note = Description of Artificial Sequence: Synthetic peptide
  MOD_RES 4: note = D-Beta-(2-naphthyl)alanine
  MOD_RES 13: note = 8-amino-3,6-dioxaoctanoic acid
CEHXRWACPPKDXYGRKKRRQRRR

SEQ ID NO: 171 - protein, 20 aa, synthetic construct
  REGION 1..20: note = Description of Artificial Sequence: Synthetic peptide
  MOD_RES 1: note = Nle
  MOD_RES 4: note = D-Beta-(2-naphthyl)alanine
  MOD_RES 8: note = 8-amino-3,6-dioxaoctanoic acid
  MOD_RES 9: note = 8-amino-3,6-dioxaoctanoic acid
XDHXRWKXXYGRKKRRQRRR

SEQ ID NO: 172 - protein, 24 aa, synthetic construct
  REGION 1..24: note = Description of Artificial Sequence: Synthetic peptide
  MOD_RES 4: note = D-Beta-(2-naphthyl)alanine
  MOD_RES 6: note = Beta-(2-naphthyl)alanine
  MOD_RES 13: note = Beta-Alanine
CEHXRXACPPKDAYGRKKRRQRRR

SEQ ID NO: 173 - protein, 22 aa, synthetic construct
  REGION 1..22: note = Description of Artificial Sequence: Synthetic peptide
  MOD_RES 4: note = D-Beta-(2-naphthyl)alanine
  MOD_RES 6: note = 3-benzothienylalanine
  MOD_RES 13: note = Beta-Alanine
CEHXRXACPPKDARRRRRQRRR

SEQ ID NO: 174 - protein, 23 aa, synthetic construct
  REGION 1..23: note = Description of Artificial Sequence: Synthetic peptide
  MOD_RES 4: note = D-Beta-(2-naphthyl)alanine
  MOD_RES 6: note = 3-benzothienylalanine
  MOD_RES 13: note = Beta-Alanine
CEHXRXACPPKDAGRRRRRQRRR

SEQ ID NO: 175 - protein, 24 aa, synthetic construct
  REGION 1..24: note = Description of Artificial Sequence: Synthetic peptide
  MOD_RES 4: note = D-Beta-(2-naphthyl)alanine
  MOD_RES 6: note = 3-benzothienylalanine
  MOD_RES 13: note = Beta-Alanine
CEHXRXACPPKDAYGRRRRRQRRR

SEQ ID NO: 176 - protein, 24 aa, synthetic construct
  REGION 1..24: note = Description of Artificial Sequence: Synthetic peptide
  MOD_RES 4: note = D-Beta-(2-naphthyl)alanine
  MOD_RES 13: note = Beta-Alanine
CEHXRWACPPKDAYGRKKRQRRRR

SEQ ID NO: 177 - protein, 24 aa, synthetic construct
  REGION 1..24: note = Description of Artificial Sequence: Synthetic peptide
  MOD_RES 4: note = D-Beta-(2-naphthyl)alanine
  MOD_RES 13: note = Beta-Alanine
CEHXRWACPPKDAYGRKKQRRRRR

SEQ ID NO: 178 - protein, 24 aa, synthetic construct
  REGION 1..24: note = Description of Artificial Sequence: Synthetic peptide
  MOD_RES 4: note = D-Beta-(2-naphthyl)alanine
  MOD_RES 13: note = Beta-Alanine
CEHXRWACPPKDAYGRKQKRRRRR

SEQ ID NO: 179 - protein, 24 aa, synthetic construct
  REGION 1..24: note = Description of Artificial Sequence: Synthetic peptide
  MOD_RES 4: note = D-Beta-(2-naphthyl)alanine
  MOD_RES 13: note = Beta-Alanine
CEHXRWACPPKDAYGRKKRRRRQR

SEQ ID NO: 180 - protein, 24 aa, synthetic construct
  REGION 1..24: note = Description of Artificial Sequence: Synthetic peptide
  MOD_RES 4: note = D-Beta-(2-naphthyl)alanine
  MOD_RES 6: note = 3-benzothienylalanine
  MOD_RES 13: note = Beta-Alanine
  MOD_RES 15: note = alpha-aminoisobutyric acid
CEHXRXACPPKDAYXRKKRRQRRR

SEQ ID NO: 181 - protein, 22 aa, synthetic construct
  REGION 1..22: note = Description of Artificial Sequence: Synthetic peptide
  MOD_RES 4: note = D-Beta-(2-naphthyl)alanine
  MOD_RES 6: note = Beta-(1-naphthyl)alanine
  MOD_RES 13: note = Beta-Alanine
CEHXRXACPPRDARRRRRQRRR

SEQ ID NO: 182 - protein, 22 aa, synthetic construct
  REGION 1..22: note = Description of Artificial Sequence: Synthetic peptide
  MOD_RES 4: note = D-Beta-(2-naphthyl)alanine
  MOD_RES 6: note = Beta-(1-naphthyl)alanine
  MOD_RES 13: note = Beta-Alanine
CEHXRXACPPKDARRRRRQRRR

SEQ ID NO: 183 - protein, 23 aa, synthetic construct
  REGION 1..23: note = Description of Artificial Sequence: Synthetic peptide
  MOD_RES 4: note = D-Beta-(2-naphthyl)alanine
  MOD_RES 6: note = Beta-(1-naphthyl)alanine
  MOD_RES 13: note = Beta-Alanine
CEHXRXACPPKDARRRRRRQRRR

SEQ ID NO: 184 - protein, 22 aa, synthetic construct
  REGION 1..22: note = Description of Artificial Sequence: Synthetic peptide
  MOD_RES 4: note = D-Beta-(2-naphthyl)alanine
  MOD_RES 6: note = Beta-(2-naphthyl)alanine
  MOD_RES 13: note = Beta-Alanine
CEHXRXACPPRDARRRRRQRRR

SEQ ID NO: 185 - protein, 22 aa, synthetic construct
  REGION 1..22: note = Description of Artificial Sequence: Synthetic peptide
  MOD_RES 4: note = D-Beta-(2-naphthyl)alanine
  MOD_RES 6: note = Beta-(2-naphthyl)alanine
  MOD_RES 13: note = Beta-Alanine
CEHXRXACPPKDARRRRRQRRR

SEQ ID NO: 186 - protein, 23 aa, synthetic construct
  REGION 1..23: note = Description of Artificial Sequence: Synthetic peptide
  MOD_RES 4: note = D-Beta-(2-naphthyl)alanine
  MOD_RES 6: note = Beta-(2-naphthyl)alanine
  MOD_RES 13: note = Beta-Alanine
CEHXRXACPPKDARRRRRRQRRR

SEQ ID NO: 187 - protein, 23 aa, synthetic construct
  REGION 1..23: note = Description of Artificial Sequence: Synthetic peptide
  MOD_RES 4: note = D-Beta-(2-naphthyl)alanine
  MOD_RES 6: note = 3-benzothienylalanine
  MOD_RES 13: note = Beta-Alanine
CEHXRXACPPRDARRRRRRQRRR

SEQ ID NO: 188 - protein, 22 aa, synthetic construct
  REGION 1..22: note = Description of Artificial Sequence: Synthetic peptide
  MOD_RES 4: note = D-Beta-(2-naphthyl)alanine
  MOD_RES 6: note = 3-benzothienylalanine
  MOD_RES 13: note = Beta-Alanine
CEHXRXACPPRDARRRRRQRRR

SEQ ID NO: 189 - protein, 23 aa, synthetic construct
  REGION 1..23: note = Description of Artificial Sequence: Synthetic peptide
  MOD_RES 4: note = D-Beta-(2-naphthyl)alanine
  MOD_RES 6: note = 3-benzothienylalanine
  MOD_RES 13: note = Beta-Alanine
CEHXRXACPPKDARRRRRRQRRR

SEQ ID NO: 190 - protein, 24 aa, synthetic construct
  REGION 1..24: note = Description of Artificial Sequence: Synthetic peptide
  MOD_RES 4: note = D-Beta-(2-naphthyl)alanine
  MOD_RES 13: note = Beta-Alanine
CEHXRWACPPKDAYGRKKRRRQRR

SEQ ID NO: 191 - protein, 24 aa, synthetic construct
  REGION 1..24: note = Description of Artificial Sequence: Synthetic peptide
  MOD_RES 4: note = D-Beta-(2-naphthyl)alanine
  MOD_RES 13: note = Beta-Alanine
CEHXRWACPPKDAYGRQKKRRRRR

SEQ ID NO: 192 - protein, 24 aa, synthetic construct
  REGION 1..24: note = Description of Artificial Sequence: Synthetic peptide
  MOD_RES 4: note = D-Beta-(2-naphthyl)alanine
  MOD_RES 13: note = Beta-Alanine
CEHXRWACPPKDAYGRKKRRRRRQ

SEQ ID NO: 193 - protein, 24 aa, synthetic construct
  REGION 1..24: note = Description of Artificial Sequence: Synthetic peptide
  MOD_RES 4: note = D-Beta-(2-naphthyl)alanine
  MOD_RES 6: note = Beta-(1-naphthyl)alanine
  MOD_RES 13: note = Beta-Alanine
CEHXRXACPPKDAYGRKKRRQRRR

SEQ ID NO: 194 - protein, 24 aa, synthetic construct
  REGION 1..24: note = Description of Artificial Sequence: Synthetic peptide
  MOD_RES 4: note = D-Beta-(2-naphthyl)alanine
  MOD_RES 6: note = 3-benzothienylalanine
  MOD_RES 13: note = Beta-Alanine
CEHXRXACPPKDAYGRKKRRQRRR

SEQ ID NO: 195 - protein, 22 aa, synthetic construct
  REGION 1..22: note = Description of Artificial Sequence: Synthetic peptide
  MOD_RES 4: note = D-Beta-(2-naphthyl)alanine
  MOD_RES 6: note = Beta-(1-naphthyl)alanine
  MOD_RES 13: note = Beta-Alanine
CEHXRXACPPKDARRKRRQRRR

SEQ ID NO: 196 - protein, 22 aa, synthetic construct
  REGION 1..22: note = Description of Artificial Sequence: Synthetic peptide
  MOD_RES 4: note = D-Beta-(2-naphthyl)alanine
  MOD_RES 6: note = Beta-(1-naphthyl)alanine
  MOD_RES 13: note = Beta-Alanine
CEHXRXACPPKDARKRRRQRRR

SEQ ID NO: 197 - protein, 22 aa, synthetic construct
  REGION 1..22: note = Description of Artificial Sequence: Synthetic peptide
  MOD_RES 4: note = D-Beta-(2-naphthyl)alanine
  MOD_RES 6: note = Beta-(2-naphthyl)alanine
  MOD_RES 13: note = Beta-Alanine
CEHXRXACPPKDARRKRRQRRR

SEQ ID NO: 198 - protein, 24 aa, synthetic construct
  REGION 1..24: note = Description of Artificial Sequence: Synthetic peptide
  MOD_RES 4: note = D-Beta-(2-naphthyl)alanine
  MOD_RES 6: note = Beta-(2-naphthyl)alanine
  MOD_RES 13: note = Beta-Alanine
CEHXRXACPPKDAYGRRKRRQRRR

SEQ ID NO: 199 - protein, 23 aa, synthetic construct
  REGION 1..23: note = Description of Artificial Sequence: Synthetic peptide
  MOD_RES 4: note = D-Beta-(2-naphthyl)alanine
  MOD_RES 6: note = Beta-(2-naphthyl)alanine
  MOD_RES 13: note = Beta-Alanine
CEHXRXACPPKDAGRRKRRQRRR

SEQ ID NO: 200 - protein, 23 aa, synthetic construct
  REGION 1..23: note = Description of Artificial Sequence: Synthetic peptide
  MOD_RES 4: note = D-Beta-(2-naphthyl)alanine
  MOD_RES 6: note = Beta-(2-naphthyl)alanine
  MOD_RES 13: note = Beta-Alanine
CEHXRXACPPKDAGRKRRRQRRR

SEQ ID NO: 201 - protein, 24 aa, synthetic construct
  REGION 1..24: note = Description of Artificial Sequence: Synthetic peptide
  MOD_RES 4: note = D-Beta-(2-naphthyl)alanine
  MOD_RES 6: note = Beta-(1-naphthyl)alanine
  MOD_RES 13: note = Beta-Alanine
CEHXRXACPPKDAYGRRKRRQRRR

SEQ ID NO: 202 - protein, 24 aa, synthetic construct
  REGION 1..24: note = Description of Artificial Sequence: Synthetic peptide
  MOD_RES 4: note = D-Beta-(2-naphthyl)alanine
  MOD_RES 6: note = Beta-(1-naphthyl)alanine
  MOD_RES 13: note = Beta-Alanine
CEHXRXACPPKDAYGRKRRRQRRR

SEQ ID NO: 203 - protein, 23 aa, synthetic construct
  REGION 1..23: note = Description of Artificial Sequence: Synthetic peptide
  MOD_RES 4: note = D-Beta-(2-naphthyl)alanine
  MOD_RES 6: note = Beta-(1-naphthyl)alanine
  MOD_RES 13: note = Beta-Alanine
CEHXRXACPPKDAGRRKRRQRRR

SEQ ID NO: 204 - protein, 23 aa, synthetic construct
  REGION 1..23: note = Description of Artificial Sequence: Synthetic peptide
  MOD_RES 4: note = D-Beta-(2-naphthyl)alanine
  MOD_RES 6: note = Beta-(1-naphthyl)alanine
  MOD_RES 13: note = Beta-Alanine
CEHXRXACPPKDAGRKRRRQRRR

SEQ ID NO: 205 - protein, 22 aa, synthetic construct
  REGION 1..22: note = Description of Artificial Sequence: Synthetic peptide
  MOD_RES 4: note = D-Beta-(2-naphthyl)alanine
  MOD_RES 6: note = Beta-(2-naphthyl)alanine
  MOD_RES 13: note = Beta-Alanine
CEHXRXACPPKDARRKRRQRRR

SEQ ID NO: 206 - protein, 22 aa, synthetic construct
  REGION 1..22: note = Description of Artificial Sequence: Synthetic peptide
  MOD_RES 4: note = D-Beta-(2-naphthyl)alanine
  MOD_RES 6: note = Beta-(2-naphthyl)alanine
  MOD_RES 13: note = Beta-Alanine
CEHXRXACPPKDARKRRRQRRR

SEQ ID NO: 207 - protein, 24 aa, synthetic construct
  REGION 1..24: note = Description of Artificial Sequence: Synthetic peptide
  MOD_RES 4: note = D-Beta-(2-naphthyl)alanine
  MOD_RES 6: note = Beta-(2-naphthyl)alanine
  MOD_RES 13: note = Beta-Alanine
CEHXRXACPPKDAYGRKRRRQRRR

SEQ ID NO: 208 - protein, 22 aa, synthetic construct
  REGION 1..22: note = Description of Artificial Sequence: Synthetic peptide
  MOD_RES 4: note = D-Beta-(2-naphthyl)alanine
  MOD_RES 6: note = 3-benzothienylalanine
  MOD_RES 13: note = Beta-Alanine
CEHXRXACPPKDARRKRRQRRR

SEQ ID NO: 209 - protein, 22 aa, synthetic construct
  REGION 1..22: note = Description of Artificial Sequence: Synthetic peptide
  MOD_RES 4: note = D-Beta-(2-naphthyl)alanine
  MOD_RES 6: note = 3-benzothienylalanine
  MOD_RES 13: note = Beta-Alanine
CEHXRXACPPKDARKRRRQRRR

SEQ ID NO: 210 - protein, 24 aa, synthetic construct
  REGION 1..24: note = Description of Artificial Sequence: Synthetic peptide
  MOD_RES 4: note = D-Beta-(2-naphthyl)alanine
  MOD_RES 6: note = 3-benzothienylalanine
  MOD_RES 13: note = Beta-Alanine
CEHXRXACPPKDAYGRRKRRQRRR

SEQ ID NO: 211 - protein, 24 aa, synthetic construct
  REGION 1..24: note = Description of Artificial Sequence: Synthetic peptide
  MOD_RES 4: note = D-Beta-(2-naphthyl)alanine
  MOD_RES 6: note = 3-benzothienylalanine
  MOD_RES 13: note = Beta-Alanine
CEHXRXACPPKDAYGRKRRRQRRR

SEQ ID NO: 212 - protein, 23 aa, synthetic construct
  REGION 1..23: note = Description of Artificial Sequence: Synthetic peptide
  MOD_RES 4: note = D-Beta-(2-naphthyl)alanine
  MOD_RES 6: note = 3-benzothienylalanine
  MOD_RES 13: note = Beta-Alanine
CEHXRXACPPKDAGRRKRRQRRR

SEQ ID NO: 213 - protein, 23 aa, synthetic construct
  REGION 1..23: note = Description of Artificial Sequence: Synthetic peptide
  MOD_RES 4: note = D-Beta-(2-naphthyl)alanine
  MOD_RES 6: note = 3-benzothienylalanine
  MOD_RES 13: note = Beta-Alanine
CEHXRXACPPKDAGRKRRRQRRR

SEQ ID NO: 214 - protein, 22 aa, synthetic construct
  REGION 1..22: note = Description of Artificial Sequence: Synthetic peptide
  MOD_RES 4: note = D-Beta-(2-naphthyl)alanine
  MOD_RES 13: note = Beta-Alanine
CEHXRWACPPKDARRRRRQRRR

SEQ ID NO: 215 - protein, 22 aa, synthetic construct
  REGION 1..22: note = Description of Artificial Sequence: Synthetic peptide
  MOD_RES 4: note = D-Beta-(2-naphthyl)alanine
  MOD_RES 13: note = Beta-Alanine
CEHXRWACPPRDARRRRRQRRR

SEQ ID NO: 216 - protein, 24 aa, synthetic construct
  REGION 1..24: note = Description of Artificial Sequence: Synthetic peptide
  MOD_RES 4: note = D-Beta-(2-naphthyl)alanine
  MOD_RES 13: note = Beta-Alanine
CEHXRWACPPKDAYGRRRRRQRRR

SEQ ID NO: 217 - protein, 24 aa, synthetic construct
  REGION 1..24: note = Description of Artificial Sequence: Synthetic peptide
  MOD_RES 4: note = D-Beta-(2-naphthyl)alanine
  MOD_RES 13: note = Beta-Alanine
CEHXRWACPPRDAYGRRRRRQRRR

SEQ ID NO: 218 - protein, 23 aa, synthetic construct
  REGION 1..23: note = Description of Artificial Sequence: Synthetic peptide
  MOD_RES 4: note = D-Beta-(2-naphthyl)alanine
  MOD_RES 13: note = Beta-Alanine
CEHXRWACPPKDARRRRRQRRRR

SEQ ID NO: 219 - protein, 23 aa, synthetic construct
  REGION 1..23: note = Description of Artificial Sequence: Synthetic peptide
  MOD_RES 4: note = D-Beta-(2-naphthyl)alanine
  MOD_RES 13: note = Beta-Alanine
CEHXRWACPPRDARRRRRQRRRR

SEQ ID NO: 220 - protein, 25 aa, synthetic construct
  REGION 1..25: note = Description of Artificial Sequence: Synthetic peptide
  MOD_RES 4: note = D-Beta-(2-naphthyl)alanine
  MOD_RES 13: note = Beta-Alanine
CEHXRWACPPKDAYGRRRRRQRRRR

SEQ ID NO: 221 - protein, 25 aa, synthetic construct
  REGION 1..25: note = Description of Artificial Sequence: Synthetic peptide
  MOD_RES 4: note = D-Beta-(2-naphthyl)alanine
  MOD_RES 13: note = Beta-Alanine
CEHXRWACPPRDAYGRRRRRQRRRR

SEQ ID NO: 222 - protein, 23 aa, synthetic construct
  REGION 1..23: note = Description of Artificial Sequence: Synthetic peptide
  MOD_RES 4: note = D-Beta-(2-naphthyl)alanine
  MOD_RES 6: note = Beta-(1-naphthyl)alanine
  MOD_RES 13: note = Beta-Alanine
CEHXRXACPPKDARRRRRQRRRR

SEQ ID NO: 223 - protein, 23 aa, synthetic construct
  REGION 1..23: note = Description of Artificial Sequence: Synthetic peptide
  MOD_RES 4: note = D-Beta-(2-naphthyl)alanine
  MOD_RES 6: note = Beta-(1-naphthyl)alanine
  MOD_RES 13: note = Beta-Alanine
CEHXRXACPPRDARRRRRQRRRR

SEQ ID NO: 224 - protein, 23 aa, synthetic construct
  REGION 1..23: note = Description of Artificial Sequence: Synthetic peptide
  MOD_RES 4: note = D-Beta-(2-naphthyl)alanine
  MOD_RES 6: note = Beta-(1-naphthyl)alanine
  MOD_RES 13: note = Beta-Alanine
CEHXRXACPPRDARRRRRRQRRR

SEQ ID NO: 225 - protein, 24 aa, synthetic construct
  REGION 1..24: note = Description of Artificial Sequence: Synthetic peptide
  MOD_RES 4: note = D-Beta-(2-naphthyl)alanine
  MOD_RES 6: note = Beta-(1-naphthyl)alanine
  MOD_RES 13: note = Beta-Alanine
CEHXRXACPPKDAYGRRRRRQRRR

SEQ ID NO: 226 - protein, 24 aa, synthetic construct
  REGION 1..24: note = Description of Artificial Sequence: Synthetic peptide
  MOD_RES 4: note = D-Beta-(2-naphthyl)alanine
  MOD_RES 6: note = Beta-(1-naphthyl)alanine
  MOD_RES 13: note = Beta-Alanine
CEHXRXACPPRDAYGRRRRRQRRR

SEQ ID NO: 227 - protein, 25 aa, synthetic construct
  REGION 1..25: note = Description of Artificial Sequence: Synthetic peptide
  MOD_RES 4: note = D-Beta-(2-naphthyl)alanine
  MOD_RES 6: note = Beta-(1-naphthyl)alanine
  MOD_RES 13: note = Beta-Alanine
CEHXRXACPPKDAYGRRRRRQRRRR

SEQ ID NO: 228 - protein, 25 aa, synthetic construct
  REGION 1..25: note = Description of Artificial Sequence: Synthetic peptide
  MOD_RES 4: note = D-Beta-(2-naphthyl)alanine
  MOD_RES 6: note = Beta-(1-naphthyl)alanine
  MOD_RES 13: note = Beta-Alanine
CEHXRXACPPRDAYGRRRRRQRRRR

SEQ ID NO: 229 - protein, 25 aa, synthetic construct
  REGION 1..25: note = Description of Artificial Sequence: Synthetic peptide
  MOD_RES 4: note = D-Beta-(2-naphthyl)alanine
  MOD_RES 6: note = Beta-(1-naphthyl)alanine
  MOD_RES 13: note = Beta-Alanine
CEHXRXACPPKDAYGRRRRRRQRRR

SEQ ID NO: 230 - protein, 25 aa, synthetic construct
  REGION 1..25: note = Description of Artificial Sequence: Synthetic peptide
  MOD_RES 4: note = D-Beta-(2-naphthyl)alanine
  MOD_RES 6: note = Beta-(1-naphthyl)alanine
  MOD_RES 13: note = Beta-Alanine
CEHXRXACPPRDAYGRRRRRRQRRR

SEQ ID NO: 231 - protein, 23 aa, synthetic construct
  REGION 1..23: note = Description of Artificial Sequence: Synthetic peptide
  MOD_RES 4: note = D-Beta-(2-naphthyl)alanine
  MOD_RES 6: note = Beta-(2-naphthyl)alanine
  MOD_RES 13: note = Beta-Alanine
CEHXRXACPPRDARRRRRRQRRR

SEQ ID NO: 232 - protein, 23 aa, synthetic construct
  REGION 1..23: note = Description of Artificial Sequence: Synthetic peptide
  MOD_RES 4: note = D-Beta-(2-naphthyl)alanine
  MOD_RES 6: note = Beta-(2-naphthyl)alanine
  MOD_RES 13: note = Beta-Alanine
CEHXRXACPPKDARRRRRQRRRR

SEQ ID NO: 233 - protein, 23 aa, synthetic construct
  REGION 1..23: note = Description of Artificial Sequence: Synthetic peptide
  MOD_RES 4: note = D-Beta-(2-naphthyl)alanine
  MOD_RES 6: note = Beta-(2-naphthyl)alanine
  MOD_RES 13: note = Beta-Alanine
CEHXRXACPPRDARRRRRQRRRR

SEQ ID NO: 234 - protein, 24 aa, synthetic construct
  REGION 1..24: note = Description of Artificial Sequence: Synthetic peptide
  MOD_RES 4: note = D-Beta-(2-naphthyl)alanine
  MOD_RES 6: note = Beta-(2-naphthyl)alanine
  MOD_RES 13: note = Beta-Alanine
CEHXRXACPPKDAYGRRRRRQRRR

SEQ ID NO: 235 - protein, 24 aa, synthetic construct
  REGION 1..24: note = Description of Artificial Sequence: Synthetic peptide
  MOD_RES 4: note = D-Beta-(2-naphthyl)alanine
  MOD_RES 6: note = Beta-(2-naphthyl)alanine
  MOD_RES 13: note = Beta-Alanine
CEHXRXACPPRDAYGRRRRRQRRR

SEQ ID NO: 236 - protein, 25 aa, synthetic construct
  REGION 1..25: note = Description of Artificial Sequence: Synthetic peptide
  MOD_RES 4: note = D-Beta-(2-naphthyl)alanine
  MOD_RES 6: note = Beta-(2-naphthyl)alanine
  MOD_RES 13: note = Beta-Alanine
CEHXRXACPPKDAYGRRRRRRQRRR

SEQ ID NO: 237 - protein, 25 aa, synthetic construct
  REGION 1..25: note = Description of Artificial Sequence: Synthetic peptide
  MOD_RES 4: note = D-Beta-(2-naphthyl)alanine
  MOD_RES 6: note = Beta-(2-naphthyl)alanine
  MOD_RES 13: note = Beta-Alanine
CEHXRXACPPRDAYGRRRRRRQRRR

SEQ ID NO: 238 - protein, 25 aa, synthetic construct
  REGION 1..25: note = Description of Artificial Sequence: Synthetic peptide
  MOD_RES 4: note = D-Beta-(2-naphthyl)alanine
  MOD_RES 6: note = Beta-(2-naphthyl)alanine
  MOD_RES 13: note = Beta-Alanine
CEHXRXACPPKDAYGRRRRRQRRRR

SEQ ID NO: 239 - protein, 25 aa, synthetic construct
  REGION 1..25: note = Description of Artificial Sequence: Synthetic peptide
  MOD_RES 4: note = D-Beta-(2-naphthyl)alanine
  MOD_RES 6: note = Beta-(2-naphthyl)alanine
  MOD_RES 13: note = Beta-Alanine
CEHXRXACPPRDAYGRRRRRQRRRR

SEQ ID NO: 240 - protein, 23 aa, synthetic construct
  REGION 1..23: note = Description of Artificial Sequence: Synthetic peptide
  MOD_RES 4: note = D-Beta-(2-naphthyl)alanine
  MOD_RES 6: note = 3-benzothienylalanine
  MOD_RES 13: note = Beta-Alanine
CEHXRXACPPKDARRRRRQRRRR

SEQ ID NO: 241 - protein, 23 aa, synthetic construct
  REGION 1..23: note = Description of Artificial Sequence: Synthetic peptide
  MOD_RES 4: note = D-Beta-(2-naphthyl)alanine
  MOD_RES 6: note = 3-benzothienylalanine
  MOD_RES 13: note = Beta-Alanine
CEHXRXACPPRDARRRRRQRRRR

SEQ ID NO: 242 - protein, 24 aa, synthetic construct
  REGION 1..24: note = Description of Artificial Sequence: Synthetic peptide
  MOD_RES 4: note = D-Beta-(2-naphthyl)alanine
  MOD_RES 6: note = 3-benzothienylalanine
  MOD_RES 13: note = Beta-Alanine
CEHXRXACPPRDAYGRRRRRQRRR

SEQ ID NO: 243 - protein, 25 aa, synthetic construct
  REGION 1..25: note = Description of Artificial Sequence: Synthetic peptide
  MOD_RES 4: note = D-Beta-(2-naphthyl)alanine
  MOD_RES 6: note = 3-benzothienylalanine
  MOD_RES 13: note = Beta-Alanine
CEHXRXACPPKDAYGRRRRRQRRRR

SEQ ID NO: 244 - protein, 25 aa, synthetic construct
  REGION 1..25: note = Description of Artificial Sequence: Synthetic peptide
  MOD_RES 4: note = D-Beta-(2-naphthyl)alanine
  MOD_RES 6: note = 3-benzothienylalanine
  MOD_RES 13: note = Beta-Alanine
CEHXRXACPPRDAYGRRRRRQRRRR

SEQ ID NO: 245 - protein, 25 aa, synthetic construct
  REGION 1..25: note = Description of Artificial Sequence: Synthetic peptide
  MOD_RES 4: note = D-Beta-(2-naphthyl)alanine
  MOD_RES 6: note = 3-benzothienylalanine
  MOD_RES 13: note = Beta-Alanine
CEHXRXACPPKDAYGRRRRRRQRRR

SEQ ID NO: 246 - protein, 25 aa, synthetic construct
  REGION 1..25: note = Description of Artificial Sequence: Synthetic peptide
  MOD_RES 4: note = D-Beta-(2-naphthyl)alanine
  MOD_RES 6: note = 3-benzothienylalanine
  MOD_RES 13: note = Beta-Alanine
CEHXRXACPPRDAYGRRRRRRQRRR

SEQ ID NO: 247 - protein, 21 aa, synthetic construct
  REGION 1..21: note = Description of Artificial Sequence: Synthetic peptide
  MOD_RES 1: note = Nle
  MOD_RES 3: note = D-Alanine
  MOD_RES 5: note = D-Phenylalanine
  MOD_RES 9: note = 8-amino-3,6-dioxaoctanoic acid
  MOD_RES 10: note = 8-amino-3,6-dioxaoctanoic acid
XCAHFRWCXXYGRKKRRQRRR

SEQ ID NO: 248 - protein, 20 aa, synthetic construct
  REGION 1..20: note = Description of Artificial Sequence: Synthetic peptide
  MOD_RES 1: note = Nle
  MOD_RES 3: note = D-Alanine
  MOD_RES 5: note = D-Phenylalanine
  MOD_RES 9: note = Beta-Alanine
XCAHFRWCAYGRKKRQRRRR

SEQ ID NO: 249 - protein, 20 aa, synthetic construct
  REGION 1..20: note = Description of Artificial Sequence: Synthetic peptide
  MOD_RES 1: note = Nle
  MOD_RES 3: note = D-Alanine
  MOD_RES 5: note = D-Phenylalanine
  MOD_RES 9: note = 8-amino-3,6-dioxaoctanoic acid
XCAHFRWCXYGRKKRRQRRR

SEQ ID NO: 250 - protein, 18 aa, synthetic construct
  REGION 1..18: note = Description of Artificial Sequence: Synthetic peptide
  MOD_RES 1: note = Nle
  MOD_RES 3: note = D-Alanine
  MOD_RES 5: note = D-Phenylalanine
  MOD_RES 9: note = Beta-Alanine
XCAHFRWCARRRRRQRRR

SEQ ID NO: 251 - protein, 19 aa, synthetic construct
  REGION 1..19: note = Description of Artificial Sequence: Synthetic peptide
  MOD_RES 1: note = Nle
  MOD_RES 3: note = D-Alanine
  MOD_RES 5: note = D-Phenylalanine
  MOD_RES 9: note = Beta-Alanine
XCAHFRWCAGRRRRRQRRR

SEQ ID NO: 252 - protein, 20 aa, synthetic construct
  REGION 1..20: note = Description of Artificial Sequence: Synthetic peptide
  MOD_RES 1: note = Nle
  MOD_RES 3: note = D-Alanine
  MOD_RES 5: note = D-Phenylalanine
  MOD_RES 9: note = Beta-Alanine
XCAHFRWCAYGRRRRRQRRR

SEQ ID NO: 253 - protein, 20 aa, synthetic construct
  REGION 1..20: note = Description of Artificial Sequence: Synthetic peptide
  MOD_RES 1: note = Nle
  MOD_RES 3: note = D-Alanine
  MOD_RES 5: note = D-Phenylalanine
  MOD_RES 9: note = Beta-Alanine
XCAHFRWCAGRRRRRQRRRR

SEQ ID NO: 254 - protein, 20 aa, synthetic construct
  REGION 1..20: note = Description of Artificial Sequence: Synthetic peptide
  MOD_RES 1: note = Nle
  MOD_RES 3: note = D-Alanine
  MOD_RES 5: note = D-Phenylalanine
  MOD_RES 9: note = Beta-Alanine
XCAHFRWCAYGRRKRRQRRR

SEQ ID NO: 255 - protein, 20 aa, synthetic construct
  REGION 1..20: note = Description of Artificial Sequence: Synthetic peptide
  MOD_RES 1: note = Nle
  MOD_RES 3: note = D-Alanine
  MOD_RES 5: note = D-Phenylalanine
  MOD_RES 9: note = Beta-Alanine
XCAHFRWCAYGRKRRRQRRR

SEQ ID NO: 256 - protein, 19 aa, synthetic construct
  REGION 1..19: note = Description of Artificial Sequence: Synthetic peptide
  MOD_RES 1: note = Nle
  MOD_RES 3: note = D-Alanine
  MOD_RES 5: note = D-Phenylalanine
  MOD_RES 9: note = Beta-Alanine
XCAHFRWCAGRRKRRQRRR

SEQ ID NO: 257 - protein, 19 aa, synthetic construct
  REGION 1..19: note = Description of Artificial Sequence: Synthetic peptide
  MOD_RES 1: note = Nle
  MOD_RES 3: note = D-Alanine
  MOD_RES 5: note = D-Phenylalanine
  MOD_RES 9: note = Beta-Alanine
XCAHFRWCAGRKRRRQRRR

SEQ ID NO: 258 - protein, 18 aa, synthetic construct
  REGION 1..18: note = Description of Artificial Sequence: Synthetic peptide
  MOD_RES 1: note = Nle
  MOD_RES 3: note = D-Alanine
  MOD_RES 5: note = D-Phenylalanine
  MOD_RES 9: note = Beta-Alanine
XCAHFRWCARRKRRQRRR

SEQ ID NO: 259 - protein, 18 aa, synthetic construct
  REGION 1..18: note = Description of Artificial Sequence: Synthetic peptide
  MOD_RES 1: note = Nle
  MOD_RES 3: note = D-Alanine
  MOD_RES 5: note = D-Phenylalanine
  MOD_RES 9: note = Beta-Alanine
XCAHFRWCARKRRRQRRR

SEQ ID NO: 260 - protein, 19 aa, synthetic construct
  REGION 1..19: note = Description of Artificial Sequence: Synthetic peptide
  MOD_RES 1: note = Nle
  MOD_RES 3: note = D-Alanine
  MOD_RES 5: note = D-Phenylalanine
  MOD_RES 9: note = Beta-Alanine
  MOD_RES 10: note = Beta-Alanine
XCAHFRWCAARRRRRQRRR

SEQ ID NO: 261 - protein, 20 aa, synthetic construct
  REGION 1..20: note = Description of Artificial Sequence: Synthetic peptide
  MOD_RES 1: note = Nle
  MOD_RES 3: note = D-Alanine
  MOD_RES 5: note = D-Phenylalanine
  MOD_RES 9: note = Beta-Alanine
  MOD_RES 10: note = Beta-Alanine
XCAHFRWCAAGRRRRRQRRR

SEQ ID NO: 262 - protein, 21 aa, synthetic construct
  REGION 1..21: note = Description of Artificial Sequence: Synthetic peptide
  MOD_RES 1: note = Nle
  MOD_RES 3: note = D-Alanine
  MOD_RES 5: note = D-Phenylalanine
  MOD_RES 9: note = Beta-Alanine
  MOD_RES 10: note = Beta-Alanine
XCAHFRWCAAYGRRRRRQRRR

SEQ ID NO: 263 - protein, 18 aa, synthetic construct
  REGION 1..18: note = Description of Artificial Sequence: Synthetic peptide
  MOD_RES 1: note = Nle
  MOD_RES 3: note = D-Alanine
  MOD_RES 5: note = D-Phenylalanine
  MOD_RES 9: note = 8-amino-3,6-dioxaoctanoic acid
XCAHFRWCXRRRRRQRRR

SEQ ID NO: 264 - protein, 19 aa, synthetic construct
  REGION 1..19: note = Description of Artificial Sequence: Synthetic peptide
  MOD_RES 1: note = Nle
  MOD_RES 3: note = D-Alanine
  MOD_RES 5: note = D-Phenylalanine
  MOD_RES 9: note = 8-amino-3,6-dioxaoctanoic acid
XCAHFRWCXGRRRRRQRRR

SEQ ID NO: 265 - protein, 20 aa, synthetic construct
  REGION 1..20: note = Description of Artificial Sequence: Synthetic peptide
  MOD_RES 1: note = Nle
  MOD_RES 3: note = D-Alanine
  MOD_RES 5: note = D-Phenylalanine
  MOD_RES 9: note = 8-amino-3,6-dioxaoctanoic acid
XCAHFRWCXYGRRRRRQRRR

SEQ ID NO: 266 - protein, 19 aa, synthetic construct
  REGION 1..19: note = Description of Artificial Sequence: Synthetic peptide
  MOD_RES 1: note = Nle
  MOD_RES 3: note = D-Alanine
  MOD_RES 5: note = D-Phenylalanine
  MOD_RES 9: note = 8-amino-3,6-dioxaoctanoic acid
  MOD_RES 10: note = 8-amino-3,6-dioxaoctanoic acid
XCAHFRWCXXRRRRRQRRR

SEQ ID NO: 267 - protein, 20 aa, synthetic construct
  REGION 1..20: note = Description of Artificial Sequence: Synthetic peptide
  MOD_RES 1: note = Nle
  MOD_RES 3: note = D-Alanine
  MOD_RES 5: note = D-Phenylalanine
  MOD_RES 9: note = 8-amino-3,6-dioxaoctanoic acid
  MOD_RES 10: note = 8-amino-3,6-dioxaoctanoic acid
XCAHFRWCXXGRRRRRQRRR

SEQ ID NO: 268 - protein, 21 aa, synthetic construct
  REGION 1..21: note = Description of Artificial Sequence: Synthetic peptide
  MOD_RES 1: note = Nle
  MOD_RES 3: note = D-Alanine
  MOD_RES 5: note = D-Phenylalanine
  MOD_RES 9: note = 8-amino-3,6-dioxaoctanoic acid
  MOD_RES 10: note = 8-amino-3,6-dioxaoctanoic acid
XCAHFRWCXXYGRRRRRQRRR

SEQ ID NO: 269 - protein, 19 aa, synthetic construct
  REGION 1..19: note = Description of Artificial Sequence: Synthetic peptide
  MOD_RES 1: note = Nle
  MOD_RES 3: note = D-Alanine
  MOD_RES 5: note = D-Phenylalanine
  MOD_RES 9: note = Beta-Alanine
XCAHFRWCARRRRRQRRRR

SEQ ID NO: 270 - protein, 21 aa, synthetic construct
  REGION 1..21: note = Description of Artificial Sequence: Synthetic peptide
  MOD_RES 1: note = Nle
  MOD_RES 3: note = D-Alanine
  MOD_RES 5: note = D-Phenylalanine
  MOD_RES 9: note = Beta-Alanine
XCAHFRWCAYGRRRRRQRRRR

SEQ ID NO: 271 - protein, 20 aa, synthetic construct
  REGION 1..20: note = Description of Artificial Sequence: Synthetic peptide
  MOD_RES 1: note = Nle
  MOD_RES 3: note = D-Alanine
  MOD_RES 5: note = D-Phenylalanine
  MOD_RES 9: note = Beta-Alanine
  MOD_RES 10: note = Beta-Alanine
XCAHFRWCAARRRRRQRRRR

SEQ ID NO: 272 - protein, 21 aa, synthetic construct
  REGION 1..21: note = Description of Artificial Sequence: Synthetic peptide
  MOD_RES 1: note = Nle
  MOD_RES 3: note = D-Alanine
  MOD_RES 5: note = D-Phenylalanine
  MOD_RES 9: note = Beta-Alanine
  MOD_RES 10: note = Beta-Alanine
XCAHFRWCAAGRRRRRQRRRR

SEQ ID NO: 273 - protein, 22 aa, synthetic construct
  REGION 1..22: note = Description of Artificial Sequence: Synthetic peptide
  MOD_RES 1: note = Nle
  MOD_RES 3: note = D-Alanine
  MOD_RES 5: note = D-Phenylalanine
  MOD_RES 9: note = Beta-Alanine
  MOD_RES 10: note = Beta-Alanine
XCAHFRWCAAYGRRRRRQRRRR

SEQ ID NO: 274 - protein, 19 aa, synthetic construct
  REGION 1..19: note = Description of Artificial Sequence: Synthetic peptide
  MOD_RES 1: note = Nle
  MOD_RES 3: note = D-Alanine
  MOD_RES 5: note = D-Phenylalanine
  MOD_RES 9: note = 8-amino-3,6-dioxaoctanoic acid
XCAHFRWCXRRRRRQRRRR

SEQ ID NO: 275 - protein, 20 aa, synthetic construct
  REGION 1..20: note = Description of Artificial Sequence: Synthetic peptide
  MOD_RES 1: note = Nle
  MOD_RES 3: note = D-Alanine
  MOD_RES 5: note = D-Phenylalanine
  MOD_RES 9: note = 8-amino-3,6-dioxaoctanoic acid
XCAHFRWCXGRRRRRQRRRR

SEQ ID NO: 276 - protein, 21 aa, synthetic construct
  REGION 1..21: note = Description of Artificial Sequence: Synthetic peptide
  MOD_RES 1: note = Nle
  MOD_RES 3: note = D-Alanine
  MOD_RES 5: note = D-Phenylalanine
  MOD_RES 9: note = 8-amino-3,6-dioxaoctanoic acid
XCAHFRWCXYGRRRRRQRRRR

SEQ ID NO: 277 - protein, 20 aa, synthetic construct
  REGION 1..20: note = Description of Artificial Sequence: Synthetic peptide
  MOD_RES 1: note = Nle
  MOD_RES 3: note = D-Alanine
  MOD_RES 5: note = D-Phenylalanine
  MOD_RES 9: note = 8-amino-3,6-dioxaoctanoic acid
  MOD_RES 10: note = 8-amino-3,6-dioxaoctanoic acid
XCAHFRWCXXRRRRRQRRRR

SEQ ID NO: 278 - protein, 21 aa, synthetic construct
  REGION 1..21: note = Description of Artificial Sequence: Synthetic peptide
  MOD_RES 1: note = Nle
  MOD_RES 3: note = D-Alanine
  MOD_RES 5: note = D-Phenylalanine
  MOD_RES 9: note = 8-amino-3,6-dioxaoctanoic acid
  MOD_RES 10: note = 8-amino-3,6-dioxaoctanoic acid
XCAHFRWCXXGRRRRRQRRRR

SEQ ID NO: 279 - protein, 22 aa, synthetic construct
  REGION 1..22: note = Description of Artificial Sequence: Synthetic peptide
  MOD_RES 1: note = Nle
  MOD_RES 3: note = D-Alanine
  MOD_RES 5: note = D-Phenylalanine
  MOD_RES 9: note = 8-amino-3,6-dioxaoctanoic acid
  MOD_RES 10: note = 8-amino-3,6-dioxaoctanoic acid
XCAHFRWCXXYGRRRRRQRRRR

SEQ ID NO: 280 - protein, 20 aa, synthetic construct
  REGION 1..20: note = Description of Artificial Sequence: Synthetic peptide
  MOD_RES 1: note = Nle
  MOD_RES 4: note = D-Phenylalanine
  MOD_RES 7: note = 4-aminobutyric acid
  MOD_RES 9: note = Beta-Alanine
XCHFRWXCAYGRRRRRQRRR

SEQ ID NO: 281 - protein, 18 aa, synthetic construct
  REGION 1..18: note = Description of Artificial Sequence: Synthetic peptide
  MOD_RES 1: note = Nle
  MOD_RES 4: note = D-Phenylalanine
  MOD_RES 7: note = 4-aminobutyric acid
  MOD_RES 9: note = Beta-Alanine
XCHFRWXCARRRRRQRRR

SEQ ID NO: 282 - protein, 20 aa, synthetic construct
  REGION 1..20: note = Description of Artificial Sequence: Synthetic peptide
  MOD_RES 1: note = Nle
  MOD_RES 4: note = D-Phenylalanine
  MOD_RES 9: note = Beta-Alanine
XDHFRWAKAYGRRRRRQRRR

SEQ ID NO: 283 - protein, 18 aa, synthetic construct
  REGION 1..18: note = Description of Artificial Sequence: Synthetic peptide
  MOD_RES 1: note = Nle
  MOD_RES 4: note = D-Phenylalanine
  MOD_RES 9: note = Beta-Alanine
XDHFRWAKARRRRRQRRR

SEQ ID NO: 284 - protein, 19 aa, synthetic construct
  REGION 1..19: note = Description of Artificial Sequence: Synthetic peptide
  MOD_RES 1: note = Nle
  MOD_RES 4: note = D-Phenylalanine
  MOD_RES 8: note = Beta-Alanine
XDHFRWKAYGRRRRRQRRR

SEQ ID NO: 285 - protein, 18 aa, synthetic construct
  REGION 1..18: note = Description of Artificial Sequence: Synthetic peptide
  MOD_RES 1: note = Nle
  MOD_RES 4: note = D-Phenylalanine
  MOD_RES 8: note = Beta-Alanine
XDHFRWKAGRRRRRQRRR

SEQ ID NO: 286 - protein, 17 aa, synthetic construct
  REGION 1..17: note = Description of Artificial Sequence: Synthetic peptide
  MOD_RES 1: note = Nle
  MOD_RES 4: note = D-Phenylalanine
  MOD_RES 8: note = Beta-Alanine
XDHFRWKARRRRRQRRR

SEQ ID NO: 287 - protein, 20 aa, synthetic construct
  REGION 1..20: note = Description of Artificial Sequence: Synthetic peptide
  MOD_RES 1: note = Nle
  MOD_RES 4: note = D-Phenylalanine
  MOD_RES 8: note = Beta-Alanine
  MOD_RES 9: note = Beta-Alanine
XDHFRWKAAYGRRRRRQRRR

SEQ ID NO: 288 - protein, 19 aa, synthetic construct
  REGION 1..19: note = Description of Artificial Sequence: Synthetic peptide
  MOD_RES 1: note = Nle
  MOD_RES 4: note = D-Phenylalanine
  MOD_RES 8: note = Beta-Alanine
  MOD_RES 9: note = Beta-Alanine
XDHFRWKAAGRRRRRQRRR

SEQ ID NO: 289 - protein, 18 aa, synthetic construct
  REGION 1..18: note = Description of Artificial Sequence: Synthetic peptide
  MOD_RES 1: note = Nle
  MOD_RES 4: note = D-Phenylalanine
  MOD_RES 8: note = Beta-Alanine
  MOD_RES 9: note = Beta-Alanine
XDHFRWKAARRRRRQRRR

SEQ ID NO: 290 - protein, 19 aa, synthetic construct
  REGION 1..19: note = Description of Artificial Sequence: Synthetic peptide
  MOD_RES 1: note = Nle
  MOD_RES 4: note = D-Phenylalanine
  MOD_RES 8: note = 8-amino-3,6-dioxaoctanoic acid
XDHFRWKXYGRRRRRQRRR

SEQ ID NO: 291 - protein, 18 aa, synthetic construct
  REGION 1..18: note = Description of Artificial Sequence: Synthetic peptide
  MOD_RES 1: note = Nle
  MOD_RES 4: note = D-Phenylalanine
  MOD_RES 8: note = 8-amino-3,6-dioxaoctanoic acid
XDHFRWKXGRRRRRQRRR

SEQ ID NO: 292 - protein, 17 aa, synthetic construct
  REGION 1..17: note = Description of Artificial Sequence: Synthetic peptide
  MOD_RES 1: note = Nle
  MOD_RES 4: note = D-Phenylalanine
  MOD_RES 8: note = 8-amino-3,6-dioxaoctanoic acid
XDHFRWKXRRRRRQRRR

SEQ ID NO: 293 - protein, 20 aa, synthetic construct
  REGION 1..20: note = Description of Artificial Sequence: Synthetic peptide
  MOD_RES 1: note = Nle
  MOD_RES 4: note = D-Phenylalanine
  MOD_RES 8: note = 8-amino-3,6-dioxaoctanoic acid
  MOD_RES 9: note = 8-amino-3,6-dioxaoctanoic acid
XDHFRWKXXYGRRRRRQRRR

SEQ ID NO: 294 - protein, 19 aa, synthetic construct
  REGION 1..19: note = Description of Artificial Sequence: Synthetic peptide
  MOD_RES 1: note = Nle
  MOD_RES 4: note = D-Phenylalanine
  MOD_RES 8: note = 8-amino-3,6-dioxaoctanoic acid
  MOD_RES 9: note = 8-amino-3,6-dioxaoctanoic acid
XDHFRWKXXGRRRRRQRRR

SEQ ID NO: 295 - protein, 18 aa, synthetic construct
  REGION 1..18: note = Description of Artificial Sequence: Synthetic peptide
  MOD_RES 1: note = Nle
  MOD_RES 4: note = D-Phenylalanine
  MOD_RES 8: note = 8-amino-3,6-dioxaoctanoic acid
  MOD_RES 9: note = 8-amino-3,6-dioxaoctanoic acid
XDHFRWKXXRRRRRQRRR

SEQ ID NO: 296 - protein, 20 aa, synthetic construct
  REGION 1..20: note = Description of Artificial Sequence: Synthetic peptide
  MOD_RES 1: note = Nle
  MOD_RES 4: note = D-Phenylalanine
  MOD_RES 8: note = Beta-Alanine
XDHFRWKAYGRRRRRQRRRR

SEQ ID NO: 297 - protein, 19 aa, synthetic construct
  REGION 1..19: note = Description of Artificial Sequence: Synthetic peptide
  MOD_RES 1: note = Nle
  MOD_RES 4: note = D-Phenylalanine
  MOD_RES 8: note = Beta-Alanine
XDHFRWKAGRRRRRQRRRR

SEQ ID NO: 298 - protein, 18 aa, synthetic construct
  REGION 1..18: note = Description of Artificial Sequence: Synthetic peptide
  MOD_RES 1: note = Nle
  MOD_RES 4: note = D-Phenylalanine
  MOD_RES 8: note = Beta-Alanine
XDHFRWKARRRRRQRRRR

SEQ ID NO: 299 - protein, 21 aa, synthetic construct
  REGION 1..21: note = Description of Artificial Sequence: Synthetic peptide
  MOD_RES 1: note = Nle
  MOD_RES 4: note = D-Phenylalanine
  MOD_RES 8: note = Beta-Alanine
  MOD_RES 9: note = Beta-Alanine
XDHFRWKAAYGRRRRRQRRRR

SEQ ID NO: 300 - protein, 20 aa, synthetic construct
  REGION 1..20: note = Description of Artificial Sequence: Synthetic peptide
  MOD_RES 1: note = Nle
  MOD_RES 4: note = D-Phenylalanine
  MOD_RES 8: note = Beta-Alanine
  MOD_RES 9: note = Beta-Alanine
XDHFRWKAAGRRRRRQRRRR

SEQ ID NO: 301 - protein, 19 aa, synthetic construct
  REGION 1..19: note = Description of Artificial Sequence: Synthetic peptide
  MOD_RES 1: note = Nle
  MOD_RES 4: note = D-Phenylalanine
  MOD_RES 8: note = Beta-Alanine
  MOD_RES 9: note = Beta-Alanine
XDHFRWKAARRRRRQRRRR

SEQ ID NO: 302 - protein, 20 aa, synthetic construct
  REGION 1..20: note = Description of Artificial Sequence: Synthetic peptide
  MOD_RES 1: note = Nle
  MOD_RES 4: note = D-Phenylalanine
  MOD_RES 8: note = 8-amino-3,6-dioxaoctanoic acid
XDHFRWKXYGRRRRRQRRRR

SEQ ID NO: 303 - protein, 19 aa, synthetic construct
  REGION 1..19: note = Description of Artificial Sequence: Synthetic peptide
  MOD_RES 1: note = Nle
  MOD_RES 4: note = D-Phenylalanine
  MOD_RES 8: note = 8-amino-3,6-dioxaoctanoic acid
XDHFRWKXGRRRRRQRRRR

SEQ ID NO: 304 - protein, 18 aa, synthetic construct
  REGION 1..18: note = Description of Artificial Sequence: Synthetic peptide
  MOD_RES 1: note = Nle
  MOD_RES 4: note = D-Phenylalanine
  MOD_RES 8: note = 8-amino-3,6-dioxaoctanoic acid
XDHFRWKXRRRRRQRRRR

SEQ ID NO: 305 - protein, 21 aa, synthetic construct
  REGION 1..21: note = Description of Artificial Sequence: Synthetic peptide
  MOD_RES 1: note = Nle
  MOD_RES 4: note = D-Phenylalanine
  MOD_RES 8: note = 8-amino-3,6-dioxaoctanoic acid
  MOD_RES 9: note = 8-amino-3,6-dioxaoctanoic acid
XDHFRWKXXYGRRRRRQRRRR

SEQ ID NO: 306 - protein, 20 aa, synthetic construct
  REGION 1..20: note = Description of Artificial Sequence: Synthetic peptide
  MOD_RES 1: note = Nle
  MOD_RES 4: note = D-Phenylalanine
  MOD_RES 8: note = 8-amino-3,6-dioxaoctanoic acid
  MOD_RES 9: note = 8-amino-3,6-dioxaoctanoic acid
XDHFRWKXXGRRRRRQRRRR

SEQ ID NO: 307 - protein, 19 aa, synthetic construct
  REGION 1..19: note = Description of Artificial Sequence: Synthetic peptide
  MOD_RES 1: note = Nle
  MOD_RES 4: note = D-Phenylalanine
  MOD_RES 8: note = 8-amino-3,6-dioxaoctanoic acid
  MOD_RES 9: note = 8-amino-3,6-dioxaoctanoic acid
XDHFRWKXXRRRRRQRRRR

SEQ ID NO: 308 - protein, 20 aa, synthetic construct
  REGION 1..20: note = Description of Artificial Sequence: Synthetic peptide
  MOD_RES 1: note = Nle
  MOD_RES 4: note = D-Phenylalanine
  MOD_RES 7: note = Beta-Alanine
  MOD_RES 9: note = Beta-Alanine
XDHFRWAKAYGRRRRRQRRR

SEQ ID NO: 309 - protein, 18 aa, synthetic construct
  REGION 1..18: note = Description of Artificial Sequence: Synthetic peptide
  MOD_RES 1: note = Nle
  MOD_RES 4: note = D-Phenylalanine
  MOD_RES 7: note = Beta-Alanine
  MOD_RES 9: note = Beta-Alanine
XDHFRWAKARRRRRQRRR

SEQ ID NO: 310 - protein, 20 aa, synthetic construct
  REGION 1..20: note = Description of Artificial Sequence: Synthetic peptide
  MOD_RES 1: note = Nle
  MOD_RES 4: note = D-Phenylalanine
  MOD_RES 7: note = 6-aminohexanoic acid
  MOD_RES 9: note = Beta-Alanine
XCHFRWXCAYGRRRRRQRRR

SEQ ID NO: 311 - protein, 18 aa, synthetic construct
  REGION 1..18: note = Description of Artificial Sequence: Synthetic peptide
  MOD_RES 1: note = Nle
  MOD_RES 4: note = D-Phenylalanine
  MOD_RES 7: note = 6-aminohexanoic acid
  MOD_RES 9: note = Beta-Alanine
XCHFRWXCARRRRRQRRR

SEQ ID NO: 312 - protein, 21 aa, synthetic construct
  REGION 1..21: note = Description of Artificial Sequence: Synthetic peptide
  MOD_RES 1: note = D-Phenylalanine
  MOD_RES 4: note = D-Phenylalanine
  MOD_RES 7: note = Beta-Alanine
  MOD_RES 8: note = D-Cysteine
  MOD_RES 10: note = Beta-Alanine
FCHFRWACTAYGRRRRRQRRR

SEQ ID NO: 313 - protein, 19 aa, synthetic construct
  REGION 1..19: note = Description of Artificial Sequence: Synthetic peptide
  MOD_RES 1: note = D-Phenylalanine
  MOD_RES 4: note = D-Phenylalanine
  MOD_RES 7: note = Beta-Alanine
  MOD_RES 8: note = D-Cysteine
  MOD_RES 10: note = Beta-Alanine
FCHFRWACTARRRRRQRRR

SEQ ID NO: 314 - protein, 20 aa, synthetic construct
  REGION 1..20: note = Description of Artificial Sequence: Synthetic peptide
  MOD_RES 1: note = Nle
  MOD_RES 4: note = D-Phenylalanine
  MOD_RES 7: note = 5-aminopentanoic acid (HN-(CH2)4-C(O)
  MOD_RES 9: note = Beta-Alanine
XCHFRWXCAYGRRRRRQRRR

SEQ ID NO: 315 - protein, 18 aa, synthetic construct
  REGION 1..18: note = Description of Artificial Sequence: Synthetic peptide
  MOD_RES 1: note = Nle
  MOD_RES 4: note = D-Phenylalanine
  MOD_RES 7: note = 5-aminopentanoic acid (HN-(CH2)4-C(O)
  MOD_RES 9: note = Beta-Alanine
XCHFRWXCARRRRRQRRR

SEQ ID NO: 316 - protein, 20 aa, synthetic construct
  REGION 1..20: note = Description of Artificial Sequence: Synthetic peptide
  MOD_RES 1: note = beta-cyclohexylalanine
  MOD_RES 4: note = D-Phenylalanine
  MOD_RES 7: note = 4-aminobutyric acid
  MOD_RES 9: note = Beta-Alanine
XDHFRWXKAYGRRRRRQRRR

SEQ ID NO: 317 - protein, 18 aa, synthetic construct
  REGION 1..18: note = Description of Artificial Sequence: Synthetic peptide
  MOD_RES 1: note = beta-cyclohexylalanine
  MOD_RES 4: note = D-Phenylalanine
  MOD_RES 7: note = 4-aminobutyric acid
  MOD_RES 9: note = Beta-Alanine
XDHFRWXKARRRRRQRRR

SEQ ID NO: 318 - protein, 20 aa, synthetic construct
  REGION 1..20: note = Description of Artificial Sequence: Synthetic peptide
  MOD_RES 1: note = Nle
  MOD_RES 4: note = D-Phenylalanine
  MOD_RES 7: note = 4-aminobutyric acid
  MOD_RES 9: note = Beta-Alanine
XDHFRWXKAYGRRRRRQRRR

SEQ ID NO: 319 - protein, 18 aa, synthetic construct
  REGION 1..18: note = Description of Artificial Sequence: Synthetic peptide
  MOD_RES 1: note = Nle
  MOD_RES 4: note = D-Phenylalanine
  MOD_RES 7: note = 4-aminobutyric acid
  MOD_RES 9: note = Beta-Alanine
XDHFRWXKARRRRRQRRR

SEQ ID NO: 320 - protein, 20 aa, synthetic construct
  REGION 1..20: note = Description of Artificial Sequence: Synthetic peptide
  MOD_RES 1: note = Cyclohexylglycine
  MOD_RES 4: note = D-Phenylalanine
  MOD_RES 7: note = 4-aminobutyric acid
  MOD_RES 9: note = Beta-Alanine
XDHFRWXKAYGRRRRRQRRR

SEQ ID NO: 321 - protein, 18 aa, synthetic construct
  REGION 1..18: note = Description of Artificial Sequence: Synthetic peptide
  MOD_RES 1: note = Cyclohexylglycine
  MOD_RES 4: note = D-Phenylalanine
  MOD_RES 7: note = 4-aminobutyric acid
  MOD_RES 9: note = Beta-Alanine
XDHFRWXKARRRRRQRRR

SEQ ID NO: 322 - protein, 20 aa, synthetic construct
  REGION 1..20: note = Description of Artificial Sequence: Synthetic peptide
  MOD_RES 1: note = homo-cyclohexylalanine
  MOD_RES 4: note = D-Phenylalanine
  MOD_RES 7: note = 4-aminobutyric acid
  MOD_RES 9: note = Beta-Alanine
XDHFRWXKAYGRRRRRQRRR

SEQ ID NO: 323 - protein, 18 aa, synthetic construct
  REGION 1..18: note = Description of Artificial Sequence: Synthetic peptide
  MOD_RES 1: note = homo-cyclohexylalanine
  MOD_RES 4: note = D-Phenylalanine
  MOD_RES 7: note = 4-aminobutyric acid
  MOD_RES 9: note = Beta-Alanine
XDHFRWXKARRRRRQRRR

SEQ ID NO: 324 - protein, 21 aa, synthetic construct
  REGION 1..21: note = Description of Artificial Sequence: Synthetic peptide
  MOD_RES 1: note = homo-cyclohexylalanine
  MOD_RES 4: note = D-Phenylalanine
  MOD_RES 7: note = 4-aminobutyric acid
  MOD_RES 9: note = Beta-Alanine
  MOD_RES 10: note = Beta-Alanine
XDHFRWXKAAYGRRRRRQRRR

SEQ ID NO: 325 - protein, 19 aa, synthetic construct
  REGION 1..19: note = Description of Artificial Sequence: Synthetic peptide
  MOD_RES 1: note = homo-cyclohexylalanine
  MOD_RES 4: note = D-Phenylalanine
  MOD_RES 7: note = 4-aminobutyric acid
  MOD_RES 9: note = Beta-Alanine
  MOD_RES 10: note = Beta-Alanine
XDHFRWXKAARRRRRQRRR

SEQ ID NO: 326 - protein, 20 aa, synthetic construct
  REGION 1..20: note = Description of Artificial Sequence: Synthetic peptide
  MOD_RES 1: note = homo-cyclohexylalanine
  MOD_RES 4: note = D-Phenylalanine
  MOD_RES 7: note = 4-aminobutyric acid
  MOD_RES 9: note = 8-amino-3,6-dioxaoctanoic acid
XDHFRWXKXYGRRRRRQRRR

SEQ ID NO: 327 - protein, 18 aa, synthetic construct
  REGION 1..18: note = Description of Artificial Sequence: Synthetic peptide
  MOD_RES 1: note = homo-cyclohexylalanine
  MOD_RES 4: note = D-Phenylalanine
  MOD_RES 7: note = 4-aminobutyric acid
  MOD_RES 9: note = 8-amino-3,6-dioxaoctanoic acid
XDHFRWXKXRRRRRQRRR

SEQ ID NO: 328 - protein, 21 aa, synthetic construct
  REGION 1..21: note = Description of Artificial Sequence: Synthetic peptide
  MOD_RES 1: note = homo-cyclohexylalanine
  MOD_RES 4: note = D-Phenylalanine
  MOD_RES 7: note = 4-aminobutyric acid
  MOD_RES 9: note = 8-amino-3,6-dioxaoctanoic acid
  MOD_RES 10: note = 8-amino-3,6-dioxaoctanoic acid
XDHFRWXKXXYGRRRRRQRRR

SEQ ID NO: 329 - protein, 19 aa, synthetic construct
  REGION 1..19: note = Description of Artificial Sequence: Synthetic peptide
  MOD_RES 1: note = homo-cyclohexylalanine
  MOD_RES 4: note = D-Phenylalanine
  MOD_RES 7: note = 4-aminobutyric acid
  MOD_RES 9: note = 8-amino-3,6-dioxaoctanoic acid
  MOD_RES 10: note = 8-amino-3,6-dioxaoctanoic acid
XDHFRWXKXXRRRRRQRRR

SEQ ID NO: 330 - protein, 21 aa, synthetic construct
  REGION 1..21: note = Description of Artificial Sequence: Synthetic peptide
  MOD_RES 1: note = homo-cyclohexylalanine
  MOD_RES 4: note = D-Phenylalanine
  MOD_RES 7: note = 4-aminobutyric acid
  MOD_RES 9: note = Beta-Alanine
XDHFRWXKAYGRRRRRQRRRR

SEQ ID NO: 331 - protein, 19 aa, synthetic construct
  REGION 1..19: note = Description of Artificial Sequence: Synthetic peptide
  MOD_RES 1: note = homo-cyclohexylalanine
  MOD_RES 4: note = D-Phenylalanine
  MOD_RES 7: note = 4-aminobutyric acid
  MOD_RES 9: note = Beta-Alanine
XDHFRWXKARRRRRQRRRR

SEQ ID NO: 332 - protein, 22 aa, synthetic construct
  REGION 1..22: note = Description of Artificial Sequence: Synthetic peptide
  MOD_RES 1: note = homo-cyclohexylalanine
  MOD_RES 4: note = D-Phenylalanine
  MOD_RES 7: note = 4-aminobutyric acid
  MOD_RES 9: note = Beta-Alanine
  MOD_RES 10: note = Beta-Alanine
XDHFRWXKAAYGRRRRRQRRRR

SEQ ID NO: 333 - protein, 20 aa, synthetic construct
  REGION 1..20: note = Description of Artificial Sequence: Synthetic peptide
  MOD_RES 1: note = homo-cyclohexylalanine
  MOD_RES 4: note = D-Phenylalanine
  MOD_RES 7: note = 4-aminobutyric acid
  MOD_RES 9: note = Beta-Alanine
  MOD_RES 10: note = Beta-Alanine
XDHFRWXKAARRRRRQRRRR

SEQ ID NO: 334 - protein, 21 aa, synthetic construct
  REGION 1..21: note = Description of Artificial Sequence: Synthetic peptide
  MOD_RES 1: note = homo-cyclohexylalanine
  MOD_RES 4: note = D-Phenylalanine
  MOD_RES 7: note = 4-aminobutyric acid
  MOD_RES 9: note = 8-amino-3,6-dioxaoctanoic acid
XDHFRWXKXYGRRRRRQRRRR

SEQ ID NO: 335 - protein, 19 aa, synthetic construct
  REGION 1..19: note = Description of Artificial Sequence: Synthetic peptide
  MOD_RES 1: note = homo-cyclohexylalanine
  MOD_RES 4: note = D-Phenylalanine
  MOD_RES 7: note = 4-aminobutyric acid
  MOD_RES 9: note = 8-amino-3,6-dioxaoctanoic acid
XDHFRWXKXRRRRRQRRRR

SEQ ID NO: 336 - protein, 22 aa, synthetic construct
  REGION 1..22: note = Description of Artificial Sequence: Synthetic peptide
  MOD_RES 1: note = homo-cyclohexylalanine
  MOD_RES 4: note = D-Phenylalanine
  MOD_RES 7: note = 4-aminobutyric acid
  MOD_RES 9: note = 8-amino-3,6-dioxaoctanoic acid
  MOD_RES 10: note = 8-amino-3,6-dioxaoctanoic acid
XDHFRWXKXXYGRRRRRQRRRR

SEQ ID NO: 337 - protein, 20 aa, synthetic construct
  REGION 1..20: note = Description of Artificial Sequence: Synthetic peptide
  MOD_RES 1: note = homo-cyclohexylalanine
  MOD_RES 4: note = D-Phenylalanine
  MOD_RES 7: note = 4-aminobutyric acid
  MOD_RES 9: note = 8-amino-3,6-dioxaoctanoic acid
  MOD_RES 10: note = 8-amino-3,6-dioxaoctanoic acid
XDHFRWXKXXRRRRRQRRRR

SEQ ID NO: 338 - protein, 20 aa, synthetic construct
  REGION 1..20: note = Description of Artificial Sequence: Synthetic peptide
  MOD_RES 1: note = D-Cyclohexylglycine
  MOD_RES 4: note = D-Phenylalanine
  MOD_RES 7: note = 4-aminobutyric acid
  MOD_RES 9: note = Beta-Alanine
XDHFRWXKAYGRRRRRQRRR

SEQ ID NO: 339 - protein, 18 aa, synthetic construct
  REGION 1..18: note = Description of Artificial Sequence: Synthetic peptide
  MOD_RES 1: note = D-Cyclohexylglycine
  MOD_RES 4: note = D-Phenylalanine
  MOD_RES 7: note = 4-aminobutyric acid
  MOD_RES 9: note = Beta-Alanine
XDHFRWXKARRRRRQRRR

SEQ ID NO: 340 - protein, 20 aa, synthetic construct
  REGION 1..20: note = Description of Artificial Sequence: Synthetic peptide
  MOD_RES 4: note = D-Phenylalanine
  MOD_RES 7: note = 4-aminobutyric acid
  MOD_RES 9: note = Beta-Alanine
FDHFRWXKAYGRRRRRQRRR

SEQ ID NO: 341 - protein, 18 aa, synthetic construct
  REGION 1..18: note = Description of Artificial Sequence: Synthetic peptide
  MOD_RES 4: note = D-Phenylalanine
  MOD_RES 7: note = 4-aminobutyric acid
  MOD_RES 9: note = Beta-Alanine
FDHFRWXKARRRRRQRRR

SEQ ID NO: 342 - protein, 20 aa, synthetic construct
  REGION 1..20: note = Description of Artificial Sequence: Synthetic peptide
  MOD_RES 1: note = Nle
  MOD_RES 4: note = D-Phenylalanine
  MOD_RES 6: note = D-Tryptophan
  MOD_RES 7: note = 5-aminopentanoic acid (HN-(CH2)4-C(O)
  MOD_RES 9: note = Beta-Alanine
XCHFRWXCAYGRRRRRQRRR

SEQ ID NO: 343 - protein, 18 aa, synthetic construct
  REGION 1..18: note = Description of Artificial Sequence: Synthetic peptide
  MOD_RES 1: note = Nle
  MOD_RES 4: note = D-Phenylalanine
  MOD_RES 6: note = D-Tryptophan
  MOD_RES 7: note = 5-aminopentanoic acid (HN-(CH2)4-C(O)
  MOD_RES 9: note = Beta-Alanine
XCHFRWXCARRRRRQRRR

SEQ ID NO: 344 - protein, 20 aa, synthetic construct
  REGION 1..20: note = Description of Artificial Sequence: Synthetic peptide
  MOD_RES 1: note = Nle
  MOD_RES 4: note = D-Phenylalanine
  MOD_RES 6: note = D-Tryptophan
  MOD_RES 7: note = 6-aminohexanoic acid
  MOD_RES 9: note = Beta-Alanine
XCHFRWXCAYGRRRRRQRRR

SEQ ID NO: 345 - protein, 18 aa, synthetic construct
  REGION 1..18: note = Description of Artificial Sequence: Synthetic peptide
  MOD_RES 1: note = Nle
  MOD_RES 4: note = D-Phenylalanine
  MOD_RES 6: note = D-Tryptophan
  MOD_RES 7: note = 6-aminohexanoic acid
  MOD_RES 9: note = Beta-Alanine
XCHFRWXCARRRRRQRRR

SEQ ID NO: 346 - protein, 20 aa, synthetic construct
  REGION 1..20: note = Description of Artificial Sequence: Synthetic peptide
  MOD_RES 1: note = Nle
  MOD_RES 4: note = D-Phenylalanine
  MOD_RES 6: note = D-Tryptophan
  MOD_RES 7: note = Beta-Alanine
  MOD_RES 9: note = Beta-Alanine
XCHFRWACAYGRRRRRQRRR

SEQ ID NO: 347 - protein, 18 aa, synthetic construct
  REGION 1..18: note = Description of Artificial Sequence: Synthetic peptide
  MOD_RES 1: note = Nle
  MOD_RES 4: note = D-Phenylalanine
  MOD_RES 6: note = D-Tryptophan
  MOD_RES 7: note = Beta-Alanine
  MOD_RES 9: note = Beta-Alanine
XCHFRWACARRRRRQRRR

SEQ ID NO: 348 - protein, 20 aa, synthetic construct
  REGION 1..20: note = Description of Artificial Sequence: Synthetic peptide
  MOD_RES 1: note = Nle
  MOD_RES 3: note = D-Alanine
  MOD_RES 5: note = D-Phenylalanine
  MOD_RES 8: note = Penicillamine
  MOD_RES 9: note = Beta-Alanine
XCAHFRWXAYGRRRRRQRRR

SEQ ID NO: 349 - protein, 19 aa, synthetic construct
  REGION 1..19: note = Description of Artificial Sequence: Synthetic peptide
  MOD_RES 1: note = Nle
  MOD_RES 3: note = D-Alanine
  MOD_RES 5: note = D-Phenylalanine
  MOD_RES 8: note = Penicillamine
  MOD_RES 9: note = Beta-Alanine
XCAHFRWXAGRRRRRQRRR

SEQ ID NO: 350 - protein, 18 aa, synthetic construct
  REGION 1..18: note = Description of Artificial Sequence: Synthetic peptide
  MOD_RES 1: note = Nle
  MOD_RES 3: note = D-Alanine
  MOD_RES 5: note = D-Phenylalanine
  MOD_RES 8: note = Penicillamine
  MOD_RES 9: note = Beta-Alanine
XCAHFRWXARRRRRQRRR

SEQ ID NO: 351 - protein, 21 aa, synthetic construct
  REGION 1..21: note = Description of Artificial Sequence: Synthetic peptide
  MOD_RES 1: note = Nle
  MOD_RES 3: note = D-Alanine
  MOD_RES 5: note = D-Phenylalanine
  MOD_RES 8: note = Penicillamine
  MOD_RES 9: note = Beta-Alanine
  MOD_RES 10: note = Beta-Alanine
XCAHFRWXAAYGRRRRRQRRR

SEQ ID NO: 352 - protein, 20 aa, synthetic construct
  REGION 1..20: note = Description of Artificial Sequence: Synthetic peptide
  MOD_RES 1: note = Nle
  MOD_RES 3: note = D-Alanine
  MOD_RES 5: note = D-Phenylalanine
  MOD_RES 8: note = Penicillamine
  MOD_RES 9: note = Beta-Alanine
  MOD_RES 10: note = Beta-Alanine
XCAHFRWXAAGRRRRRQRRR

SEQ ID NO: 353 - protein, 19 aa, synthetic construct
  REGION 1..19: note = Description of Artificial Sequence: Synthetic peptide
  MOD_RES 1: note = Nle
  MOD_RES 3: note = D-Alanine
  MOD_RES 5: note = D-Phenylalanine
  MOD_RES 8: note = Penicillamine
  MOD_RES 9: note = Beta-Alanine
  MOD_RES 10: note = Beta-Alanine
XCAHFRWXAARRRRRQRRR

SEQ ID NO: 354 - protein, 20 aa, synthetic construct
  REGION 1..20: note = Description of Artificial Sequence: Synthetic peptide
  MOD_RES 1: note = Nle
  MOD_RES 3: note = D-Alanine
  MOD_RES 5: note = D-Phenylalanine
  MOD_RES 8: note = Penicillamine
  MOD_RES 9: note = 8-amino-3,6-dioxaoctanoic acid
XCAHFRWXXYGRRRRRQRRR

SEQ ID NO: 355 - protein, 19 aa, synthetic construct
  REGION 1..19: note = Description of Artificial Sequence: Synthetic peptide
  MOD_RES 1: note = Nle
  MOD_RES 3: note = D-Alanine
  MOD_RES 5: note = D-Phenylalanine
  MOD_RES 8: note = Penicillamine
  MOD_RES 9: note = 8-amino-3,6-dioxaoctanoic acid
XCAHFRWXXGRRRRRQRRR

SEQ ID NO: 356 - protein, 18 aa, synthetic construct
  REGION 1..18: note = Description of Artificial Sequence: Synthetic peptide
  MOD_RES 1: note = Nle
  MOD_RES 3: note = D-Alanine
  MOD_RES 5: note = D-Phenylalanine
  MOD_RES 8: note = Penicillamine
  MOD_RES 9: note = 8-amino-3,6-dioxaoctanoic acid
XCAHFRWXXRRRRRQRRR

SEQ ID NO: 357 - protein, 21 aa, synthetic construct
  REGION 1..21: note = Description of Artificial Sequence: Synthetic peptide
  MOD_RES 1: note = Nle
  MOD_RES 3: note = D-Alanine
  MOD_RES 5: note = D-Phenylalanine
  MOD_RES 8: note = Penicillamine
  MOD_RES 9: note = 8-amino-3,6-dioxaoctanoic acid
  MOD_RES 10: note = 8-amino-3,6-dioxaoctanoic acid
XCAHFRWXXXYGRRRRRQRRR

SEQ ID NO: 358 - protein, 20 aa, synthetic construct
  REGION 1..20: note = Description of Artificial Sequence: Synthetic peptide
  MOD_RES 1: note = Nle
  MOD_RES 3: note = D-Alanine
  MOD_RES 5: note = D-Phenylalanine
  MOD_RES 8: note = Penicillamine
  MOD_RES 9: note = 8-amino-3,6-dioxaoctanoic acid
  MOD_RES 10: note = 8-amino-3,6-dioxaoctanoic acid
XCAHFRWXXXGRRRRRQRRR

SEQ ID NO: 359 - protein, 19 aa, synthetic construct
  REGION 1..19: note = Description of Artificial Sequence: Synthetic peptide
  MOD_RES 1: note = Nle
  MOD_RES 3: note = D-Alanine
  MOD_RES 5: note = D-Phenylalanine
  MOD_RES 8: note = Penicillamine
  MOD_RES 9: note = 8-amino-3,6-dioxaoctanoic acid
  MOD_RES 10: note = 8-amino-3,6-dioxaoctanoic acid
XCAHFRWXXXRRRRRQRRR

SEQ ID NO: 360 - protein, 20 aa, synthetic construct
  REGION 1..20: note = Description of Artificial Sequence: Synthetic peptide
  MOD_RES 1: note = D-Phenylalanine
  MOD_RES 4: note = O-Ethyl-D-Tyrosine
  MOD_RES 7: note = Beta-Alanine
  MOD_RES 8: note = D-Cysteine
  MOD_RES 9: note = Beta-Alanine
FCHYRWACAYGRRRRRQRRR

SEQ ID NO: 361 - protein, 18 aa, synthetic construct
  REGION 1..18: note = Description of Artificial Sequence: Synthetic peptide
  MOD_RES 1: note = D-Phenylalanine
  MOD_RES 4: note = O-Ethyl-D-Tyrosine
  MOD_RES 7: note = Beta-Alanine
  MOD_RES 8: note = D-Cysteine
  MOD_RES 9: note = Beta-Alanine
FCHYRWACARRRRRQRRR

SEQ ID NO: 362 - protein, 19 aa, synthetic construct
  REGION 1..19: note = Description of Artificial Sequence: Synthetic peptide
  MOD_RES 1: note = D-Phenylalanine
  MOD_RES 4: note = O-Ethyl-D-Tyrosine
  MOD_RES 7: note = Beta-Alanine
  MOD_RES 8: note = D-Cysteine
  MOD_RES 9: note = Beta-Alanine
FCHYRWACAGRRRRRQRRR

SEQ ID NO: 363 - protein, 19 aa, synthetic construct
  REGION 1..19: note = Description of Artificial Sequence: Synthetic peptide
  MOD_RES 1: note = D-Phenylalanine
  MOD_RES 4: note = O-Ethyl-D-Tyrosine
  MOD_RES 7: note = Beta-Alanine
  MOD_RES 8: note = D-Cysteine
  MOD_RES 9: note = Beta-Alanine
FCHYRWACARRRRRQRRRR

SEQ ID NO: 364 - protein, 21 aa, synthetic construct
  REGION 1..21: note = Description of Artificial Sequence: Synthetic peptide
  MOD_RES 1: note = D-Phenylalanine
  MOD_RES 4: note = O-Ethyl-D-Tyrosine
  MOD_RES 7: note = Beta-Alanine
  MOD_RES 8: note = D-Cysteine
  MOD_RES 9: note = Beta-Alanine
  MOD_RES 10: note = Beta-Alanine
FCHYRWACAAYGRRRRRQRRR

SEQ ID NO: 365 - protein, 19 aa, synthetic construct
  REGION 1..19: note = Description of Artificial Sequence: Synthetic peptide
  MOD_RES 1: note = D-Phenylalanine
  MOD_RES 4: note = O-Ethyl-D-Tyrosine
  MOD_RES 7: note = Beta-Alanine
  MOD_RES 8: note = D-Cysteine
  MOD_RES 9: note = Beta-Alanine
  MOD_RES 10: note = Beta-Alanine
FCHYRWACAARRRRRQRRR

SEQ ID NO: 366 - protein, 20 aa, synthetic construct
  REGION 1..20: note = Description of Artificial Sequence: Synthetic peptide
  MOD_RES 1: note = D-Phenylalanine
  MOD_RES 4: note = O-Ethyl-D-Tyrosine
  MOD_RES 7: note = Beta-Alanine
  MOD_RES 8: note = D-Cysteine
  MOD_RES 9: note = Beta-Alanine
  MOD_RES 10: note = Beta-Alanine
FCHYRWACAAGRRRRRQRRR

SEQ ID NO: 367 - protein, 20 aa, synthetic construct
  REGION 1..20: note = Description of Artificial Sequence: Synthetic peptide
  MOD_RES 1: note = D-Phenylalanine
  MOD_RES 4: note = O-Ethyl-D-Tyrosine
  MOD_RES 7: note = Beta-Alanine
  MOD_RES 8: note = D-Cysteine
  MOD_RES 9: note = Beta-Alanine
  MOD_RES 10: note = Beta-Alanine
FCHYRWACAARRRRRQRRRR

SEQ ID NO: 368 - protein, 20 aa, synthetic construct
  REGION 1..20: note = Description of Artificial Sequence: Synthetic peptide
  MOD_RES 1: note = D-Phenylalanine
  MOD_RES 4: note = O-Ethyl-D-Tyrosine
  MOD_RES 7: note = Beta-Alanine
  MOD_RES 8: note = D-Cysteine
  MOD_RES 9: note = 8-amino-3,6-dioxaoctanoic acid
FCHYRWACXYGRRRRRQRRR

SEQ ID NO: 369 - protein, 18 aa, synthetic construct
  REGION 1..18: note = Description of Artificial Sequence: Synthetic peptide
  MOD_RES 1: note = D-Phenylalanine
  MOD_RES 4: note = O-Ethyl-D-Tyrosine
  MOD_RES 7: note = Beta-Alanine
  MOD_RES 8: note = D-Cysteine
  MOD_RES 9: note = 8-amino-3,6-dioxaoctanoic acid
FCHYRWACXRRRRRQRRR

SEQ ID NO: 370 - protein, 19 aa, synthetic construct
  REGION 1..19: note = Description of Artificial Sequence: Synthetic peptide
  MOD_RES 1: note = D-Phenylalanine
  MOD_RES 4: note = O-Ethyl-D-Tyrosine
  MOD_RES 7: note = Beta-Alanine
  MOD_RES 8: note = D-Cysteine
  MOD_RES 9: note = 8-amino-3,6-dioxaoctanoic acid
FCHYRWACXGRRRRRQRRR

SEQ ID NO: 371 - protein, 19 aa, synthetic construct
  REGION 1..19: note = Description of Artificial Sequence: Synthetic peptide
  MOD_RES 1: note = D-Phenylalanine
  MOD_RES 4: note = O-Ethyl-D-Tyrosine
  MOD_RES 7: note = Beta-Alanine
  MOD_RES 8: note = D-Cysteine
  MOD_RES 9: note = 8-amino-3,6-dioxaoctanoic acid
FCHYRWACXRRRRRQRRRR

SEQ ID NO: 372 - protein, 21 aa, synthetic construct
  REGION 1..21: note = Description of Artificial Sequence: Synthetic peptide
  MOD_RES 1: note = D-Phenylalanine
  MOD_RES 4: note = O-Ethyl-D-Tyrosine
  MOD_RES 7: note = Beta-Alanine
  MOD_RES 8: note = D-Cysteine
  MOD_RES 9: note = 8-amino-3,6-dioxaoctanoic acid
  MOD_RES 10: note = 8-amino-3,6-dioxaoctanoic acid
FCHYRWACXXYGRRRRRQRRR

SEQ ID NO: 373 - protein, 19 aa, synthetic construct
  REGION 1..19: note = Description of Artificial Sequence: Synthetic peptide
  MOD_RES 1: note = D-Phenylalanine
  MOD_RES 4: note = O-Ethyl-D-Tyrosine
  MOD_RES 7: note = Beta-Alanine
  MOD_RES 8: note = D-Cysteine
  MOD_RES 9: note = 8-amino-3,6-dioxaoctanoic acid
  MOD_RES 10: note = 8-amino-3,6-dioxaoctanoic acid
FCHYRWACXXRRRRRQRRR

SEQ ID NO: 374 - protein, 20 aa, synthetic construct
  REGION 1..20: note = Description of Artificial Sequence: Synthetic peptide
  MOD_RES 1: note = D-Phenylalanine
  MOD_RES 4: note = O-Ethyl-D-Tyrosine
  MOD_RES 7: note = Beta-Alanine
  MOD_RES 8: note = D-Cysteine
  MOD_RES 9: note = 8-amino-3,6-dioxaoctanoic acid
  MOD_RES 10: note = 8-amino-3,6-dioxaoctanoic acid
FCHYRWACXXGRRRRRQRRR

SEQ ID NO: 375 - protein, 20 aa, synthetic construct
  REGION 1..20: note = Description of Artificial Sequence: Synthetic peptide
  MOD_RES 1: note = D-Phenylalanine
  MOD_RES 4: note = O-Ethyl-D-Tyrosine
  MOD_RES 7: note = Beta-Alanine
  MOD_RES 8: note = D-Cysteine
  MOD_RES 9: note = 8-amino-3,6-dioxaoctanoic acid
  MOD_RES 10: note = 8-amino-3,6-dioxaoctanoic acid
FCHYRWACXXRRRRRQRRRR

SEQ ID NO: 376 - protein, 21 aa, synthetic construct
  REGION 1..21: note = Description of Artificial Sequence: Synthetic peptide
  MOD_RES 1: note = D-Phenylalanine
  MOD_RES 4: note = O-Ethyl-D-Tyrosine
  MOD_RES 7: note = Beta-Alanine
  MOD_RES 8: note = D-Cysteine
  MOD_RES 10: note = Beta-Alanine
FCHYRWACTAYGRRRRRQRRR

SEQ ID NO: 377 - protein, 19 aa, synthetic construct
  REGION 1..19: note = Description of Artificial Sequence: Synthetic peptide
  MOD_RES 1: note = D-Phenylalanine
  MOD_RES 4: note = O-Ethyl-D-Tyrosine
  MOD_RES 7: note = Beta-Alanine
  MOD_RES 8: note = D-Cysteine
  MOD_RES 10: note = Beta-Alanine
FCHYRWACTARRRRRQRRR

SEQ ID NO: 378 - protein, 22 aa, synthetic construct
  REGION 1..22: note = Description of Artificial Sequence: Synthetic peptide
  MOD_RES 1: note = D-Phenylalanine
  MOD_RES 4: note = O-Ethyl-D-Tyrosine
  MOD_RES 7: note = Beta-Alanine
  MOD_RES 8: note = D-Cysteine
  MOD_RES 10: note = Beta-Alanine
  MOD_RES 11: note = Beta-Alanine
FCHYRWACTAAYGRRRRRQRRR

SEQ ID NO: 379 - protein, 20 aa, synthetic construct
  REGION 1..20: note = Description of Artificial Sequence: Synthetic peptide
  MOD_RES 1: note = D-Phenylalanine
  MOD_RES 4: note = O-Ethyl-D-Tyrosine
  MOD_RES 7: note = Beta-Alanine
  MOD_RES 8: note = D-Cysteine
  MOD_RES 10: note = Beta-Alanine
  MOD_RES 11: note = Beta-Alanine
FCHYRWACTAARRRRRQRRR

SEQ ID NO: 380 - protein, 21 aa, synthetic construct
  REGION 1..21: note = Description of Artificial Sequence: Synthetic peptide
  MOD_RES 1: note = D-Phenylalanine
  MOD_RES 4: note = O-Ethyl-D-Tyrosine
  MOD_RES 7: note = Beta-Alanine
  MOD_RES 8: note = D-Cysteine
  MOD_RES 10: note = 8-amino-3,6-dioxaoctanoic acid
FCHYRWACTXYGRRRRRQRRR

SEQ ID NO: 381 - protein, 19 aa, synthetic construct
  REGION 1..19: note = Description of Artificial Sequence: Synthetic peptide
  MOD_RES 1: note = D-Phenylalanine
  MOD_RES 4: note = O-Ethyl-D-Tyrosine
  MOD_RES 7: note = Beta-Alanine
  MOD_RES 8: note = D-Cysteine
  MOD_RES 10: note = 8-amino-3,6-dioxaoctanoic acid
FCHYRWACTXRRRRRQRRR

SEQ ID NO: 382 - protein, 22 aa, synthetic construct
  REGION 1..22: note = Description of Artificial Sequence: Synthetic peptide
  MOD_RES 1: note = D-Phenylalanine
  MOD_RES 4: note = O-Ethyl-D-Tyrosine
  MOD_RES 7: note = Beta-Alanine
  MOD_RES 8: note = D-Cysteine
  MOD_RES 10: note = 8-amino-3,6-dioxaoctanoic acid
  MOD_RES 11: note = 8-amino-3,6-dioxaoctanoic acid
FCHYRWACTXXYGRRRRRQRRR

SEQ ID NO: 383 - protein, 22 aa, synthetic construct
  REGION 1..22: note = Description of Artificial Sequence: Synthetic peptide
  MOD_RES 1: note = D-Phenylalanine
  MOD_RES 4: note = O-Ethyl-D-Tyrosine
  MOD_RES 7: note = Beta-Alanine
  MOD_RES 8: note = D-Cysteine
  MOD_RES 10: note = Beta-Alanine
FCHYRWACTAYGRRRRRQRRRR

SEQ ID NO: 384 - protein, 20 aa, synthetic construct
  REGION 1..20: note = Description of Artificial Sequence: Synthetic peptide
  MOD_RES 1: note = D-Phenylalanine
  MOD_RES 4: note = O-Ethyl-D-Tyrosine
  MOD_RES 7: note = Beta-Alanine
  MOD_RES 8: note = D-Cysteine
  MOD_RES 10: note = Beta-Alanine
FCHYRWACTARRRRRQRRRR

SEQ ID NO: 385 - protein, 23 aa, synthetic construct
  REGION 1..23: note = Description of Artificial Sequence: Synthetic peptide
  MOD_RES 1: note = D-Phenylalanine
  MOD_RES 4: note = O-Ethyl-D-Tyrosine
  MOD_RES 7: note = Beta-Alanine
  MOD_RES 8: note = D-Cysteine
  MOD_RES 10: note = Beta-Alanine
  MOD_RES 11: note = Beta-Alanine
FCHYRWACTAAYGRRRRRQRRRR

SEQ ID NO: 386 - protein, 21 aa, synthetic construct
  REGION 1..21: note = Description of Artificial Sequence: Synthetic peptide
  MOD_RES 1: note = D-Phenylalanine
  MOD_RES 4: note = O-Ethyl-D-Tyrosine
  MOD_RES 7: note = Beta-Alanine
  MOD_RES 8: note = D-Cysteine
  MOD_RES 10: note = Beta-Alanine
  MOD_RES 11: note = Beta-Alanine
FCHYRWACTAARRRRRQRRRR

SEQ ID NO: 387 - protein, 22 aa, synthetic construct
  REGION 1..22: note = Description of Artificial Sequence: Synthetic peptide
  MOD_RES 1: note = D-Phenylalanine
  MOD_RES 4: note = O-Ethyl-D-Tyrosine
  MOD_RES 7: note = Beta-Alanine
  MOD_RES 8: note = D-Cysteine
  MOD_RES 10: note = 8-amino-3,6-dioxaoctanoic acid
FCHYRWACTXYGRRRRRQRRRR

SEQ ID NO: 388 - protein, 20 aa, synthetic construct
  REGION 1..20: note = Description of Artificial Sequence: Synthetic peptide
  MOD_RES 1: note = D-Phenylalanine
  MOD_RES 4: note = O-Ethyl-D-Tyrosine
  MOD_RES 7: note = Beta-Alanine
  MOD_RES 8: note = D-Cysteine
  MOD_RES 10: note = 8-amino-3,6-dioxaoctanoic acid
FCHYRWACTXRRRRRQRRRR

SEQ ID NO: 389 - protein, 23 aa, synthetic construct
  REGION 1..23: note = Description of Artificial Sequence: Synthetic peptide
  MOD_RES 1: note = D-Phenylalanine
  MOD_RES 4: note = O-Ethyl-D-Tyrosine
  MOD_RES 7: note = Beta-Alanine
  MOD_RES 8: note = D-Cysteine
  MOD_RES 10: note = 8-amino-3,6-dioxaoctanoic acid
  MOD_RES 11: note = 8-amino-3,6-dioxaoctanoic acid
FCHYRWACTXXYGRRRRRQRRRR

SEQ ID NO: 390 - protein, 21 aa, synthetic construct
  REGION 1..21: note = Description of Artificial Sequence: Synthetic peptide
  MOD_RES 1: note = D-Phenylalanine
  MOD_RES 4: note = O-Ethyl-D-Tyrosine
  MOD_RES 7: note = Beta-Alanine
  MOD_RES 8: note = D-Cysteine
  MOD_RES 10: note = 8-amino-3,6-dioxaoctanoic acid
  MOD_RES 11: note = 8-amino-3,6-dioxaoctanoic acid
FCHYRWACTXXRRRRRQRRRR

SEQ ID NO: 391 - protein, 21 aa, synthetic construct
  REGION 1..21: note = Description of Artificial Sequence: Synthetic peptide
  MOD_RES 1: note = D-Phenylalanine
  MOD_RES 4: note = O-Ethyl-D-Tyrosine
  MOD_RES 6: note = 4,4 -biphenylalanine
  MOD_RES 7: note = Beta-Alanine
  MOD_RES 8: note = D-Cysteine
  MOD_RES 10: note = Beta-Alanine
FCHYRXACTAYGRRRRRQRRR

SEQ ID NO: 392 - protein, 22 aa, synthetic construct
  REGION 1..22: note = Description of Artificial Sequence: Synthetic peptide
  MOD_RES 1: note = D-Phenylalanine
  MOD_RES 4: note = O-Ethyl-D-Tyrosine
  MOD_RES 6: note = 4,4 -biphenylalanine
  MOD_RES 7: note = Beta-Alanine
  MOD_RES 8: note = D-Cysteine
  MOD_RES 10: note = Beta-Alanine
FCHYRXACTAYGRRRRRQRRRR

SEQ ID NO: 393 - protein, 19 aa, synthetic construct
  REGION 1..19: note = Description of Artificial Sequence: Synthetic peptide
  MOD_RES 1: note = D-Phenylalanine
  MOD_RES 4: note = O-Ethyl-D-Tyrosine
  MOD_RES 6: note = 4,4 -biphenylalanine
  MOD_RES 7: note = Beta-Alanine
  MOD_RES 8: note = D-Cysteine
  MOD_RES 10: note = Beta-Alanine
FCHYRXACTARRRRRQRRR

SEQ ID NO: 394 - protein, 22 aa, synthetic construct
  REGION 1..22: note = Description of Artificial Sequence: Synthetic peptide
  MOD_RES 1: note = D-Phenylalanine
  MOD_RES 4: note = O-Ethyl-D-Tyrosine
  MOD_RES 6: note = 4,4 -biphenylalanine
  MOD_RES 7: note = Beta-Alanine
  MOD_RES 8: note = D-Cysteine
  MOD_RES 10: note = Beta-Alanine
  MOD_RES 11: note = Beta-Alanine
FCHYRXACTAAYGRRRRRQRRR

SEQ ID NO: 395 - protein, 20 aa, synthetic construct
  REGION 1..20: note = Description of Artificial Sequence: Synthetic peptide
  MOD_RES 1: note = D-Phenylalanine
  MOD_RES 4: note = O-Ethyl-D-Tyrosine
  MOD_RES 6: note = 4,4 -biphenylalanine
  MOD_RES 7: note = Beta-Alanine
  MOD_RES 8: note = D-Cysteine
  MOD_RES 10: note = Beta-Alanine
  MOD_RES 11: note = Beta-Alanine
FCHYRXACTAARRRRRQRRR

SEQ ID NO: 396 - protein, 21 aa, synthetic construct
  REGION 1..21: note = Description of Artificial Sequence: Synthetic peptide
  MOD_RES 1: note = D-Phenylalanine
  MOD_RES 4: note = O-Ethyl-D-Tyrosine
  MOD_RES 6: note = 4,4 -biphenylalanine
  MOD_RES 7: note = Beta-Alanine
  MOD_RES 8: note = D-Cysteine
  MOD_RES 10: note = 8-amino-3,6-dioxaoctanoic acid
FCHYRXACTXYGRRRRRQRRR

SEQ ID NO: 397 - protein, 22 aa, synthetic construct
  REGION 1..22: note = Description of Artificial Sequence: Synthetic peptide
  MOD_RES 1: note = D-Phenylalanine
  MOD_RES 4: note = O-Ethyl-D-Tyrosine
  MOD_RES 6: note = 4,4 -biphenylalanine
  MOD_RES 7: note = Beta-Alanine
  MOD_RES 8: note = D-Cysteine
  MOD_RES 10: note = 8-amino-3,6-dioxaoctanoic acid
FCHYRXACTXYGRRRRRQRRRR

SEQ ID NO: 398 - protein, 19 aa, synthetic construct
  REGION 1..19: note = Description of Artificial Sequence: Synthetic peptide
  MOD_RES 1: note = D-Phenylalanine
  MOD_RES 4: note = O-Ethyl-D-Tyrosine
  MOD_RES 6: note = 4,4 -biphenylalanine
  MOD_RES 7: note = Beta-Alanine
  MOD_RES 8: note = D-Cysteine
  MOD_RES 10: note = 8-amino-3,6-dioxaoctanoic acid
FCHYRXACTXRRRRRQRRR

SEQ ID NO: 399 - protein, 22 aa, synthetic construct
  REGION 1..22: note = Description of Artificial Sequence: Synthetic peptide
  MOD_RES 1: note = D-Phenylalanine
  MOD_RES 4: note = O-Ethyl-D-Tyrosine
  MOD_RES 6: note = 4,4 -biphenylalanine
  MOD_RES 7: note = Beta-Alanine
  MOD_RES 8: note = D-Cysteine
  MOD_RES 10: note = 8-amino-3,6-dioxaoctanoic acid
  MOD_RES 11: note = 8-amino-3,6-dioxaoctanoic acid
FCHYRXACTXXYGRRRRRQRRR

SEQ ID NO: 400 - protein, 20 aa, synthetic construct
  REGION 1..20: note = Description of Artificial Sequence: Synthetic peptide
  MOD_RES 1: note = D-Phenylalanine
  MOD_RES 4: note = O-Ethyl-D-Tyrosine
  MOD_RES 6: note = 4,4 -biphenylalanine
  MOD_RES 7: note = Beta-Alanine
  MOD_RES 8: note = D-Cysteine
  MOD_RES 10: note = 8-amino-3,6-dioxaoctanoic acid
  MOD_RES 11: note = 8-amino-3,6-dioxaoctanoic acid
FCHYRXACTXXRRRRRQRRR

SEQ ID NO: 401 - protein, 21 aa, synthetic construct
  REGION 1..21: note = Description of Artificial Sequence: Synthetic peptide
  MOD_RES 1: note = Nle
  MOD_RES 3: note = D-Alanine
  MOD_RES 5: note = D-Phenylalanine
  MOD_RES 10: note = Beta-Alanine
XCAHFRWGCAYGRRRRRQRRR

SEQ ID NO: 402 - protein, 19 aa, synthetic construct
  REGION 1..19: note = Description of Artificial Sequence: Synthetic peptide
  MOD_RES 1: note = Nle
  MOD_RES 3: note = D-Alanine
  MOD_RES 5: note = D-Phenylalanine
  MOD_RES 10: note = Beta-Alanine
XCAHFRWGCARRRRRQRRR

SEQ ID NO: 403 - protein, 20 aa, synthetic construct
  REGION 1..20: note = Description of Artificial Sequence: Synthetic peptide
  MOD_RES 1: note = Nle
  MOD_RES 4: note = D-Phenylalanine
  MOD_RES 7: note = 5-aminopentanoic acid (HN-(CH2)4-C(O)
  MOD_RES 9: note = Beta-Alanine
XCHFRWXCAYGRRRRRQRRR

SEQ ID NO: 404 - protein, 18 aa, synthetic construct
  REGION 1..18: note = Description of Artificial Sequence: Synthetic peptide
  MOD_RES 1: note = Nle
  MOD_RES 4: note = D-Phenylalanine
  MOD_RES 7: note = 5-aminopentanoic acid (HN-(CH2)4-C(O)
  MOD_RES 9: note = Beta-Alanine
XCHFRWXCARRRRRQRRR

SEQ ID NO: 405 - protein, 21 aa, synthetic construct
  REGION 1..21: note = Description of Artificial Sequence: Synthetic peptide
  MOD_RES 1: note = Nle
  MOD_RES 4: note = D-Phenylalanine
  MOD_RES 7: note = 5-aminopentanoic acid (HN-(CH2)4-C(O)
  MOD_RES 9: note = Beta-Alanine
  MOD_RES 10: note = Beta-Alanine
XCHFRWXCAAYGRRRRRQRRR

SEQ ID NO: 406 - protein, 19 aa, synthetic construct
  REGION 1..19: note = Description of Artificial Sequence: Synthetic peptide
  MOD_RES 1: note = Nle
  MOD_RES 4: note = D-Phenylalanine
  MOD_RES 7: note = 5-aminopentanoic acid (HN-(CH2)4-C(O)
  MOD_RES 9: note = Beta-Alanine
  MOD_RES 10: note = Beta-Alanine
XCHFRWXCAARRRRRQRRR

SEQ ID NO: 407 - protein, 21 aa, synthetic construct
  REGION 1..21: note = Description of Artificial Sequence: Synthetic peptide
  MOD_RES 1: note = Nle
  MOD_RES 4: note = D-Phenylalanine
  MOD_RES 7: note = 5-aminopentanoic acid (HN-(CH2)4-C(O)
  MOD_RES 9: note = Beta-Alanine
XCHFRWXCAYGRRRRRQRRRR

SEQ ID NO: 408 - protein, 19 aa, synthetic construct
  REGION 1..19: note = Description of Artificial Sequence: Synthetic peptide
  MOD_RES 1: note = Nle
  MOD_RES 4: note = D-Phenylalanine
  MOD_RES 7: note = 5-aminopentanoic acid (HN-(CH2)4-C(O)
  MOD_RES 9: note = Beta-Alanine
XCHFRWXCARRRRRQRRRR

SEQ ID NO: 409 - protein, 22 aa, synthetic construct
  REGION 1..22: note = Description of Artificial Sequence: Synthetic peptide
  MOD_RES 1: note = Nle
  MOD_RES 4: note = D-Phenylalanine
  MOD_RES 7: note = 5-aminopentanoic acid (HN-(CH2)4-C(O)
  MOD_RES 9: note = Beta-Alanine
  MOD_RES 10: note = Beta-Alanine
XCHFRWXCAAYGRRRRRQRRRR

SEQ ID NO: 410 - protein, 20 aa, synthetic construct
  REGION 1..20: note = Description of Artificial Sequence: Synthetic peptide
  MOD_RES 1: note = Nle
  MOD_RES 4: note = D-Phenylalanine
  MOD_RES 7: note = 5-aminopentanoic acid (HN-(CH2)4-C(O)
  MOD_RES 9: note = Beta-Alanine
  MOD_RES 10: note = Beta-Alanine
XCHFRWXCAARRRRRQRRRR

SEQ ID NO: 411 - protein, 20 aa, synthetic construct
  REGION 1..20: note = Description of Artificial Sequence: Synthetic peptide
  MOD_RES 1: note = Nle
  MOD_RES 4: note = D-Phenylalanine
  MOD_RES 7: note = 5-aminopentanoic acid (HN-(CH2)4-C(O)
  MOD_RES 9: note = 8-amino-3,6-dioxaoctanoic acid
XCHFRWXCXYGRRRRRQRRR

SEQ ID NO: 412 - protein, 18 aa, synthetic construct
  REGION 1..18: note = Description of Artificial Sequence: Synthetic peptide
  MOD_RES 1: note = Nle
  MOD_RES 4: note = D-Phenylalanine
  MOD_RES 7: note = 5-aminopentanoic acid (HN-(CH2)4-C(O)
  MOD_RES 9: note = 8-amino-3,6-dioxaoctanoic acid
XCHFRWXCXRRRRRQRRR

SEQ ID NO: 413 - protein, 21 aa, synthetic construct
  REGION 1..21: note = Description of Artificial Sequence: Synthetic peptide
  MOD_RES 1: note = Nle
  MOD_RES 4: note = D-Phenylalanine
  MOD_RES 7: note = 5-aminopentanoic acid (HN-(CH2)4-C(O)
  MOD_RES 9: note = 8-amino-3,6-dioxaoctanoic acid
  MOD_RES 10: note = 8-amino-3,6-dioxaoctanoic acid
XCHFRWXCXXYGRRRRRQRRR

SEQ ID NO: 414 - protein, 19 aa, synthetic construct
  REGION 1..19: note = Description of Artificial Sequence: Synthetic peptide
  MOD_RES 1: note = Nle
  MOD_RES 4: note = D-Phenylalanine
  MOD_RES 7: note = 5-aminopentanoic acid (HN-(CH2)4-C(O)
  MOD_RES 9: note = 8-amino-3,6-dioxaoctanoic acid
  MOD_RES 10: note = 8-amino-3,6-dioxaoctanoic acid
XCHFRWXCXXRRRRRQRRR

SEQ ID NO: 415 - protein, 21 aa, synthetic construct
  REGION 1..21: note = Description of Artificial Sequence: Synthetic peptide
  MOD_RES 1: note = Nle
  MOD_RES 4: note = D-Phenylalanine
  MOD_RES 7: note = 5-aminopentanoic acid (HN-(CH2)4-C(O)
  MOD_RES 9: note = 8-amino-3,6-dioxaoctanoic acid
XCHFRWXCXYGRRRRRQRRRR

SEQ ID NO: 416 - protein, 19 aa, synthetic construct
  REGION 1..19: note = Description of Artificial Sequence: Synthetic peptide
  MOD_RES 1: note = Nle
  MOD_RES 4: note = D-Phenylalanine
  MOD_RES 7: note = 5-aminopentanoic acid (HN-(CH2)4-C(O)
  MOD_RES 9: note = 8-amino-3,6-dioxaoctanoic acid
XCHFRWXCXRRRRRQRRRR

SEQ ID NO: 417 - protein, 22 aa, synthetic construct
  REGION 1..22: note = Description of Artificial Sequence: Synthetic peptide
  MOD_RES 1: note = Nle
  MOD_RES 4: note = D-Phenylalanine
  MOD_RES 7: note = 5-aminopentanoic acid (HN-(CH2)4-C(O)
  MOD_RES 9: note = 8-amino-3,6-dioxaoctanoic acid
  MOD_RES 10: note = 8-amino-3,6-dioxaoctanoic acid
XCHFRWXCXXYGRRRRRQRRRR

SEQ ID NO: 418 - protein, 20 aa, synthetic construct
  REGION 1..20: note = Description of Artificial Sequence: Synthetic peptide
  MOD_RES 1: note = Nle
  MOD_RES 4: note = D-Phenylalanine
  MOD_RES 7: note = 5-aminopentanoic acid (HN-(CH2)4-C(O)
  MOD_RES 9: note = 8-amino-3,6-dioxaoctanoic acid
  MOD_RES 10: note = 8-amino-3,6-dioxaoctanoic acid
XCHFRWXCXXRRRRRQRRRR

SEQ ID NO: 419 - protein, 20 aa, synthetic construct
  REGION 1..20: note = Description of Artificial Sequence: Synthetic peptide
  MOD_RES 1: note = Nle
  MOD_RES 3: note = D-Leucine
  MOD_RES 5: note = D-Phenylalanine
  MOD_RES 9: note = Beta-Alanine
XCLHFRWCAYGRRRRRQRRR

SEQ ID NO: 420 - protein, 18 aa, synthetic construct
  REGION 1..18: note = Description of Artificial Sequence: Synthetic peptide
  MOD_RES 1: note = Nle
  MOD_RES 3: note = D-Leucine
  MOD_RES 5: note = D-Phenylalanine
  MOD_RES 9: note = Beta-Alanine
XCLHFRWCARRRRRQRRR

SEQ ID NO: 421 - protein, 21 aa, synthetic construct
  REGION 1..21: note = Description of Artificial Sequence: Synthetic peptide
  MOD_RES 1: note = Nle
  MOD_RES 3: note = D-Leucine
  MOD_RES 5: note = D-Phenylalanine
  MOD_RES 9: note = Beta-Alanine
  MOD_RES 10: note = Beta-Alanine
XCLHFRWCAAYGRRRRRQRRR

SEQ ID NO: 422 - protein, 19 aa, synthetic construct
  REGION 1..19: note = Description of Artificial Sequence: Synthetic peptide
  MOD_RES 1: note = Nle
  MOD_RES 3: note = D-Leucine
  MOD_RES 5: note = D-Phenylalanine
  MOD_RES 9: note = Beta-Alanine
  MOD_RES 10: note = Beta-Alanine
XCLHFRWCAARRRRRQRRR

SEQ ID NO: 423 - protein, 20 aa, synthetic construct
  REGION 1..20: note = Description of Artificial Sequence: Synthetic peptide
  MOD_RES 1: note = Nle
  MOD_RES 3: note = D-Leucine
  MOD_RES 5: note = D-Phenylalanine
  MOD_RES 9: note = 8-amino-3,6-dioxaoctanoic acid
XCLHFRWCXYGRRRRRQRRR

SEQ ID NO: 424 - protein, 18 aa, synthetic construct
  REGION 1..18: note = Description of Artificial Sequence: Synthetic peptide
  MOD_RES 1: note = Nle
  MOD_RES 3: note = D-Leucine
  MOD_RES 5: note = D-Phenylalanine
  MOD_RES 9: note = 8-amino-3,6-dioxaoctanoic acid
XCLHFRWCXRRRRRQRRR

SEQ ID NO: 425 - protein, 21 aa, synthetic construct
  REGION 1..21: note = Description of Artificial Sequence: Synthetic peptide
  MOD_RES 1: note = Nle
  MOD_RES 3: note = D-Leucine
  MOD_RES 5: note = D-Phenylalanine
  MOD_RES 9: note = 8-amino-3,6-dioxaoctanoic acid
  MOD_RES 10: note = 8-amino-3,6-dioxaoctanoic acid
XCLHFRWCXXYGRRRRRQRRR

SEQ ID NO: 426 - protein, 19 aa, synthetic construct
  REGION 1..19: note = Description of Artificial Sequence: Synthetic peptide
  MOD_RES 1: note = Nle
  MOD_RES 3: note = D-Leucine
  MOD_RES 5: note = D-Phenylalanine
  MOD_RES 9: note = 8-amino-3,6-dioxaoctanoic acid
  MOD_RES 10: note = 8-amino-3,6-dioxaoctanoic acid
XCLHFRWCXXRRRRRQRRR

SEQ ID NO: 427 - protein, 21 aa, synthetic construct
  REGION 1..21: note = Description of Artificial Sequence: Synthetic peptide
  MOD_RES 1: note = Nle
  MOD_RES 3: note = D-Leucine
  MOD_RES 5: note = D-Phenylalanine
  MOD_RES 9: note = Beta-Alanine
XCLHFRWCAYGRRRRRQRRRR

SEQ ID NO: 428 - protein, 19 aa, synthetic construct
  REGION 1..19: note = Description of Artificial Sequence: Synthetic peptide
  MOD_RES 1: note = Nle
  MOD_RES 3: note = D-Leucine
  MOD_RES 5: note = D-Phenylalanine
  MOD_RES 9: note = Beta-Alanine
XCLHFRWCARRRRRQRRRR

SEQ ID NO: 429 - protein, 22 aa, synthetic construct
  REGION 1..22: note = Description of Artificial Sequence: Synthetic peptide
  MOD_RES 1: note = Nle
  MOD_RES 3: note = D-Leucine
  MOD_RES 5: note = D-Phenylalanine
  MOD_RES 9: note = Beta-Alanine
  MOD_RES 10: note = Beta-Alanine
XCLHFRWCAAYGRRRRRQRRRR

SEQ ID NO: 430 - protein, 20 aa, synthetic construct
  REGION 1..20: note = Description of Artificial Sequence: Synthetic peptide
  MOD_RES 1: note = Nle
  MOD_RES 3: note = D-Leucine
  MOD_RES 5: note = D-Phenylalanine
  MOD_RES 9: note = Beta-Alanine
  MOD_RES 10: note = Beta-Alanine
XCLHFRWCAARRRRRQRRRR

SEQ ID NO: 431 - protein, 21 aa, synthetic construct
  REGION 1..21: note = Description of Artificial Sequence: Synthetic peptide
  MOD_RES 1: note = Nle
  MOD_RES 3: note = D-Leucine
  MOD_RES 5: note = D-Phenylalanine
  MOD_RES 9: note = 8-amino-3,6-dioxaoctanoic acid
XCLHFRWCXYGRRRRRQRRRR

SEQ ID NO: 432 - protein, 19 aa, synthetic construct
  REGION 1..19: note = Description of Artificial Sequence: Synthetic peptide
  MOD_RES 1: note = Nle
  MOD_RES 3: note = D-Leucine
  MOD_RES 5: note = D-Phenylalanine
  MOD_RES 9: note = 8-amino-3,6-dioxaoctanoic acid
XCLHFRWCXRRRRRQRRRR

SEQ ID NO: 433 - protein, 22 aa, synthetic construct
  REGION 1..22: note = Description of Artificial Sequence: Synthetic peptide
  MOD_RES 1: note = Nle
  MOD_RES 3: note = D-Leucine
  MOD_RES 5: note = D-Phenylalanine
  MOD_RES 9: note = 8-amino-3,6-dioxaoctanoic acid
  MOD_RES 10: note = 8-amino-3,6-dioxaoctanoic acid
XCLHFRWCXXYGRRRRRQRRRR

SEQ ID NO: 434 - protein, 20 aa, synthetic construct
  REGION 1..20: note = Description of Artificial Sequence: Synthetic peptide
  MOD_RES 1: note = Nle
  MOD_RES 3: note = D-Leucine
  MOD_RES 5: note = D-Phenylalanine
  MOD_RES 9: note = 8-amino-3,6-dioxaoctanoic acid
  MOD_RES 10: note = 8-amino-3,6-dioxaoctanoic acid
XCLHFRWCXXRRRRRQRRRR

SEQ ID NO: 435 - protein, 20 aa, synthetic construct
  REGION 1..20: note = Description of Artificial Sequence: Synthetic peptide
  MOD_RES 1: note = Nle
  MOD_RES 3: note = D-beta-cyclohexylalanine
  MOD_RES 5: note = D-Phenylalanine
  MOD_RES 9: note = Beta-Alanine
XCXHFRWCAYGRRRRRQRRR

SEQ ID NO: 436 - protein, 18 aa, synthetic construct
  REGION 1..18: note = Description of Artificial Sequence: Synthetic peptide
  MOD_RES 1: note = Nle
  MOD_RES 3: note = D-beta-cyclohexylalanine
  MOD_RES 5: note = D-Phenylalanine
  MOD_RES 9: note = Beta-Alanine
XCXHFRWCARRRRRQRRR

SEQ ID NO: 437 - protein, 21 aa, synthetic construct
  REGION 1..21: note = Description of Artificial Sequence: Synthetic peptide
  MOD_RES 1: note = Nle
  MOD_RES 3: note = D-beta-cyclohexylalanine
  MOD_RES 5: note = D-Phenylalanine
  MOD_RES 9: note = Beta-Alanine
  MOD_RES 10: note = Beta-Alanine
XCXHFRWCAAYGRRRRRQRRR

SEQ ID NO: 438 - protein, 19 aa, synthetic construct
  REGION 1..19: note = Description of Artificial Sequence: Synthetic peptide
  MOD_RES 1: note = Nle
  MOD_RES 3: note = D-beta-cyclohexylalanine
  MOD_RES 5: note = D-Phenylalanine
  MOD_RES 9: note = Beta-Alanine
  MOD_RES 10: note = Beta-Alanine
XCXHFRWCAARRRRRQRRR

SEQ ID NO: 439 - protein, 20 aa, synthetic construct
  REGION 1..20: note = Description of Artificial Sequence: Synthetic peptide
  MOD_RES 1: note = Nle
  MOD_RES 3: note = D-beta-cyclohexylalanine
  MOD_RES 5: note = D-Phenylalanine
  MOD_RES 9: note = 8-amino-3,6-dioxaoctanoic acid
XCXHFRWCXYGRRRRRQRRR

SEQ ID NO: 440 - protein, 18 aa, synthetic construct
  REGION 1..18: note = Description of Artificial Sequence: Synthetic peptide
  MOD_RES 1: note = Nle
  MOD_RES 3: note = D-beta-cyclohexylalanine
  MOD_RES 5: note = D-Phenylalanine
  MOD_RES 9: note = 8-amino-3,6-dioxaoctanoic acid
XCXHFRWCXRRRRRQRRR

SEQ ID NO: 441 - protein, 21 aa, synthetic construct
  REGION 1..21: note = Description of Artificial Sequence: Synthetic peptide
  MOD_RES 1: note = Nle
  MOD_RES 3: note = D-beta-cyclohexylalanine
  MOD_RES 5: note = D-Phenylalanine
  MOD_RES 9: note = 8-amino-3,6-dioxaoctanoic acid
  MOD_RES 10: note = 8-amino-3,6-dioxaoctanoic acid
XCXHFRWCXXYGRRRRRQRRR

SEQ ID NO: 442 - protein, 19 aa, synthetic construct
  REGION 1..19: note = Description of Artificial Sequence: Synthetic peptide
  MOD_RES 1: note = Nle
  MOD_RES 3: note = D-beta-cyclohexylalanine
  MOD_RES 5: note = D-Phenylalanine
  MOD_RES 9: note = 8-amino-3,6-dioxaoctanoic acid
  MOD_RES 10: note = 8-amino-3,6-dioxaoctanoic acid
XCXHFRWCXXRRRRRQRRR

SEQ ID NO: 443 - protein, 21 aa, synthetic construct
  REGION 1..21: note = Description of Artificial Sequence: Synthetic peptide
  MOD_RES 1: note = Nle
  MOD_RES 3: note = D-beta-cyclohexylalanine
  MOD_RES 5: note = D-Phenylalanine
  MOD_RES 9: note = Beta-Alanine
XCXHFRWCAYGRRRRRQRRRR

SEQ ID NO: 444 - protein, 19 aa, synthetic construct
  REGION 1..19: note = Description of Artificial Sequence: Synthetic peptide
  MOD_RES 1: note = Nle
  MOD_RES 3: note = D-beta-cyclohexylalanine
  MOD_RES 5: note = D-Phenylalanine
  MOD_RES 9: note = Beta-Alanine
XCXHFRWCARRRRRQRRRR

SEQ ID NO: 445 - protein, 22 aa, synthetic construct
  REGION 1..22: note = Description of Artificial Sequence: Synthetic peptide
  MOD_RES 1: note = Nle
  MOD_RES 3: note = D-beta-cyclohexylalanine
  MOD_RES 5: note = D-Phenylalanine
  MOD_RES 9: note = Beta-Alanine
  MOD_RES 10: note = Beta-Alanine
XCXHFRWCAAYGRRRRRQRRRR

SEQ ID NO: 446 - protein, 20 aa, synthetic construct
  REGION 1..20: note = Description of Artificial Sequence: Synthetic peptide
  MOD_RES 1: note = Nle
  MOD_RES 3: note = D-beta-cyclohexylalanine
  MOD_RES 5: note = D-Phenylalanine
  MOD_RES 9: note = Beta-Alanine
  MOD_RES 10: note = Beta-Alanine
XCXHFRWCAARRRRRQRRRR

SEQ ID NO: 447 - protein, 21 aa, synthetic construct
  REGION 1..21: note = Description of Artificial Sequence: Synthetic peptide
  MOD_RES 1: note = Nle
  MOD_RES 3: note = D-beta-cyclohexylalanine
  MOD_RES 5: note = D-Phenylalanine
  MOD_RES 9: note = 8-amino-3,6-dioxaoctanoic acid
XCXHFRWCXYGRRRRRQRRRR

SEQ ID NO: 448 - protein, 19 aa, synthetic construct
  REGION 1..19: note = Description of Artificial Sequence: Synthetic peptide
  MOD_RES 1: note = Nle
  MOD_RES 3: note = D-beta-cyclohexylalanine
  MOD_RES 5: note = D-Phenylalanine
  MOD_RES 9: note = 8-amino-3,6-dioxaoctanoic acid
XCXHFRWCXRRRRRQRRRR

SEQ ID NO: 449 - protein, 22 aa, synthetic construct
  REGION 1..22: note = Description of Artificial Sequence: Synthetic peptide
  MOD_RES 1: note = Nle
  MOD_RES 3: note = D-beta-cyclohexylalanine
  MOD_RES 5: note = D-Phenylalanine
  MOD_RES 9: note = 8-amino-3,6-dioxaoctanoic acid
  MOD_RES 10: note = 8-amino-3,6-dioxaoctanoic acid
XCXHFRWCXXYGRRRRRQRRRR

SEQ ID NO: 450 - protein, 20 aa, synthetic construct
  REGION 1..20: note = Description of Artificial Sequence: Synthetic peptide
  MOD_RES 1: note = Nle
  MOD_RES 3: note = D-beta-cyclohexylalanine
  MOD_RES 5: note = D-Phenylalanine
  MOD_RES 9: note = 8-amino-3,6-dioxaoctanoic acid
  MOD_RES 10: note = 8-amino-3,6-dioxaoctanoic acid
XCXHFRWCXXRRRRRQRRRR

SEQ ID NO: 451 - protein, 20 aa, synthetic construct
  REGION 1..20: note = Description of Artificial Sequence: Synthetic peptide
  MOD_RES 1: note = Nle
  MOD_RES 4: note = D-Phenylalanine
  MOD_RES 7: note = 4-aminobutyric acid
  MOD_RES 9: note = Beta-Alanine
XCHFRWXCAYGRRRRRQRRR

SEQ ID NO: 452 - protein, 18 aa, synthetic construct
  REGION 1..18: note = Description of Artificial Sequence: Synthetic peptide
  MOD_RES 1: note = Nle
  MOD_RES 4: note = D-Phenylalanine
  MOD_RES 7: note = 4-aminobutyric acid
  MOD_RES 9: note = Beta-Alanine
XCHFRWXCARRRRRQRRR

SEQ ID NO: 453 - protein, 21 aa, synthetic construct
  REGION 1..21: note = Description of Artificial Sequence: Synthetic peptide
  MOD_RES 1: note = Nle
  MOD_RES 4: note = D-Phenylalanine
  MOD_RES 7: note = 4-aminobutyric acid
  MOD_RES 9: note = Beta-Alanine
  MOD_RES 10: note = Beta-Alanine
XCHFRWXCAAYGRRRRRQRRR

SEQ ID NO: 454 - protein, 19 aa, synthetic construct
  REGION 1..19: note = Description of Artificial Sequence: Synthetic peptide
  MOD_RES 1: note = Nle
  MOD_RES 4: note = D-Phenylalanine
  MOD_RES 7: note = 4-aminobutyric acid
  MOD_RES 9: note = Beta-Alanine
  MOD_RES 10: note = Beta-Alanine
XCHFRWXCAARRRRRQRRR

SEQ ID NO: 455 - protein, 21 aa, synthetic construct
  REGION 1..21: note = Description of Artificial Sequence: Synthetic peptide
  MOD_RES 1: note = Nle
  MOD_RES 4: note = D-Phenylalanine
  MOD_RES 7: note = 4-aminobutyric acid
  MOD_RES 9: note = Beta-Alanine
XCHFRWXCAYGRRRRRQRRRR

SEQ ID NO: 456 - protein, 19 aa, synthetic construct
  REGION 1..19: note = Description of Artificial Sequence: Synthetic peptide
  MOD_RES 1: note = Nle
  MOD_RES 4: note = D-Phenylalanine
  MOD_RES 7: note = 4-aminobutyric acid
  MOD_RES 9: note = Beta-Alanine
XCHFRWXCARRRRRQRRRR

SEQ ID NO: 457 - protein, 22 aa, synthetic construct
  REGION 1..22: note = Description of Artificial Sequence: Synthetic peptide
  MOD_RES 1: note = Nle
  MOD_RES 4: note = D-Phenylalanine
  MOD_RES 7: note = 4-aminobutyric acid
  MOD_RES 9: note = Beta-Alanine
  MOD_RES 10: note = Beta-Alanine
XCHFRWXCAAYGRRRRRQRRRR

SEQ ID NO: 458 - protein, 20 aa, synthetic construct
  REGION 1..20: note = Description of Artificial Sequence: Synthetic peptide
  MOD_RES 1: note = Nle
  MOD_RES 4: note = D-Phenylalanine
  MOD_RES 7: note = 4-aminobutyric acid
  MOD_RES 9: note = Beta-Alanine
  MOD_RES 10: note = Beta-Alanine
XCHFRWXCAARRRRRQRRRR

SEQ ID NO: 459 - protein, 20 aa, synthetic construct
  REGION 1..20: note = Description of Artificial Sequence: Synthetic peptide
  MOD_RES 1: note = Nle
  MOD_RES 4: note = D-Phenylalanine
  MOD_RES 7: note = 4-aminobutyric acid
  MOD_RES 9: note = 8-amino-3,6-dioxaoctanoic acid
XCHFRWXCXYGRRRRRQRRR

SEQ ID NO: 460 - protein, 18 aa, synthetic construct
  REGION 1..18: note = Description of Artificial Sequence: Synthetic peptide
  MOD_RES 1: note = Nle
  MOD_RES 4: note = D-Phenylalanine
  MOD_RES 7: note = 4-aminobutyric acid
  MOD_RES 9: note = 8-amino-3,6-dioxaoctanoic acid
XCHFRWXCXRRRRRQRRR

SEQ ID NO: 461 - protein, 21 aa, synthetic construct
  REGION 1..21: note = Description of Artificial Sequence: Synthetic peptide
  MOD_RES 1: note = Nle
  MOD_RES 4: note = D-Phenylalanine
  MOD_RES 7: note = 4-aminobutyric acid
  MOD_RES 9: note = 8-amino-3,6-dioxaoctanoic acid
  MOD_RES 10: note = 8-amino-3,6-dioxaoctanoic acid
XCHFRWXCXXYGRRRRRQRRR

SEQ ID NO: 462 - protein, 19 aa, synthetic construct
  REGION 1..19: note = Description of Artificial Sequence: Synthetic peptide
  MOD_RES 1: note = Nle
  MOD_RES 4: note = D-Phenylalanine
  MOD_RES 7: note = 4-aminobutyric acid
  MOD_RES 9: note = 8-amino-3,6-dioxaoctanoic acid
  MOD_RES 10: note = 8-amino-3,6-dioxaoctanoic acid
XCHFRWXCXXRRRRRQRRR

SEQ ID NO: 463 - protein, 21 aa, synthetic construct
  REGION 1..21: note = Description of Artificial Sequence: Synthetic peptide
  MOD_RES 1: note = Nle
  MOD_RES 4: note = D-Phenylalanine
  MOD_RES 7: note = 4-aminobutyric acid
  MOD_RES 9: note = 8-amino-3,6-dioxaoctanoic acid
XCHFRWXCXYGRRRRRQRRRR

SEQ ID NO: 464 - protein, 19 aa, synthetic construct
  REGION 1..19: note = Description of Artificial Sequence: Synthetic peptide
  MOD_RES 1: note = Nle
  MOD_RES 4: note = D-Phenylalanine
  MOD_RES 7: note = 4-aminobutyric acid
  MOD_RES 9: note = 8-amino-3,6-dioxaoctanoic acid
XCHFRWXCXRRRRRQRRRR

SEQ ID NO: 465 - protein, 22 aa, synthetic construct
  REGION 1..22: note = Description of Artificial Sequence: Synthetic peptide
  MOD_RES 1: note = Nle
  MOD_RES 4: note = D-Phenylalanine
  MOD_RES 7: note = 4-aminobutyric acid
  MOD_RES 9: note = 8-amino-3,6-dioxaoctanoic acid
  MOD_RES 10: note = 8-amino-3,6-dioxaoctanoic acid
XCHFRWXCXXYGRRRRRQRRRR

SEQ ID NO: 466 - protein, 20 aa, synthetic construct
  REGION 1..20: note = Description of Artificial Sequence: Synthetic peptide
  MOD_RES 1: note = Nle
  MOD_RES 4: note = D-Phenylalanine
  MOD_RES 7: note = 4-aminobutyric acid
  MOD_RES 9: note = 8-amino-3,6-dioxaoctanoic acid
  MOD_RES 10: note = 8-amino-3,6-dioxaoctanoic acid
XCHFRWXCXXRRRRRQRRRR

SEQ ID NO: 467 - protein, 12 aa, synthetic construct
  REGION 1..12: note = Description of Artificial Sequence: Synthetic peptide
  MOD_RES 4: note = D-4-bromo-phenylalanine
CEHFRWGCPPKD

SEQ ID NO: 468 - protein, 12 aa, synthetic construct
  REGION 1..12: note = Description of Artificial Sequence: Synthetic peptide
  MOD_RES 4: note = D-Beta-(2-naphthyl)alanine
CEHXRWACPPKD

SEQ ID NO: 469 - protein, 12 aa, synthetic construct
  REGION 1..12: note = Description of Artificial Sequence: Synthetic peptide
  MOD_RES 4: note = D-Beta-(2-naphthyl)alanine
  MOD_RES 6: note = Beta-(2-naphthyl)alanine
CEHXRXACPPKD

SEQ ID NO: 470 - protein, 12 aa, synthetic construct
  REGION 1..12: note = Description of Artificial Sequence: Synthetic peptide
  MOD_RES 4: note = D-Beta-(2-naphthyl)alanine
  MOD_RES 6: note = Beta-(1-naphthyl)alanine
CEHXRXACPPKD

SEQ ID NO: 471 - protein, 12 aa, synthetic construct
  REGION 1..12: note = Description of Artificial Sequence: Synthetic peptide
  MOD_RES 4: note = D-Beta-(2-naphthyl)alanine
  MOD_RES 6: note = 3-benzothienylalanine
CEHXRXACPPKD

SEQ ID NO: 472 - protein, 12 aa, synthetic construct
  REGION 1..12: note = Description of Artificial Sequence: Synthetic peptide
  MOD_RES 4: note = D-Beta-(2-naphthyl)alanine
  MOD_RES 6: note = Beta-(2-naphthyl)alanine
  MOD_RES 7: note = Beta-Alanine
CEHXRXACPPKD

SEQ ID NO: 473 - protein, 12 aa, synthetic construct
  REGION 1..12: note = Description of Artificial Sequence: Synthetic peptide
  MOD_RES 4: note = D-Beta-(2-naphthyl)alanine
  MOD_RES 6: note = Beta-(2-naphthyl)alanine
  MOD_RES 7: note = alpha-aminoisobutyric acid
CEHXRXXCPPKD

SEQ ID NO: 474 - protein, 7 aa, synthetic construct
  REGION 1..7: note = Description of Artificial Sequence: Synthetic peptide
  MOD_RES 2: note = D-Alanine
  MOD_RES 4: note = D-Phenylalanine
CAHFRWC

SEQ ID NO: 475 - protein, 7 aa, synthetic construct
  REGION 1..7: note = Description of Artificial Sequence: Synthetic peptide
  MOD_RES 2: note = D-Alanine
  MOD_RES 4: note = D-Phenylalanine
CAHFRWC

SEQ ID NO: 476 - protein, 7 aa, synthetic construct
  REGION 1..7: note = Description of Artificial Sequence: Synthetic peptide
  MOD_RES 2: note = D-Alanine
  MOD_RES 4: note = D-Beta-(2-naphthyl)alanine
CAHXRWC

SEQ ID NO: 477 - protein, 7 aa, synthetic construct
  REGION 1..7: note = Description of Artificial Sequence: Synthetic peptide
  MOD_RES 2: note = D-Alanine
  MOD_RES 4: note = D-Beta-(2-naphthyl)alanine
CAHXRWC

SEQ ID NO: 478 - protein, 7 aa, synthetic construct
  REGION 1..7: note = Description of Artificial Sequence: Synthetic peptide
  MOD_RES 2: note = D-Alanine
  MOD_RES 4: note = D-Phenylalanine
DAHFRWK

SEQ ID NO: 479 - protein, 7 aa, synthetic construct
  REGION 1..7: note = Description of Artificial Sequence: Synthetic peptide
  MOD_RES 2: note = D-Alanine
  MOD_RES 4: note = D-Phenylalanine
  MOD_RES 7: note = Ornithine
DAHFRWX

SEQ ID NO: 480 - protein, 7 aa, synthetic construct
  REGION 1..7: note = Description of Artificial Sequence: Synthetic peptide
  MOD_RES 2: note = D-Alanine
  MOD_RES 4: note = D-Phenylalanine
  MOD_RES 7: note = 2,4-diaminobutyric acid
DAHFRWX

SEQ ID NO: 481 - protein, 7 aa, synthetic construct
  REGION 1..7: note = Description of Artificial Sequence: Synthetic peptide
  MOD_RES 2: note = D-Alanine
  MOD_RES 4: note = D-Phenylalanine
  MOD_RES 7: note = 2,3-diaminopropionic acid
DAHFRWX

SEQ ID NO: 482 - protein, 6 aa, synthetic construct
  REGION 1..6: note = Description of Artificial Sequence: Synthetic peptide
  MOD_RES 3: note = D-Beta-(2-naphthyl)alanine
DHXRWK

SEQ ID NO: 483 - protein, 6 aa, synthetic construct
  REGION 1..6: note = Description of Artificial Sequence: Synthetic peptide
  MOD_RES 3: note = D-Phenylalanine
DHFRWK

SEQ ID NO: 484 - protein, 6 aa, synthetic construct
  REGION 1..6: note = Description of Artificial Sequence: Synthetic peptide
  MOD_RES 2: note = 1-amino-1 cyclopropanecarboxylic acid
  MOD_RES 3: note = D-Phenylalanine
DXFRWK

SEQ ID NO: 485 - protein, 6 aa, synthetic construct
  REGION 1..6: note = Description of Artificial Sequence: Synthetic peptide
  MOD_RES 2: note = 1-amino-1-cyclopentanecarboxylic acid
  MOD_RES 3: note = D-Phenylalanine
DXFRWK

SEQ ID NO: 486 - protein, 6 aa, synthetic construct
  REGION 1..6: note = Description of Artificial Sequence: Synthetic peptide
  MOD_RES 2: note = 1-amino-1-cyclohexanecarboxylic acid
  MOD_RES 3: note = D-Phenylalanine
DXFRWK

SEQ ID NO: 487 - protein, 6 aa, synthetic construct
  REGION 1..6: note = Description of Artificial Sequence: Synthetic peptide
  MOD_RES 2: note = 1-amino-1 cyclopropanecarboxylic acid
  MOD_RES 3: note = D-Beta-(2-naphthyl)alanine
DXXRWK

SEQ ID NO: 488 - protein, 6 aa, synthetic construct
  REGION 1..6: note = Description of Artificial Sequence: Synthetic peptide
  MOD_RES 2: note = 1-amino-1-cyclopentanecarboxylic acid
  MOD_RES 3: note = D-Beta-(2-naphthyl)alanine
DXXRWK

SEQ ID NO: 489 - protein, 6 aa, synthetic construct
  REGION 1..6: note = Description of Artificial Sequence: Synthetic peptide
  MOD_RES 2: note = 1-amino-1-cyclohexanecarboxylic acid
  MOD_RES 3: note = D-Beta-(2-naphthyl)alanine
DXXRWK

SEQ ID NO: 490 - protein, 6 aa, synthetic construct
  REGION 1..6: note = Description of Artificial Sequence: Synthetic peptide
  MOD_RES 2: note = 2-aminoindan-2-carboxylic acid
  MOD_RES 3: note = D-Phenylalanine
DXFRWK

SEQ ID NO: 491 - protein, 6 aa, synthetic construct
  REGION 1..6: note = Description of Artificial Sequence: Synthetic peptide
  MOD_RES 2: note = 4-amino-piperidine-4-carboxylic acid
  MOD_RES 3: note = D-Phenylalanine
DXFRWK

SEQ ID NO: 492 - protein, 6 aa, synthetic construct
  REGION 1..6: note = Description of Artificial Sequence: Synthetic peptide
  MOD_RES 2: note = 2-aminoindan-2-carboxylic acid
  MOD_RES 3: note = D-Beta-(2-naphthyl)alanine
DXXRWK

SEQ ID NO: 493 - protein, 6 aa, synthetic construct
  REGION 1..6: note = Description of Artificial Sequence: Synthetic peptide
  MOD_RES 2: note = 4-amino-piperidine-4-carboxylic acid
  MOD_RES 3: note = D-Beta-(2-naphthyl)alanine
DXXRWK

SEQ ID NO: 494 - protein, 7 aa, synthetic construct
  REGION 1..7: note = Description of Artificial Sequence: Synthetic peptide
  MOD_RES 2: note = D-Alanine
  MOD_RES 4: note = D-Phenylalanine
  MOD_RES 7: note = Ornithine
EAHFRWX

SEQ ID NO: 495 - protein, 7 aa, synthetic construct
  REGION 1..7: note = Description of Artificial Sequence: Synthetic peptide
  MOD_RES 2: note = D-Alanine
  MOD_RES 4: note = D-Phenylalanine
  MOD_RES 7: note = 2,4-diaminobutyric acid
EAHFRWX

SEQ ID NO: 496 - protein, 7 aa, synthetic construct
  REGION 1..7: note = Description of Artificial Sequence: Synthetic peptide
  MOD_RES 2: note = D-Alanine
  MOD_RES 4: note = D-Phenylalanine
  MOD_RES 7: note = 2,3-diaminopropionic acid
EAHFRWX

SEQ ID NO: 497 - protein, 7 aa, synthetic construct
  REGION 1..7: note = Description of Artificial Sequence: Synthetic peptide
  MOD_RES 2: note = D-Alanine
  MOD_RES 4: note = D-Phenylalanine
EAHFRWK

SEQ ID NO: 498 - protein, 6 aa, synthetic construct
  REGION 1..6: note = Description of Artificial Sequence: Synthetic peptide
  MOD_RES 3: note = D-Phenylalanine
  MOD_RES 6: note = 2,3-diaminopropionic acid
EHFRWX

SEQ ID NO: 499 - protein, 6 aa, synthetic construct
  REGION 1..6: note = Description of Artificial Sequence: Synthetic peptide
  MOD_RES 3: note = D-Phenylalanine
EHFRWK

SEQ ID NO: 500 - protein, 9 aa, synthetic construct
  REGION 1..9: note = Description of Artificial Sequence: Synthetic peptide
  MOD_RES 6: note = D-Phenylalanine
RGCEHFRWC

SEQ ID NO: 501 - protein, 9 aa, synthetic construct
  REGION 1..9: note = Description of Artificial Sequence: Synthetic peptide
  MOD_RES 1: note = Nle
  MOD_RES 6: note = D-Phenylalanine
XGCEHFRWC

SEQ ID NO: 502 - protein, 9 aa, synthetic construct
  REGION 1..9: note = Description of Artificial Sequence: Synthetic peptide
  MOD_RES 6: note = D-Phenylalanine
GGCEHFRWC

SEQ ID NO: 503 - protein, 9 aa, synthetic construct
  REGION 1..9: note = Description of Artificial Sequence: Synthetic peptide
  MOD_RES 1: note = Nle
  MOD_RES 4: note = D-Alanine
  MOD_RES 6: note = D-Phenylalanine
XGCAHFRWC

SEQ ID NO: 504 - protein, 9 aa, synthetic construct
  REGION 1..9: note = Description of Artificial Sequence: Synthetic peptide
  MOD_RES 4: note = D-Alanine
  MOD_RES 6: note = D-Phenylalanine
GGCAHFRWC

SEQ ID NO: 505 - protein, 9 aa, synthetic construct
  REGION 1..9: note = Description of Artificial Sequence: Synthetic peptide
  MOD_RES 1: note = Nle
  MOD_RES 4: note = D-Alanine
  MOD_RES 6: note = D-Phenylalanine
  MOD_RES 9: note = Penicillamine
XGCAHFRWX

SEQ ID NO: 506 - protein, 9 aa, synthetic construct
  REGION 1..9: note = Description of Artificial Sequence: Synthetic peptide
  MOD_RES 4: note = D-Alanine
  MOD_RES 6: note = D-Phenylalanine
  MOD_RES 9: note = Penicillamine
GGCAHFRWX

SEQ ID NO: 507 - protein, 9 aa, synthetic construct
  REGION 1..9: note = Description of Artificial Sequence: Synthetic peptide
  MOD_RES 4: note = D-Alanine
  MOD_RES 6: note = D-Phenylalanine
AGCAHFRWC

SEQ ID NO: 508 - protein, 9 aa, synthetic construct
  REGION 1..9: note = Description of Artificial Sequence: Synthetic peptide
  MOD_RES 1: note = D-Alanine
  MOD_RES 4: note = D-Alanine
  MOD_RES 6: note = D-Phenylalanine
AGCAHFRWC

SEQ ID NO: 509 - protein, 9 aa, synthetic construct
  REGION 1..9: note = Description of Artificial Sequence: Synthetic peptide
  MOD_RES 1: note = alpha-aminoisobutyric acid
  MOD_RES 4: note = D-Alanine
  MOD_RES 6: note = D-Phenylalanine
XGCAHFRWC

SEQ ID NO: 510 - protein, 9 aa, synthetic construct
  REGION 1..9: note = Description of Artificial Sequence: Synthetic peptide
  MOD_RES 4: note = D-Alanine
  MOD_RES 6: note = D-Phenylalanine
VGCAHFRWC

SEQ ID NO: 511 - protein, 9 aa, synthetic construct
  REGION 1..9: note = Description of Artificial Sequence: Synthetic peptide
  MOD_RES 4: note = D-Alanine
  MOD_RES 6: note = D-Phenylalanine
IGCAHFRWC

SEQ ID NO: 512 - protein, 9 aa, synthetic construct
  REGION 1..9: note = Description of Artificial Sequence: Synthetic peptide
  MOD_RES 4: note = D-Alanine
  MOD_RES 6: note = D-Phenylalanine
LGCAHFRWC

SEQ ID NO: 513 - protein, 9 aa, synthetic construct
  REGION 1..9: note = Description of Artificial Sequence: Synthetic peptide
  MOD_RES 6: note = D-Beta-(2-naphthyl)alanine
GGCEHXRWC

SEQ ID NO: 514 - protein, 9 aa, synthetic construct
  REGION 1..9: note = Description of Artificial Sequence: Synthetic peptide
  MOD_RES 1: note = Nle
  MOD_RES 6: note = D-Beta-(2-naphthyl)alanine
XGCEHXRWC

SEQ ID NO: 515 - protein, 9 aa, synthetic construct
  REGION 1..9: note = Description of Artificial Sequence: Synthetic peptide
  MOD_RES 1: note = D-Arginine
  MOD_RES 6: note = D-Phenylalanine
RGCEHFRWC

SEQ ID NO: 516 - protein, 9 aa, synthetic construct
  REGION 1..9: note = Description of Artificial Sequence: Synthetic peptide
  MOD_RES 1: note = D-Arginine
  MOD_RES 4: note = D-Alanine
  MOD_RES 6: note = D-Phenylalanine
RGCAHFRWC

SEQ ID NO: 517 - protein, 9 aa, synthetic construct
  REGION 1..9: note = Description of Artificial Sequence: Synthetic peptide
  MOD_RES 4: note = D-Alanine
  MOD_RES 6: note = D-Phenylalanine
RGCAHFRWC

SEQ ID NO: 518 - protein, 9 aa, synthetic construct
  REGION 1..9: note = Description of Artificial Sequence: Synthetic peptide
  MOD_RES 1: note = D-Arginine
  MOD_RES 4: note = D-Alanine
  MOD_RES 6: note = D-Beta-(2-naphthyl)alanine
RGCAHXRWC

SEQ ID NO: 519 - protein, 9 aa, synthetic construct
  REGION 1..9: note = Description of Artificial Sequence: Synthetic peptide
  MOD_RES 4: note = D-Alanine
  MOD_RES 6: note = D-Beta-(2-naphthyl)alanine
RGCAHXRWC

SEQ ID NO: 520 - protein, 9 aa, synthetic construct
  REGION 1..9: note = Description of Artificial Sequence: Synthetic peptide
  MOD_RES 2: note = Nle
  MOD_RES 6: note = D-Phenylalanine
AXCEHFRWC

SEQ ID NO: 521 - protein, 9 aa, synthetic construct
  REGION 1..9: note = Description of Artificial Sequence: Synthetic peptide
  MOD_RES 2: note = Nle
  MOD_RES 6: note = D-Phenylalanine
VXCEHFRWC

SEQ ID NO: 522 - protein, 9 aa, synthetic construct
  REGION 1..9: note = Description of Artificial Sequence: Synthetic peptide
  MOD_RES 2: note = Nle
  MOD_RES 6: note = D-Phenylalanine
GXCEHFRWC

SEQ ID NO: 523 - protein, 9 aa, synthetic construct
  REGION 1..9: note = Description of Artificial Sequence: Synthetic peptide
  MOD_RES 1: note = 1-amino-1-cyclohexanecarboxylic acid
  MOD_RES 2: note = Nle
  MOD_RES 4: note = D-Alanine
  MOD_RES 6: note = D-Phenylalanine
XXCAHFRWC

SEQ ID NO: 524 - protein, 9 aa, synthetic construct
  REGION 1..9: note = Description of Artificial Sequence: Synthetic peptide
  MOD_RES 2: note = Nle
  MOD_RES 4: note = D-Alanine
  MOD_RES 6: note = D-Phenylalanine
GXCAHFRWC

SEQ ID NO: 525 - protein, 9 aa, synthetic construct
  REGION 1..9: note = Description of Artificial Sequence: Synthetic peptide
  MOD_RES 2: note = Nle
  MOD_RES 4: note = D-Alanine
  MOD_RES 6: note = D-Phenylalanine
AXCAHFRWC

SEQ ID NO: 526 - protein, 9 aa, synthetic construct
  REGION 1..9: note = Description of Artificial Sequence: Synthetic peptide
  MOD_RES 1: note = D-Alanine
  MOD_RES 2: note = Nle
  MOD_RES 4: note = D-Alanine
  MOD_RES 6: note = D-Phenylalanine
AXCAHFRWC

SEQ ID NO: 527 - protein, 9 aa, synthetic construct
  REGION 1..9: note = Description of Artificial Sequence: Synthetic peptide
  MOD_RES 2: note = Nle
  MOD_RES 4: note = D-Alanine
  MOD_RES 6: note = D-Phenylalanine
VXCAHFRWC

SEQ ID NO: 528 - protein, 9 aa, synthetic construct
  REGION 1..9: note = Description of Artificial Sequence: Synthetic peptide
  MOD_RES 2: note = Nle
  MOD_RES 4: note = D-Alanine
  MOD_RES 6: note = D-Phenylalanine
LXCAHFRWC

SEQ ID NO: 529 - protein, 9 aa, synthetic construct
  REGION 1..9: note = Description of Artificial Sequence: Synthetic peptide
  MOD_RES 1: note = beta-cyclohexylalanine
  MOD_RES 2: note = Nle
  MOD_RES 4: note = D-Alanine
  MOD_RES 6: note = D-Phenylalanine
XXCAHFRWC

SEQ ID NO: 530 - protein, 9 aa, synthetic construct
  REGION 1..9: note = Description of Artificial Sequence: Synthetic peptide
  MOD_RES 1: note = alpha-aminoisobutyric acid
  MOD_RES 2: note = Nle
  MOD_RES 4: note = D-Alanine
  MOD_RES 6: note = D-Phenylalanine
XXCAHFRWC

SEQ ID NO: 531 - protein, 9 aa, synthetic construct
  REGION 1..9: note = Description of Artificial Sequence: Synthetic peptide
  MOD_RES 6: note = D-Phenylalanine
GRCEHFRWC

SEQ ID NO: 532 - protein, 9 aa, synthetic construct
  REGION 1..9: note = Description of Artificial Sequence: Synthetic peptide
  MOD_RES 6: note = D-Beta-(2-naphthyl)alanine
GRCEHXRWC

SEQ ID NO: 533 - protein, 9 aa, synthetic construct
  REGION 1..9: note = Description of Artificial Sequence: Synthetic peptide
  MOD_RES 4: note = D-Alanine
  MOD_RES 6: note = D-Phenylalanine
GRCAHFRWC

SEQ ID NO: 534 - protein, 9 aa, synthetic construct
  REGION 1..9: note = Description of Artificial Sequence: Synthetic peptide
  MOD_RES 4: note = D-Alanine
  MOD_RES 6: note = D-Beta-(2-naphthyl)alanine
GRCAHXRWC

SEQ ID NO: 535 - protein, 9 aa, synthetic construct
  REGION 1..9: note = Description of Artificial Sequence: Synthetic peptide
  MOD_RES 2: note = D-Arginine
  MOD_RES 6: note = D-Phenylalanine
GRCEHFRWC

SEQ ID NO: 536 - protein, 9 aa, synthetic construct
  REGION 1..9: note = Description of Artificial Sequence: Synthetic peptide
  MOD_RES 2: note = D-Arginine
  MOD_RES 4: note = D-Alanine
  MOD_RES 6: note = D-Phenylalanine
GRCAHFRWC

SEQ ID NO: 537 - protein, 9 aa, synthetic construct
  REGION 1..9: note = Description of Artificial Sequence: Synthetic peptide
  MOD_RES 2: note = D-Arginine
  MOD_RES 4: note = D-Alanine
  MOD_RES 6: note = D-Beta-(2-naphthyl)alanine
GRCAHXRWC

SEQ ID NO: 538 - protein, 9 aa, synthetic construct
  REGION 1..9: note = Description of Artificial Sequence: Synthetic peptide
  MOD_RES 1: note = Nle
  MOD_RES 6: note = D-Phenylalanine
XACEHFRWC

SEQ ID NO: 539 - protein, 8 aa, synthetic construct
  REGION 1..8: note = Description of Artificial Sequence: Synthetic peptide
  MOD_RES 1: note = Nle
  MOD_RES 3: note = D-Alanine
  MOD_RES 5: note = D-Phenylalanine
XCAHFRWC

SEQ ID NO: 540 - protein, 8 aa, synthetic construct
  REGION 1..8: note = Description of Artificial Sequence: Synthetic peptide
  MOD_RES 3: note = D-Alanine
  MOD_RES 5: note = D-Phenylalanine
ACAHFRWC

SEQ ID NO: 541 - protein, 8 aa, synthetic construct
  REGION 1..8: note = Description of Artificial Sequence: Synthetic peptide
  MOD_RES 1: note = D-Alanine
  MOD_RES 3: note = D-Alanine
  MOD_RES 5: note = D-Phenylalanine
ACAHFRWC

SEQ ID NO: 542 - protein, 8 aa, synthetic construct
  REGION 1..8: note = Description of Artificial Sequence: Synthetic peptide
  MOD_RES 1: note = alpha-aminoisobutyric acid
  MOD_RES 3: note = D-Alanine
  MOD_RES 5: note = D-Phenylalanine
XCAHFRWC

SEQ ID NO: 543 - protein, 8 aa, synthetic construct
  REGION 1..8: note = Description of Artificial Sequence: Synthetic peptide
  MOD_RES 3: note = D-Alanine
  MOD_RES 5: note = D-Phenylalanine
VCAHFRWC

SEQ ID NO: 544 - protein, 8 aa, synthetic construct
  REGION 1..8: note = Description of Artificial Sequence: Synthetic peptide
  MOD_RES 1: note = alpha-aminobutyric acid
  MOD_RES 3: note = D-Alanine
  MOD_RES 5: note = D-Phenylalanine
XCAHFRWC

SEQ ID NO: 545 - protein, 8 aa, synthetic construct
  REGION 1..8: note = Description of Artificial Sequence: Synthetic peptide
  MOD_RES 3: note = D-Alanine
  MOD_RES 5: note = D-Phenylalanine
LCAHFRWC

SEQ ID NO: 546 - protein, 8 aa, synthetic construct
  REGION 1..8: note = Description of Artificial Sequence: Synthetic peptide
  MOD_RES 3: note = D-Alanine
  MOD_RES 5: note = D-Phenylalanine
ICAHFRWC

SEQ ID NO: 547 - protein, 8 aa, synthetic construct
  REGION 1..8: note = Description of Artificial Sequence: Synthetic peptide
  MOD_RES 1: note = beta-cyclohexylalanine
  MOD_RES 3: note = D-Alanine
  MOD_RES 5: note = D-Phenylalanine
XCAHFRWC

SEQ ID NO: 548 - protein, 8 aa, synthetic construct
  REGION 1..8: note = Description of Artificial Sequence: Synthetic peptide
  MOD_RES 1: note = 1-amino-1-cyclohexanecarboxylic acid
  MOD_RES 3: note = D-Alanine
  MOD_RES 5: note = D-Phenylalanine
XCAHFRWC

SEQ ID NO: 549 - protein, 8 aa, synthetic construct
  REGION 1..8: note = Description of Artificial Sequence: Synthetic peptide
  MOD_RES 3: note = D-Alanine
  MOD_RES 5: note = D-Phenylalanine
FCAHFRWC

SEQ ID NO: 550 - protein, 8 aa, synthetic construct
  REGION 1..8: note = Description of Artificial Sequence: Synthetic peptide
  MOD_RES 3: note = D-Alanine
  MOD_RES 5: note = D-Phenylalanine
GCAHFRWC

SEQ ID NO: 551 - protein, 8 aa, synthetic construct
  REGION 1..8: note = Description of Artificial Sequence: Synthetic peptide
  MOD_RES 5: note = D-Phenylalanine
GCEHFRWC

SEQ ID NO: 552 - protein, 9 aa, synthetic construct
  REGION 1..9: note = Description of Artificial Sequence: Synthetic peptide
  MOD_RES 4: note = D-Alanine
  MOD_RES 6: note = D-Phenylalanine
YRCAHFRWC

SEQ ID NO: 553 - protein, 9 aa, synthetic construct
  REGION 1..9: note = Description of Artificial Sequence: Synthetic peptide
  MOD_RES 1: note = Beta-(2-naphthyl)alanine
  MOD_RES 4: note = D-Alanine
  MOD_RES 6: note = D-Phenylalanine
XRCAHFRWC

SEQ ID NO: 554 - protein, 9 aa, synthetic construct
  REGION 1..9: note = Description of Artificial Sequence: Synthetic peptide
  MOD_RES 1: note = Beta-(1-naphthyl)alanine
  MOD_RES 4: note = D-Alanine
  MOD_RES 6: note = D-Phenylalanine
XRCAHFRWC

SEQ ID NO: 555 - protein, 9 aa, synthetic construct
  REGION 1..9: note = Description of Artificial Sequence: Synthetic peptide
  MOD_RES 4: note = D-Alanine
  MOD_RES 6: note = D-Phenylalanine
FRCAHFRWC

SEQ ID NO: 556 - protein, 9 aa, synthetic construct
  REGION 1..9: note = Description of Artificial Sequence: Synthetic peptide
  MOD_RES 4: note = D-Alanine
  MOD_RES 6: note = D-Phenylalanine
WRCAHFRWC

SEQ ID NO: 557 - protein, 9 aa, synthetic construct
  REGION 1..9: note = Description of Artificial Sequence: Synthetic peptide
  MOD_RES 1: note = (S)-pentafluorophenylalanine
  MOD_RES 4: note = D-Alanine
  MOD_RES 6: note = D-Phenylalanine
XRCAHFRWC

SEQ ID NO: 558 - protein, 9 aa, synthetic construct
  REGION 1..9: note = Description of Artificial Sequence: Synthetic peptide
  MOD_RES 4: note = D-Alanine
  MOD_RES 6: note = D-Phenylalanine
HRCAHFRWC

SEQ ID NO: 559 - protein, 9 aa, synthetic construct
  REGION 1..9: note = Description of Artificial Sequence: Synthetic peptide
  MOD_RES 4: note = D-Alanine
  MOD_RES 6: note = D-Phenylalanine
HRCAHFRWC

SEQ ID NO: 560-561 - skipped (2 entries)

SEQ ID NO: 562 - protein, 7 aa, synthetic construct
  REGION 1..7: note = Description of Artificial Sequence: Synthetic peptide
  MOD_RES 1: note = Nle
  MOD_RES 4: note = D-Phenylalanine
XDHFRWK

SEQ ID NO: 563 - protein, 267 aa, Homo sapiens
MPRSCCSRSGALLLALLLQASMEVRGWCLESSQCQDLTTESNLLECIRACKPDLSAETPMFPGNGDEQPLTENPRKYVMGHFRWDRFGRRNSSSSGSSGAGQKREDVSAGEDCGPLPEGGPEPRSDGAKPGPREGKRSYSMEHFRWGKPVGKKRRPVKVYPNGAEDESAEAFPLEFKRELTGQRLREGDGPDGPADDGAGAQADLEHSLLVAAEKKDEGPYRMEHFRWGSPPKDKRYGGFMTSEKSQTPLVTLFKNAIIKNAYKKGE

SEQ ID NO: 564 - DNA, 8658 bp, Homo sapiens
  source 1..8658: mol_type = genomic DNA
ctgctcttcacagcatcaccctctccccatttaatggtttaggttaacaggactttttccttgaggcttgggacacggaagggagcctcccctaaaccaggcccttggagagcaggccccaggggagcagtgcaactcaccttcacacccacaagacggctcctgacttctgctccctcctcccctccccaaagtggaacagagagaatatgattccccacgacttccacatcacagtttccaaacaatggggaaatcggaggcctccccgtgtgcagacggtgatatttaccgccaaatgcgaaccaggcagatgccagccccagcacgcacgcaggtaacttcaccctcgcctcaacgacctcagaggctgcccggcctgccccacacgggggtgctaagcctcccgcccgttctaagcggagacccaacgccatccataattaagttcttcctgagggcgagcggccaggtgcgccttcggcaggacagtgctaattccagcccctttccagcgcgtctccccgcgctcgtcccccgtctggaagcccccctcccacgccccgcggccccccttcccctggcccggggagctgctccttgtgctgccgggaaggtcaaagtcccgcgcccaccaggagagctcggcaagtatataaggacagaggagcgcgggaccaagcggcggcgaaggaggggaagaagagccgcgaccgagagaggccgccgagcgtccccgccctcagagagcagcctcccgagacaggtaagggcgcagcgtgggggacccgtgctctttccccgggatcccctgtccccgtcctcgcgatgcagtcggccggctccggctccgaaggcggacctgggcgcctctggctctccgcggtcccgagttctcgacaaactttctgcgccgactgcggcatgagaagccgccagtagctgagctggagggcccacgtccggcccctgggcggacggccgcgaagctgcaggcgctgtctccagggagccggcggcctcctctcccccaggggctcgcggcggtccggaggctccgagagcttgctaggaggtcttgggacaacccggtctttttttttttttttgagacggagtttcgctcttgttgcccatgctggagagcaaaggggtgatctctgctcaccgcaaccttcgcctcccgggttcaagcgattctcctgcttcagcctcccgagtagctgggattacaggcatgcgccaccacgcccggctaatttttgtatttttagtagtgacggagtttctccatgttggtcaggctggtctcaaactcccgacaacaggtgatccgcccgccttggccccccaaagttctggcattacaggcgcgagccaccgcccccggccagcccggtcttttagtatctcttgctcccagtttccaggataggtgtcacatcttgaaagtcaaattccatacacgctatcgcaaattaatgttggaaacggggcagcagagaaaaggataaaagtcataatgaacgccctgccttccggattttttcggattcagacccctgaatccttgtttccttgcccaccttagcgcacccgaggtggccgcgctatgataattacatgataactgggtcaattacaatgcagaatagttgggtctcttctctccaagacctagctggggttaaaaacaggtggccggggcgggagctgtcctagatcctgaaacgcactgtctagtttcggatgccctcaacagaaccggggtggacggtttatggcgcagatcctgggttgagggcacgggcagccatttggaatgatcaaggctcaggtaaggggcgtttccagcgaaggagagacagtccacttggcatttggattccccaaattcttcatgtttaaatggggcagggagggttcttacagaatggctggaaggagccaaggaaaataaaagtgtgtgtggattttttttgtgtgtgtgtcagtttataaactctgcacagattatggccactttaatgacttactgttcctttgatgcttttgttataggactcgatgcatgtatgtcatggtgtaaggacaaaactcggcccctgtgctcctctaatctttacaaaaggtcatggccagcgtgcagttttacagtaacaagcaaaatgatttgttgagctcatagagagcccctcacacctatgaagttctaataagtgtagttctactataaagttaatctcaggatgagcaaatttcaagtttctatttttccagagctttccatttttggattataatactttccctacttaaaaaagcacaacatttgatatttccccaataatttgttgctttaaaaatgacacaaaaggtactatttgttcattgtagagaactgaaaatacacataagcaaatacacatacacataagcaaaatatacaatacaaacacaagaccatctttcagggaagaatctgaagttttagcaatagcagccatctaaccagtttagcaacagaatataagctctgagagggtgggagtgaatatgttaccacattgtacaacacagcacatagggcataaggaggggaaatgctctctggggctttccaggaaggcctgaagtcattgcttctagcaaatggaaatcactccagagtagttatctttgacaagaattgaaatataattgagggaactatcagacctgtaagattttgttttttcctttactaatatgttactttacatttgcatttggtgacatacgtaactaccatttttctgtgactgtaacatctgggcatttttcagagctaaatgtgctatggtcaacttggagctttaatctaattgcctggtccaccaagttctggctgtgtacttgaatagatcactggcagggtacaatgggaacagcctgtcccttggagccaggagaggacaccaaggttgaccaaagctcgttcagttgcccctttagccgaagcgcacctgggccagtcactggctgccagtgccatctaatggctgctctgaaaatgctcagccttgcccggcaacccttcagaagctagcaccgtgcaggcccagcgcctggggaatagggcgagggtggggtagagagaaggaagtggcctcctgaagtagaaatcagcgcttcagaggactttcacttccaaagcctcccctatataaaaaagatttggcccacgcctccccaaatgagagatttattttaggcaaacttattttaaaatgccagcgttcattaggagtgacaagacacttagtcatccacgctttaatgtgaattacttttctcatctaattacatttctttctagcagctggctgagaagatcttctgaaatccaaaatgattgtagggttggcggtgagctgatctccggcctcgaggtggcttcagggggcccacctggttaagggaaatttggcagtgcgagggtagtgctggagagaggggtgggtacagggggctaggggcaccatggatgccccctccttactgtcccctggtgtcttgacctcagcttctgcccacaggcacttgctggattctccaaaagtatctgcagtggctgttccaccaggaggtaattcccttctggtctctttcccctccacatctgcatcctcttcaaatcctgccatttcagaccacatttgagagctctagagaacaagacatctgacacgtgacgtgtccagaagatgagccagatttcaaagaactgagatctgctttaaaaacgaagctctccaaagttactggagtctgggtaatagtgatcaccagagtaatttgtgtgcaggacatcaaatcaggctgctcgaaatgctgcctaaattggccagtggttttatttgcttttctgtcaacctaatattcataggaaatagagtttcagaggaatgataggatcctggtggaataaaaagggaaaagaccatcttgagcaggagtttcagggtcctccgtttttcccaagttactttcactcctgagatcttgcatgttagaactacagcttaatgtagtgaaataggaaagttctctgttaggagcttagccttaccttgtcatggacattaaagtaattgtctctctttgggcttcaattttcccatctctcatgggaagggctgaaccaagcaatccccaaaatagcttccagccttaacctttttaggggtctcgtttaaatagaagataacagggaaatggtcacagtttacccaggtccattccctcctccttatcacaacttataccaccgctgtactgcacacctcctttctcagcattgctgctgtccttaaaatgcctttaactccacaagagagtgtgttgttaatgttggctcaaggtccttcctggtgagtggccaacattgttttgctccttgcaggggtcccaccaatcttgtttgcttctgcagagcctcagcctgcctggaagatgccgagatcgtgctgcagccgctcgggggccctgttgctggccttgctgcttcaggcctccatggaagtgcgtggctggtgcctggagagcagccagtgtcaggacctcaccacggaaagcaacctgctggtacgtgggccatgactgccatcttggcttagacattagatgggactggagctgggaaagctcaaaagaaaagggtgtggggaaagggaaattcattcccagtgataggcgtgattcaatccagggcaggagcaaaactttgcagtgaagtaagaaatgggagaagaaatcagggaaggaagcagcttcagggagaggggttgagtccacaatttctgcttggttatccttacttcttgccccatcttttatggagaccttgaaccctttaagctagagatggtgctataagagcaataatggacccctcaatctattctgtactttacatctttagcttcccaaactattcctttttaagaagctcatatcacttgccattttcattccatatttcttacccttttatctactaccggttgcaaaaccagccaggtagttcttcaaatcatctctggaagaaggaaaaaccaggggcccttttttttttttctttaattggtgccaaatgtctcatgtttattctggaggactggccttctgctgtgttcctctacagtctttccagagcatgtgaaggcctttgcatcaggcaggagctccctccaggtcaccacagggtgtatgtatctgcctgtggggggtgtgtgtgtgtgtgtgttggggggcataaatgagtaatgatgccaaatccagagattaaaaggcacactgagaccaggcgagatggctcatggctgtaatcccagcacttttagatgctaaggtgggaggattgcttgagcccagggattcaagacaagcctgggcaacatagtgagacctccacttctacaaaaaataaaaaagttagccagatgtggtggcatgtgcctgtagtcctagctacttgggaggttcacttgaggccaggagtctgacgacacagtaagctatgatcacaccattgcactccagtctgggtaacagaatgagaccttgtctcaaaacaaaacaaaatgaaacaaacaaacaaacaaacccccatactgttagtgtcagtgaccggaattttaatcttgttgccatcacctggcaggtgctgagggtggaatgtacataactacattctgtgtattttgtcaatgcagaagctgagttaaggtgaagatagaatgaggtcctcaaagacacagaccagttttcatgtgtaatataaaatagaaacaaagagcccaggggattctgtgagttccagtttggaaagacccaagagtctcttgacttgagacacccacagcacagctcaccagggagggtgcactggacacagtcaggacccatgggttctagacccagttttgaggtgtgggaccttgaccaggtcctatcacctctctgagtctcctgtttcactatctgtccacgggaggggagtgtaaattagttttttccattgttaacgttccacagagttgtaattctgaacacctggagtaggcaatgtccagctcaacagagtgggtaggatccttttattttctcctttgctattcccaagaaagagagcagccagtgagcttttcatctttttatcactgaaaactcaaggctgcagcctatgcagccattttcctaagctaatatgtaccacaatagagtcctctagggacaaggagcagagacacaggttccacagacggtgcaatggaaataacgctagctttccacccctccctccagtcagaatgagattacagggaaataagcttgccccagagctcactgggggatctctcagaaatcagctcagaagtcgtgaaagaaccaaggtgcagttttggaggcttagtgcagagatggagctggggtagggcataaagtaggttttccatcactgaggtaaggttgaggcattattttttattttttgtttatttatttatttttttgagacggagtctcgctctatcacccaggctggagtgcagtggcgcgatctcccctcactgcaagctccacctcccaggttcacacaggttgaagcattattaaaaatatgtttaaaaatatgggccctagtagccagacttctatcacctggagagattatcccccaaatttcagccccactcccctcctggacttgaattaaaccatatgtatttattcaatattctttttatttatttatttatttttttgagacggagtcttgctctgttgccctggctggagtgtggagtgcagtggtgtgatcttggctcactgcaacctctacctcccaggttcaagcggttctcctgcctcaggctccagagtagctgggattacaggcgcccgccaccacacccagcttatttatttatttatactagagatggtatttcaccatagttggccaggctggtcttgaactcctgacctcatgtgatctgcctgccttggcctcccaaagtgctgggattataggtgtgagccaccatgcccggccctcaatattcattaagtgccaacaactaccacccgtctgcctttcttggagccactcctttatgtcaggcatatgacagtaagactttggtcctgttcacaaaagctaggggtggctagatggctagacaaaccatggaatgggatgggaagtgtgttgcagttgccagcagaagcatgaaggggatgggacaaaagaggcggtggcaagatcttagatgcccacgagtgccaagaaagcaggtgggcagacctgctctgtagggaggcctcgacgcttgacacgcccgacactgtgccctgtgtcctcggcacgtggcgagggcggccagggcctaggcgcagtgacgggcgcggcagccgggccggggtgcggggcacgggctgccctcatgccctcgcgtcttcccccaggagtgcatccgggcctgcaagcccgacctctcggccgagactcccatgttcccgggaaatggcgacgagcagcctctgaccgagaacccccggaagtacgtcatgggccacttccgctgggaccgattcggccgccgcaacagcagcagcagcggcagcagcggcgcagggcagaagcgcgaggacgtctcagcgggcgaagactgcggcccgctgcctgagggcggccccgagccccgcagcgatggtgccaagccgggcccgcgcgagggcaagcgctcctactccatggagcacttccgctggggcaagccggtgggcaagaagcggcgcccagtgaaggtgtaccctaacggcgccgaggacgagtcggccgaggccttccccctggagttcaagagggagctgactggccagcgactccgggagggagatggccccgacggccctgccgatgacggcgcaggggcccaggccgacctggagcacagcctgctggtggcggccgagaagaaggacgagggcccctacaggatggagcacttccgctggggcagcccgcccaaggacaagcgctacggcggtttcatgacctccgagaagagccagacgcccctggtgacgctgttcaaaaacgccatcatcaagaacgcctacaagaagggcgagtgagggcacagcgggccccagggctaccctcccccaggaggtcgaccccaaagccccttgctctcccctgccctgctgccgcctcccagcctggggggtcgtggcagataatcagcctcttaaagctgcctgtagttaggaaataaaacctttcaaatttcacatccacctctgactttgaatgtaaactgtgtgaataaagtaaaaatacgtagccgtcaaataacagcagcatggatcggaggagcacagtggtttccatgcggtaggatatttcacaggacttagtgagcgtgaaaggaaaatgtgcttcctgcccccacccccaaatggatcttcgagggatcagatagtttgggtgaaggcacagggtggctccagcacctctaggatggccgtattttccacacactccactgagtgggagactgctcagctagcacacgtgtaaaggcaggattcctgcaagagtgaccc

SEQ ID NO: 565 - protein, 9 aa, synthetic construct
  REGION 1..9: note = Description of Artificial Sequence: Synthetic peptide
RKKRRQRRR

SEQ ID NO: 566 - protein, 11 aa, synthetic construct
  REGION 1..11: note = Description of Artificial Sequence: Synthetic peptide
YARKARRQARR

SEQ ID NO: 567 - protein, 11 aa, synthetic construct
  REGION 1..11: note = Description of Artificial Sequence: Synthetic peptide
YARAARRAARR

SEQ ID NO: 568 - protein, 11 aa, synthetic construct
  REGION 1..11: note = Description of Artificial Sequence: Synthetic peptide
YARRRRRRRRR

SEQ ID NO: 569 - protein, 11 aa, synthetic construct
  REGION 1..11: note = Description of Artificial Sequence: Synthetic peptide
YAAARRRRRRR

SEQ ID NO: 570 - protein, 11 aa, synthetic construct
  REGION 1..11: note = Description of Artificial Sequence: Synthetic peptide
YARAPRRARRR

SEQ ID NO: 571 - protein, 10 aa, synthetic construct
  REGION 1..10: note = Description of Artificial Sequence: Synthetic peptide
YARAPRRPRR

SEQ ID NO: 572 - protein, 9 aa, synthetic construct
  REGION 1..9: note = Description of Artificial Sequence: Synthetic peptide
RKQKRRRRR

SEQ ID NO: 573 - protein, 9 aa, synthetic construct
  REGION 1..9: note = Description of Artificial Sequence: Synthetic peptide
RKKRQRRRR

SEQ ID NO: 574 - protein, 9 aa, synthetic construct
  REGION 1..9: note = Description of Artificial Sequence: Synthetic peptide
RKKRRRQRR

SEQ ID NO: 575 - protein, 9 aa, synthetic construct
  REGION 1..9: note = Description of Artificial Sequence: Synthetic peptide
RKKRRRRQR

SEQ ID NO: 576 - protein, 9 aa, synthetic construct
  REGION 1..9: note = Description of Artificial Sequence: Synthetic peptide
RKKRRRRRQ

SEQ ID NO: 577 - protein, 9 aa, synthetic construct
  REGION 1..9: note = Description of Artificial Sequence: Synthetic peptide
RKKQRRRRR

SEQ ID NO: 578 - protein, 9 aa, synthetic construct
  REGION 1..9: note = Description of Artificial Sequence: Synthetic peptide
RQKKRRRRR

SEQ ID NO: 579 - protein, 9 aa, synthetic construct
  REGION 1..9: note = Description of Artificial Sequence: Synthetic peptide
RQRRRRRRR

SEQ ID NO: 580 - protein, 10 aa, synthetic construct
  REGION 1..10: note = Description of Artificial Sequence: Synthetic peptide
RQRRRRRRRR

SEQ ID NO: 581 - protein, 9 aa, synthetic construct
  REGION 1..9: note = Description of Artificial Sequence: Synthetic peptide
RRQRRRRRR

SEQ ID NO: 582 - protein, 10 aa, synthetic construct
  REGION 1..10: note = Description of Artificial Sequence: Synthetic peptide
RRQRRRRRRR

SEQ ID NO: 583 - protein, 9 aa, synthetic construct
  REGION 1..9: note = Description of Artificial Sequence: Synthetic peptide
RRRQRRRRR

SEQ ID NO: 584 - protein, 10 aa, synthetic construct
  REGION 1..10: note = Description of Artificial Sequence: Synthetic peptide
RRRQRRRRRR

SEQ ID NO: 585 - protein, 9 aa, synthetic construct
  REGION 1..9: note = Description of Artificial Sequence: Synthetic peptide
RRRRQRRRR

SEQ ID NO: 586 - protein, 10 aa, synthetic construct
  REGION 1..10: note = Description of Artificial Sequence: Synthetic peptide
RRRRQRRRRR

SEQ ID NO: 587 - protein, 5 aa, synthetic construct
  REGION 1..5: note = Description of Artificial Sequence: Synthetic peptide
RRRRR

SEQ ID NO: 588 - protein, 9 aa, synthetic construct
  REGION 1..9: note = Description of Artificial Sequence: Synthetic peptide
RRRRRQRRR

SEQ ID NO: 589 - protein, 10 aa, synthetic construct
  REGION 1..10: note = Description of Artificial Sequence: Synthetic peptide
RRRRRQRRRR

SEQ ID NO: 590 - protein, 6 aa, synthetic construct
  REGION 1..6: note = Description of Artificial Sequence: Synthetic peptide
RRRRRR

SEQ ID NO: 591 - protein, 10 aa, synthetic construct
  REGION 1..10: note = Description of Artificial Sequence: Synthetic peptide
RRRRRRQRRR

SEQ ID NO: 592 - protein, 7 aa, synthetic construct
  REGION 1..7: note = Description of Artificial Sequence: Synthetic peptide
RRRRRRR

SEQ ID NO: 593 - protein, 10 aa, synthetic construct
  REGION 1..10: note = Description of Artificial Sequence: Synthetic peptide
RRRRRRRQRR

SEQ ID NO: 594 - protein, 8 aa, synthetic construct
  REGION 1..8: note = Description of Artificial Sequence: Synthetic peptide
RRRRRRRR

SEQ ID NO: 595 - protein, 9 aa, synthetic construct
  REGION 1..9: note = Description of Artificial Sequence: Synthetic peptide
  REGION 1..7: note = MISC_FEATURE - This region may encompass 1-7 residues
RRRRRRRQR

SEQ ID NO: 596 - protein, 9 aa, synthetic construct
  REGION 1..9: note = Description of Artificial Sequence: Synthetic peptide
RRRRRRRRR

SEQ ID NO: 597 - protein, 10 aa, synthetic construct
  REGION 1..10: note = Description of Artificial Sequence: Synthetic peptide
RRRRRRRRRQ

SEQ ID NO: 598 - protein, 5 aa, synthetic construct
  REGION 1..5: note = Description of Artificial Sequence: Synthetic peptide
  MOD_RES 1..5: note = D-Arginine
RRRRR

SEQ ID NO: 599 - protein, 6 aa, synthetic construct
  REGION 1..6: note = Description of Artificial Sequence: Synthetic peptide
  MOD_RES 1..6: note = D-Arginine
RRRRRR

SEQ ID NO: 600 - protein, 7 aa, synthetic construct
  REGION 1..7: note = Description of Artificial Sequence: Synthetic peptide
  MOD_RES 1..7: note = D-Arginine
RRRRRRR

SEQ ID NO: 601 - protein, 8 aa, synthetic construct
  REGION 1..8: note = Description of Artificial Sequence: Synthetic peptide
  MOD_RES 1..8: note = D-Arginine
RRRRRRRR

SEQ ID NO: 602 - protein, 9 aa, synthetic construct
  REGION 1..9: note = Description of Artificial Sequence: Synthetic peptide
  MOD_RES 1..9: note = D-Arginine
RRRRRRRRR

SEQ ID NO: 603 - protein, 9 aa, synthetic construct
  REGION 1..9: note = Description of Artificial Sequence: Synthetic peptide
QRKKRRRRR

SEQ ID NO: 604 - protein, 9 aa, synthetic construct
  REGION 1..9: note = Description of Artificial Sequence: Synthetic peptide
QRRRRRRRR

SEQ ID NO: 605 - protein, 10 aa, synthetic construct
  REGION 1..10: note = Description of Artificial Sequence: Synthetic peptide
QRRRRRRRRR

SEQ ID NO: 606 - protein, 11 aa, synthetic construct
  REGION 1..11: note = Description of Artificial Sequence: Synthetic peptide
YGRKKRRQRRR

SEQ ID NO: 607 - protein, 12 aa, synthetic construct
  REGION 1..12: note = Description of Artificial Sequence: Synthetic peptide
  MOD_RES 12: note = 8-amino-3,6-dioxaoctanoic acid
YGRKKRRQRRRX

SEQ ID NO: 608 - protein, 4 aa, synthetic construct
  REGION 1..4: note = Description of Artificial Sequence: Synthetic peptide
  MOD_RES 1..2: note = Beta-Alanine
AAYG

SEQ ID NO: 609 - skipped

SEQ ID NO: 610 - protein, 9 aa, synthetic construct
  REGION 1..9: note = Description of Artificial Sequence: Synthetic peptide
RKRRRQRRR

SEQ ID NO: 611 - protein, 9 aa, synthetic construct
  REGION 1..9: note = Description of Artificial Sequence: Synthetic peptide
RRKRRQRRR

SEQ ID NO: 612 - protein, 9 aa, synthetic construct
  REGION 1..9: note = Description of Artificial Sequence: Synthetic peptide
  REGION 3..9: note = MISC_FEATURE - This region may encompass 1-7 residues
RQRRRRRRR

SEQ ID NO: 613 - protein, 11 aa, synthetic construct
  REGION 1..11: note = Description of Artificial Sequence: Synthetic peptide
  REGION 1..7: note = MISC_FEATURE - This region may encompass 1-7 residues
RRRRRRRQRRR

SEQ ID NO: 614 - protein, 12 aa, synthetic construct
  REGION 1..12: note = Description of Artificial Sequence: Synthetic peptide
  VARIANT 4: note = D-isomer of halogen substituted Phenylalanine or Beta-(2-naphthyl)alanine
  VARIANT 6: note = 3-benzothienylalanine, Beta-(1-naphthyl)alanine, Beta-(2-naphthyl)alanine or Tryptophan
  VARIANT 7: note = alpha-aminoisobutyric acid, Alanine, Beta-Alanine or Glycine
CEHXRXXCPPKD